European Patent Specification EP 3 957 367 B1, published January 14, 2026. Title: ANTIMICROBIAL COMPOSITION AGAINST DRUG-RESISTANT BACTERIUM OR PRO-INFLAMMATORY BACTERIUM. Applicant: KEIO UNIVERSITY. The sequence listing filed with the application follows.

SEQUENCE LISTING (235 sequences)

SEQ ID NO: 1 - DNA, 1391 bp, Unknown
  K01
gcaagtcgagcgaagcgctgttttcagaatcttcggaggaagaggacagcgactgagcggcggacgggtgagtaacgcgtgggcaacctgcctcatacagggggataacagttagaaatgactgctaataccgcataagcgcacgggaccgcatggtctagtgtgaaaaactccggtggtatgagatggacccgcgtctgattaggtagttggtggggtaaaggcctaccaagccgacgatcagtagccgacctgagagggtgaccggccacattgggactgagacacggcccaaactcctacgggaggcagcagtggggaatattgcacaatgggggaaaccctgatgcagcgacgccgcgtgaaggaagaagtatttcggtatgtaaacttctatcagcagggaagaaaatgacggtacctgagtaagaagcaccggctaaatacgtgccagcagccgcggtaatacgtatggtgcaagcgttatccggatttactgggtgtaaagggagcgtagacggataggcaagtctggagtgaaaacccagggctcaaccctgggactgctttggaaactgcagatctggagtgccggagaggtaagcggaattcctagtgtagcggtgaaatgcgtagatattaggaggaacaccagtggcgaaggcggcttactggacggtgactgacgttgaggctcgaaagcgtggggagcaaacaggattagataccctggtagtccacgccgtaaacgatgactactaggtgtcggtgtgcaaagcacatcggtgccgcagcaaacgcaataagtagtccacctggggagtacgttcgcaagaatgaaactcaaaggaattgacggggacccgcacaagcggtggagcatgtggtttaattcgaagcaacgcgaagaaccttacctggtcttgacatccggatgacgggcgagtaatgtcgccgtcccttcggggcatccgagacaggtggtgcatggttgtcgtcagctcgtgtcgtgagatgttgggttaagtcccgcaacgagcgcaacccttatcttcagtagccagcatataaggtgggcactctggagagactgccagggagaacctggaggaaggtggggatgacgtcaaatcatcatgccccttatggccagggctacacacgtgctacaatggcgtaaacaaagggaagcgagagggtgacctgaagcgaatcccaaaaataacgtctcagttcggattgtagtctgcaactcgactacatgaagctggaatcgctagtaatcgcggatcagcatgccgcggtgaatacgttcccgggtcttgtacacaccgcccgtcacaccatgggagtcagtaacgcccgaagccagtgacccaaccttgaggagg

SEQ ID NO: 2 - DNA, 1383 bp, Unknown
  K02
tcgaggggcagcattttagtttgcttgcaaactgaagatggcgaccggcgcacgggtgagtaacacgtatccaacctgccgataactccggaatagcctttcgaaagaaagattaataccggatagcatacgaatatcgcatgatatttttattaaagaatttcggttatcgatggggatgcgttccattagtttgttggcggggtaacggcccaccaagactacgatggataggggttctgagaggaaggtcccccacattggaactgagacacggtccaaactcctacgggaggcagcagtgaggaatattggtcaatgggcgagagcctgaaccagccaagtagcgtgaaggatgaaggctctatgggtcgtaaacttcttttatatgggaataaagttttccacgtgtggaattttgtatgtaccatatgaataaggatcggctaactccgtgccagcagccgcggtaatacggaggatccgagcgttatccggatttattgggtttaaagggagcgtaggtggattgttaagtcagttgtgaaagtttgcggctcaaccgtaaaattgcagttgaaactggcagtcttgagtacagtagaggtgggcggaattcgtggtgtagcggtgaaatgcttagatatcacgaagaactccgattgcgaaggcagctcactagactgttactgacactgatgctcgaaagtgtgggtatcaaacaggattagataccctggtagtccacacagtaaacgatgaatactcgctgtttgcgatatacagtaagcggccaagcgaaagcattaagtattccacctggggagtacgccggcaacggtgaaactcaaaggaattgacgggggcccgcacaagcggaggaacatgtggtttaattcgatgatacgcgaggaaccttacccgggcttaaattgcaacagaatatattggaaacagtatagccgtaaggctgttgtgaaggtgctgcatggttgtcgtcagctcgtgccgtgaggtgtcggcttaagtgccataacgagcgcaacccttatctttagttactaacaggttatgctgaggactctagagagactgccgtcgtaagatgtgaggaaggtggggatgacgtcaaatcagcacggcccttacgtccggggctacacacgtgttacaatggggggtacagaaggcggctacctggtgacaggatgctaatcccaaaaacctctctcagttcggatcgaagtctgcaacccgacttcgtgaagctggattcgctagtaatcgcgcatcagccatggcgcggtgaatacgttcccgggccttgtacacaccgcccgtcaagccatgaaagccgggggtacctgaagtacgtaaccgcaa

SEQ ID NO: 3 - DNA, 1396 bp, Unknown
  K03
tgcagtcgagcgaagcgctaagacaggatttcttcggattgaagtctttgtgactgagcggcggacgggtgagtaacgcgtgggtaacctgcctcatacagggggataacagttagaaatgactgctaataccgcataagcgcacaggaccgcatggtctggtgtgaaaaactccggtggtatgagatggacccgcgtctgattagctagttggaggggtaacggcccaccaaggcgacgatcagtagccggcctgagagggtgaacggccacattgggactgagacacggcccagactcctacgggaggcagcagtggggaatattgcacaatgggggaaaccctgatgcagcgacgccgcgtgaaggaagaagtatctcggtatgtaaacttctatcagcagggaagaaaatgacggtacctgactaagaagccccggctaactacgtgccagcagccgcggtaatacgtagggggcaagcgttatccggatttactgggtgtaaagggagcgtagacggaagagcaagtctgatgtgaaaggctggggcttaaccccaggactgcattggaaactgttgttctagagtgccggagaggtaagcggaattcctagtgtagcggtgaaatgcgtagatattaggaggaacaccagtggcgaaggcggcttactggacggtaactgacgttgaggctcgaaagcgtggggagcaaacaggattagataccctggtagtccacgccgtaaacgatgaatactaggtgtcgggtggcaaagccattcggtgccgcagcaaacgcaataagtattccacctggggagtacgttcgcaagaatgaaactcaaaggaattgacggggacccgcacaagcggtggagcatgtggtttaattcgaagcaacgcgaagaaccttaccaagtcttgacatccctctgaccgtcccgtaacgggggcttcccttcggggcagaggagacaggtggtgcatggttgtcgtcagctcgtgtcgtgagatgttgggttaagtcccgcaacgagcgcaacccttatccttagtagccagcacatgatggtgggcactctagggagactgccggggataacccggaggaaggcggggacgacgtcaaatcatcatgccccttatgatttgggctacacacgtgctacaatggcgtaaacaaagggaagcgagacagcgatgttgagcgaatcccaaaaataacgtcccagttcggactgcagtctgcaactcgactgcacgaagctggaatcgctagtaatcgcggatcagaatgccgcggtgaatacgttcccgggtcttgtacacaccgcccgtcacaccatgggagtcagtaacgcccgaagtcagtgacctaaccgaaaggaaggag

SEQ ID NO: 4 - DNA, 1395 bp, Unknown
  K04
cagtcgagcgaagcgtcttagaatgatctcttcggattgagtcttatatgactgagcggcggacgggtgagtaacgcgtgggtaacctgcctcatacagggggataacagttagaaatgactgctaataccgcataagcgcacagggctgcatggcctggtgtgaaaaactccggtggtatgagatggacccgcgtctgattagctagttggaggggtaacggcccaccaaggcgacgatcagtagccggcctgagagggtgaacggccacattgggactgagacacggcccagactcctacgggaggcagcagtggggaatattgcacaatgggggaaaccctgatgcagcgacgccgcgtgaaggaagaagtatctcggtatgtaaacttctatcagcagggaagaaaatgacggtacctgactaagaagccccggctaactacgtgccagcagccgcggtaatacgtagggggcaagcgttatccggatttactgggtgtaaagggagcgtagacggaagagcaagtctgatgtgaaaggctggggcttaaccccaggactgcattggaaactgtttttctagagtgccggagaggtaagcggaattcctagtgtagcggtgaaatgcgtagatattaggaggaacaccagtggcgaaggcggcttactggacggtaactgacgttgaggctcgaaagcgtggggagcaaacaggattagataccctggtagtccacgccgtaaacgatgaatactaggtgtcgggtggcaaagccattcggtgccgcagcaaacgcaataagtattccacctggggagtacgttcgcaagaatgaaactcaaaggaattgacggggacccgcacaagcggtggagcatgtggtttaattcgaagcaacgcgaagaaccttaccaagtcttgacatccttctgacgtgcccgtaacggggcattcccttcggggcagaggagacaggtggtgcatggttgtcgtcagctcgtgtcgtgagatgttgggttaagtcccgcaacgagcgcaacccctatccttagtagccagcacatcatggtgggcactctagggagactgccggggataacccggaggaaggcggggacgacgtcaaatcatcatgccccttatgatttgggctacacacgtgctacaatggcgtaaacaaagggaagcgagacagcgatgtttagcaaatcccaaaaataacgtcccagttcggactgcagtctgcaactcgactgcacgaagctggaatcgctagtaatcgcgaatcagaatgtcgcggtgaatacgttcccgggtcttgtacacaccgcccgtcacaccatgggagtcagtaacgcccgaagtcagtgacccaacctcacggagggagc

SEQ ID NO: 5 - DNA, 1411 bp, Unknown
  K05
gcagtcgaacgtgaaagtccttcgggacgagtaaagtggcgcacgggtgagtaacgcgtggataatctacccttaagatggggataacggctggaaacggtcgctaataccgaatacgctcccgattttatcattggggggaaagatggcctctgcttgcaagctatcgcttaaggatgagtccgcgtcccattagctagttggcggggtaacggcccaccaaggcgacgatgggtagccggtctgagaggatgaccggccacactggaactggaacacggtccagactcctacgggaggcagcagtggggaatattgcgcaatgggcgaaagcctgacgcagcgacgccgcgtgagggatgaaggttctcggatcgtaaacctctgtcaggggggaagaaaccccctcgtgtgaataatgcgagggcttgacggtacccccaaaggaagcaccggctaactccgtgccagcagccgcggtaatacggagggtgcaagcgttaatcggaatcactgggcgtaaagcgcacgtaggcggcttggtaagtcaggggtgaaatcccacagcccaactgtggaactgcctttgatactgccaggcttgagtaccggagagggtggcggaattccaggtgtaggagtgaaatccgtagatatctggaggaacaccggtggcgaaggcggccacctggacggtaactgacgctgaggtgcgaaagcgtgggtagcaaacaggattagataccctggtagtccacgctgtaaacgatgggtgctgggtgctgggatgtatgtctcggtgccgtagctaacgcgataagcaccccgcctggggagtacggtcgcaaggctgaaactcaaagaaattgacgggggcccgcacaagcggtggagtatgtggtttaattcgatgcaacgcgaagaaccttacccaggcttgacatctagggaacccttcggaaatgaaggggtgcccttcggggagccctaagacaggtgctgcatggctgtcgtcagctcgtgccgtgaggtgttgggttaagtcccgcaacgagcgcaacccctatcttcagttgccagcaggtaaggctgggcactctggagagaccgccccggtcaacggggaggaaggtggggacgacgtcaagtcatcatggcccttacgcctggggctacacacgtactacaatggcgcgcacaaagggtagcgagaccgcgaggtggagccaatcccaaaaaacgcgtcccagtccggattggagtctgcaactcgactccatgaagtcggaatcgctagtaattcgagatcagcatgctcgggtgaatgcgttcccgggccttgtacacaccgcccgtcacaccacgaaagtcggttttacccgaagccggtgagctaactcgcaagagaagc

SEQ ID NO: 6 - DNA, 1383 bp, Unknown
  K06
gaggggcatcgggattgaagcttgcttcaattgccggcgaccggcgcacgggtgcgtaacgcgtatgtaacctacctataacaggggcataacactgagaaattggtactaattccccataatattcggagaggcatctctccgggttgaaaactccggtggttatagatggacatgcgttgtattagctagttggtgaggtaacggctcaccaaggcaacgatacatagggggactgagaggttaaccccccacactggtactgagacacggaccagactcctacgggaggcagcagtgaggaatattggtcaatggacgcaagtctgaaccagccatgccgcgtgcaggaagacggctctatgagttgtaaactgcttttgtacgagggtaaactcacctacgtgtaggtgactgaaagtatcgtacgaataaggatcggctaactccgtgccagcagccgcggtaatacggaggattcaagcgttatccggatttattgggtttaaagggtgcgtaggcggtttgataagttagaggtgaaatcccggggcttaactccggaactgcctctaatactgttagactagagagtagttgcggtaggcggaatgtatggtgtagcggtgaaatgcttagagatcatacagaacaccgattgcgaaggcagcttaccaaactatatctgacgttgaggcacgaaagcgtggggagcaaacaggattagataccctggtagtccacgcagtaaacgatgataactcgttgtcggcgatacacagtcggtgactaagcgaaagcgataagttatccacctgggggagtacgttcgcaagaatgaaactcaaaggaattgacgggggcccgcacaagcggaggaacatgtggtttaattcgatgatacgcgaggaaccttacccgggcttgaaagttactgacgattctggaaacaggatttcccttcggggcaggaaactaggtgctgcatggttgtcgtcagctcgtgccgtgaggtgtcgggttaagtcccataacgagcgcaacccctaccgttagttgccatcaggtcaagctgggcactctggcgggactgccggtgtaagccgagaggaaggtggggatgacgtcaaatcagcacggcccttacgtccggggctacacacgtgttacaatggtaggtacagagggtcgctaccccgtgaggggatgccaatctcgaaagcctatctcagttcggattggaggctgaaacccgcctccatgaagttggattcgctagtaatcgcgcatcagccatggcgcggtgaatacgttcccgggccttgtacacaccgcccgtcaagccatggaagctgggggtgcctgaagttcgtgaccgcaagg

SEQ ID NO: 7 - DNA, 1393 bp, Unknown
  K07
cagtcgaacggagttatgcagaggaagttttcggatggaatcggcgtaacttagtggcggacgggtgagtaacgcgtgggaaacctgccctgtaccgggggataacacttagaaataggtgctaataccgcataagcgcacagcttcacatgaggcagtgtgaaaaactccggtggtacaggatggtcccgcgtctgattagccagttggcagggtaacggcctaccaaagcgacgatcagtagccggcctgagagggtgaacggccacattgggactgagacacggcccaaactcctacgggaggcagcagtggggaatattgcacaatgggggaaaccctgatgcagcgacgccgcgtgagtgaagaagtatttcggtatgtaaagctctatcagcagggaagaaaatgacggtacctgactaagaagccccggctaactacgtgccagcagccgcggtaatacgtagggggcaagcgttatccggatttactgggtgtaaagggagcgtagacggcatgacaagccagatgtgaaaacccagggctcaaccctgggactgcatttggaactgccaggctggagtgcaggagaggtaagcggaattcctagtgtagcggtgaaatgcgtagatattaggaggaacaccagtggcgaaggcggcttactggactgtaactgacgttgaggctcgaaagcgtggggagcaaacaggattagataccctggtagtccacgcggtaaacgatgattgctaggtgtaggtgggtatggacccatcggtgccgcagctaacgcaataagcaatccacctgggggagtacgttcgcaagaatgaaactcaaaggaattgacggggacccgcacaagcggtggagcatgtggtttaattcgaagcaacgcgaagaaccttaccaagtcttgacatcccaatgacgtgtccgtaacggggcattctcttcggagcattggagacaggtggtgcatggttgtcgtcagctcgtgtcgtgagatgttgggttaagtcccgcaacgagcgcaacccttatccttagtagccagcaggtagagctgggcactctagggagactgccggggataacccggaggaaggcggggatgacgtcaaatcatcatgccccttatgatttgggctacacacgtgctacaatggcgtaaacaaagggaagcgagacagtgatgttgagcaaatcccagaaataacgtctcagttcggattgtagtctgcaactcgactacatgaagctggaatcgctagtaatcgcgaatcagcatgtcgcggtgaatacgttcccgggtcttgtacacaccgcccgtcacaccatgggagttggaaatgcccgaagcctgtgacctaaccgcaagggagga

SEQ ID NO: 8 - DNA, 1402 bp, Unknown
  K08
  misc_feature (947)..(949): n is a, c, g, or t
  misc_feature (953)..(955): n is a, c, g, or t
  misc_feature (967)..(970): n is a, c, g, or t
caagtcgaacgaagtttcgaggaagcttgcttccaaagagacttagtggcgaacgggtgagtaacacgtaggtaacctgcccatgtgtccgggataactgctggaaacggtagctaaaaccggataggtatacagagcgcatgctcagtatattaaagcgcccatcaaggcgtgaacatggatggacctgcggcgcattagctagttggtgaggtaacggcccaccaaggcgatgatgcgtagccggcctgagagggtaaacggccacattgggactgagacacggcccaaactcctacgggaggcagcagtagggaattttcgtcaatgggggaaaccctgaacgagcaatgccgcgtgagtgaagaaggtcttcggatcgtaaagctctgttgtaagtgaagaacggctcatagaggaaatgctatgggagtgacggtagcttaccagaaagccacggctaactacgtgccagcagccgcggtaatacgtaggtggcaagcgttatccggaatcattgggcgtaaagggtgcgtaggtggcgtactaagtctgtagtaaaaggcaatggctcaaccattgtaagctatggaaactggtatgctggagtgcagaagagggcgatggaattccatgtgtagcggtaaaatgcgtagatatatggaggaacaccagtggcgaaggcggtcgcctggtctgtaactgacactgaggcacgaaagcgtggggagcaaataggattagataccctagtagtccacgccgtaaacgatgagaactaagtgttggaggaattcagtgctgcagttaacgcaataagttctccgcctggggagtatgcacgcaagtgtgaaactcaaaggaattgacgggggcccgcacaagcggtggagtatgtggtttaattcgaagcaacgcgaagaaccttaccaggccttgacatggannnaaannncctagagatagnnnnataattatggatcacacaggtggtgcatggttgtcgtcagctcgtgtcgtgagatgttgggttaagtcccgcaacgagcgcaacccttgtcgcatgttaccagcatcaagttggggactcatgcgagactgccggtgacaaaccggaggaaggtggggatgacgtcaaatcatcatgccccttatggcctgggctacacacgtactacaatggcgaccacaaagagcagcgacacagtgatgtgaagcgaatctcataaaggtcgtctcagttcggattgaagtctgcaactcgacttcatgaagtcggaatcgctagtaatcgcagatcagcatgctgcggtgaatacgttctcgggccttgtacacaccgcccgtcaaaccatgggagtcagtaatacccgaagccggtggcataaccgtaaggagtgag

SEQ ID NO: 9 - DNA, 1386 bp, Unknown
  K09
agtcgaggggcatcaggaagaaagcttgctttctttgctggcgaccggcgcacgggtgagtaacacgtatccaacctgccctttactcggggatagcctttcgaaagaaagattaatacccgatggcataatgattccgcatggtttcattattaaaggattccggtaaaggatggggatgcgttccattaggttgttggtgaggtaacggctcaccaagccttcgatggataggggttctgagaggaaggtcccccacattggaactgagacacggtccaaactcctacgggaggcagcagtgaggaatattggtcaatgggcgctagcctgaaccagccaagtagcgtgaaggatgaaggctctatgggtcgtaaacttcttttatataagaataaagtgcagtatgtatactgttttgtatgtattatatgaataaggatcggctaactccgtgccagcagccgcggtaatacggaggatccgagcgttatccggatttattgggtttaaagggagcgtaggtggactggtaagtcagttgtgaaagtttgcggctcaaccgtaaaattgcagttgatactgtcagtcttgagtacagtagaggtgggcggaattcgtggtgtagcggtgaaatgcttagatatcacgaagaactccgattgcgaaggcagctcactggactgcaactgacactgatgctcgaaagtgtgggtatcaaacaggattagataccctggtagtccacacagtaaacgatgaatactcgctgtttgcgatatacagtaagcggccaagcgaaagcattaagtattccacctggggagtacgccggcaacggtgaaactcaaaggaattgacgggggcccgcacaagcggaggaacatgtggtttaattcgatgatacgcgaggaaccttacccgggcttaaattgcagtggaatgatgtggaaacatgtcagtgagcaatcaccgctgtgaaggtgctgcatggttgtcgtcagctcgtgccgtgaggtgtcggcttaagtgccataacgagcgcaacccttatcttcagttactaacaggtcatgctgaggactctggagagactgccgtcgtaagatgtgaggaaggtggggatgacgtcaaatcagcacggcccttacgtccggggctacacacgtgttacaatggggggtacagaaggcagctagcgggtgaccgtatgctaatcccaaaatcctctctcagttcggatcgaagtctgcaacccgacttcgtgaagctggattcgctagtaatcgcgcatcagccacggcgcggtgaatacgttcccgggccttgtacacaccgcccgtcaagccatgggagccgggggtacctgaagtacgtaaccgcaag

SEQ ID NO: 10 - DNA, 1366 bp, Unknown
  K10
agtcgaacgatgaaaccgccctcgggcggacatgaagtggcgaacgggtgagtaacacgtgaccaacctgccccttgctccgggacaaccttgggaaaccgaggctaataccggatactcctcgcccccctcctggggggcccgggaaagcccagacggcaagggatggggtcgcggcccattaggtagtaggcggggtaacggcccacctagcccgcgatgggtagccgggttgagagaccgaccggccacattgggactgagatacggcccagactcctacgggaggcagcagtggggaattttgcgcaatgggggaaaccctgacgcagcaacgccgcgtgcgggacgacggccttcgggttgtaaaccgctttcagcagggaagaaattcgacggtacctgcagaagaagctccggctaactacgtgccagcagccgcggtaatacgtagggagcgagcgttatccggattcattgggcgtaaagagcgcgtaggcggcctctcaagcgggatctctaatccgagggctcaacccccggccggatcccgaactgggaggctcgagttcggtagaggcaggcggaattcccggtgtagcggtggaatgcgcagatatcgggaagaacaccgatggcgaaggcagcctgctgggccgcaactgacgctgaggcgcgaaagctaggggagcgaacaggattagataccctggtagtcctagccgtaaacgatggatactaggtgtggggggctccgccctccgtgccgcagccaacgcattaagtatcccgcctggggagtacggccgcaaggctaaaactcaaaggaattgacgggggcccgcacaagcagcggagcatgtggcttaattcgaagcaacgcgaagaaccttaccagggcttgacatggacgtgaagccggggaaacccggtggccgagaggagcgtccgcaggtggtgcatggctgtcgtcagctcgtgtcgtgagatgttgggttaagtcccgcaacgagcgcaacccctgccccatgttgccagcattaggttggggactcatgggggactgccggcgtcaagccggaggaaggtggggacgacgtcaagtcatcatgccctttatgccctgggctgcacacgtgctacaatggccggtacaacgggctgcgagaccgcgaggtcgagcgaatccctcaaagccggccccagttcggatcggaggctgcaacccgcctccgtgaagtcggagttgctagtaatcgcggatcagcatgccgcggtgaatacgttcccgggccttgtacacaccgcccgtcacaccacccgagtcgtctgcacccgaagccgccggccgaacccgcaaggggcg

SEQ ID NO: 11 - DNA, 1395 bp, Unknown
  K11
cagtcgaacgaagtgaagatagcttgctattggaacttagtggcgaacgggtgagtaacacgtagataacctgcctgtatgaccgggataacagttggaaacgactgctaataccggataggcagagaggaggcatctcttctctgttaaagttgggatacaacgcaaacagatggatctgcggtgcattagctagttggtgaggtaacggcccaccaaggcgatgatgcatagccggcctgagagggcgaacggccacattgggactgagacacggcccaaactcctacgggaggcagcagtagggaattttcggcaatgggggaaaccctgaccgagcaatgccgcgtgagtgaagacggccttcgggttgtaaagctctgttgtaagggaagaacggcatagagagggaatgctctatgagtgacggtaccttaccagaaagccacggctaactacgtgccagcagccgcggtaatacgtaggtggcaagcgttatccggaattattgggcgtaaagggtgcgtaggcggcgagataagtctgaggtaaaagcccgtggctcaaccacggtaagccttggaaactgtctggctggagtgcaggagaggacaatggaattccatgtgtagcggtaaaatgcgtagatatatggaggaacaccagtggcgaaggcggttgtctggcctgtaactgacgctgaagcacgaaagcgtggggagcaaataggattagataccctagtagtccacgccgtaaacgatgagaactaagtgttggggaaactcagtgctgcagttaacgcaataagttctccgcctggggagtatgcacgcaagtgtgaaactcaaaggaattgacgggggcccgcacaagcggtggagtatgtggtttaattcgacgcaacgcgaagaaccttaccaggccttgacatggtatcaaaggccctagagatagggagatagttatgatacacacaggtggtgcatggttgtcgtcagctcgtgtcgtgagatgttgggttaagtcccgcaacgagcgcaacccttgtttctagttaccaacagtaagatggggactctagagagactgccggtgacaaaccggaggaaggtggggatgacgtcaaatcatcatgccccttatggcctgggctacacacgtactacaatggcgtctacaaagagcagcgagcaggtgactgtaagcgaatctcataaaggacgtctcagttcggattgaagtctgcaactcgacttcatgaagtcggaatcgctagtaatcgcggatcagcatgccgcggtgaatacgttctcgggccttgtacacaccgcccgtcaaaccatgggagttgataatacccgaagccggtggcctaaccatttatggagggag

SEQ ID NO: 12 - DNA, 1383 bp, Unknown
  K12
cagtcgaacgcgagcacttgtgctcgagtggcgaacgggtgagtaatacataagtaacctgccctagacagggggataactattggaaacgatagctaagaccgcataggtacggacactgcatggtgaccgtattaaaagtgcctcaaagcactggtagaggatggacttatggcgcattagctggttggcggggtaacggcccaccaaggcgacgatgcgtagccgacctgagagggtgaccggccacactgggactgagacacggcccagactcctacgggaggcagcagtagggaattttcggcaatgggggaaaccctgaccgagcaacgccgcgtgaaggaagaaggttttcggattgtaaacttctgttataaaggaagaacggcggctacaggaaatggtagccgagtgacggtactttattagaaagccacggctaactacgtgccagcagccgcggtaatacgtaggtggcaagcgttatccggaattattgggcgtaaagagggagcaggcggcagcaagggtctgtggtgaaagcctgaagcttaacttcagtaagccatagaaaccaggcagctagagtgcaggagaggatcgtggaattccatgtgtagcggtgaaatgcgtagatatatggaggaacaccagtggcgaaggcgacgatctggcctgcaactgacgctcagtcccgaaagcgtggggagcaaataggattagataccctagtagtccacgccgtaaacgatgagtactaagtgttggatgtcaaagttcagtgctgcagttaacgcaataagtactccgcctgagtagtacgttcgcaagaatgaaactcaaaggaattgacgggggcccgcacaagcggtggagcatgtggtttaattcgaagcaacgcgaagaaccttaccaggtcttgacatactcataaaggctccagagatggagagatagctatatgagatacaggtggtgcatggttgtcgtcagctcgtgtcgtgagatgttgggttaagtcccgcaacgagcgcaacccttatcgttagttaccatcattaagttggggactctagcgagactgccagtgacaagctggaggaaggcggggatgacgtcaaatcatcatgccccttatgacctgggctacacacgtgctacaatggatggtgcagagggaagcgaagccgcgaggtgaagcaaaacccataaaaccattctcagttcggattgtagtctgcaactcgactacatgaagttggaatcgctagtaatcgcgaatcagcatgtcgcggtgaatacgttctcgggccttgtacacaccgcccgtcacaccacgagagttgataacacccgaagccggtggcctaaccgcaagga

SEQ ID NO: 13 - DNA, 1423 bp, Unknown
  K13
  misc_feature (4)..(4): n is a, c, g, or t
tgcnagtcgaacgcttctttcctcccgagtgcttgcactcaattggaaagaggagtggcggacgggtgagtaacacgtgggtaacctacccatcagagggggataacacttggaaacaggtgctaataccgcataacagtttatgccgcatggcataagagtgaaaggcgctttcgggtgtcgctgatggatggacccgcggtgcattagctagttggtgaggtaacggctcaccaaggccacgatgcatagccgacctgagagggtgatcggccacactgggactgagacacggcccagactcctacgggaggcagcagtagggaatcttcggcaatggacgaaagtctgaccgagcaacgccgcgtgagtgaagaaggttttcggatcgtaaaactctgttgttagagaagaacaaggacgttagtaactgaacgtcccctgacggtatctaaccagaaagccacggctaactacgtgccagcagccgcggtaatacgtaggtggcaagcgttgtccggatttattgggcgtaaagcgagcgcaggcggtttcttaagtctgatgtgaaagcccccggctcaaccggggagggtcattggaaactgggagacttgagtgcagaagaggagagtggaattccatgtgtagcggtgaaatgcgtagatatatggaggaacaccagtggcgaaggcggctctctggtctgtaactgacgctgaggctcgaaagcgtggggagcaaacaggattagataccctggtagtccacgccgtaaacgatgagtgctaagtgttggagggtttccgcccttcagtgctgcagcaaacgcattaagcactccgcctggggagtacgaccgcaaggttgaaactcaaaggaattgacgggggcccgcacaagcggtggagcatgtggtttaattcgaagcaacgcgaagaaccttaccaggtcttgacatcctttgaccactctagagatagagctttcccttcggggacaaagtgacaggtggtgcatggttgtcgtcagctcgtgtcgtgagatgttgggttaagtcccgcaacgagcgcaacccttattgttagttgccatcatttagttgggcactctagcgagactgccggtgacaaaccggaggaaggtggggatgacgtcaaatcatcatgccccttatgacctgggctacacacgtgctacaatgggaagtacaacgagtcgctagaccgcgaggtcatgcaaatctcttaaagcttctctcagttcggattgcaggctgcaactcgcctgcatgaagccggaatcgctagtaatcgcggatcagcacgccgcggtgaatacgttcccgggccttgtacacaccgcccgtcacaccacgagagtttgtaacacccgaagtcggtgaggtaacctttttggagcc

SEQ ID NO: 14 - DNA, 1381 bp, Unknown
  K14
aagtcgaggggcatcatgacctagcaataggttgatggcgaccggcgcacgggtgagtaacacgtatccaacctgccgattattccgggatagcctttcgaaagaaagattaatactggatagcataacgagaaggcatcttcttgttattaaagaatttcgataatcgatggggatgcgttccattagtttgttggcggggtaacggcccaccaagacatcgatggataggggttctgagaggaaggtcccccacattggaactgagacacggtccaaactcctacgggaggcagcagtgaggaatattggtcaatggacgagagtctgaaccagccaagtagcgtgaaggatgactgccctatgggttgtaaacttcttttatatgggaataaagtgcagtatgtatactgttttgtatgtaccatacgaataaggatcggctaactccgtgccagcagccgcggtaatacggaggatccgagcgttatccggatttattgggtttaaagggagcgtaggcggattattaagtcagttgtgaaagtttgcggctcaaccgtaaaattgcagttgatactggtagtcttgagtgcagcagaggtaggcggaattcgtggtgtagcggtgaaatgcttagatatcacgaagaactccgattgcgaaggcagcttactggactgtaactgacgctgatgctcgaaagtgtgggtatcaaacaggattagataccctggtagtccacacagtaaacgatgaatactcgctgtttgcgatatacagcaagcggccaagcgaaagcattaagtattccacctggggagtacgccggcaacggtgaaactcaaaggaattgacgggggcccgcacaagcggaggaacatgtggtttaattcgatgatacgcgaggaaccttacccgggcttaaattgcaactgacggatttggaaacagatcttccttcgggcagttgtgaaggtgctgcatggttgtcgtcagctcgtgccgtgaggtgtcggcttaagtgccataacgagcgcaacccttatctttagttactaacaggtcatgctgaggactctagagagactgccgtcgtaagatgtgaggaaggtggggatgacgtcaaatcagcacggcccttacgtccggggctacacacgtgttacaatggggggtacagaaggcagctacacagcgatgtgatgctaatcccaaaagcctctctcagttcggattggagtctgcaacccgactccatgaagctggattcgctagtaatcgcgcatcagccacggcgcggtgaatacgttcccgggccttgtacacaccgcccgtcaagccatgaaagccgggggtacctgaagtacgtaaccgcaag

SEQ ID NO: 15 - DNA, 1391 bp, Unknown
  K15
cagtcgaacgaagcgatttaacggaagttttcggatggaagttggattgactgagtggcggacgggtgagtaacgcgtgggtaacctgccttgtactgggggacaacagttagaaatgactgctaataccgcataagcgcacagtatcgcatgatacagtgtgaaaaactccggtggtacaagatggacccgcgtctgattagctagttggtaaggtaacggcttaccaaggcgacgatcagtagccgacctgagagggtgaccggccacattgggactgagacacggcccaaactcctacgggaggcagcagtggggaatattgcacaatgggcgaaagcctgatgcagcgacgccgcgtgagtgaagaagtatttcggtatgtaaagctctatcagcagggaagaaaatgacggtacctgactaagaagccccggctaactacgtgccagcagccgcggtaatacgtagggggcaagcgttatccggatttactgggtgtaaagggagcgtagacggtaaagcaagtctgaagtgaaagcccgcggctcaactgcgggactgctttggaaactgtttaactggagtgtcggagaggtaagtggaattcctagtgtagcggtgaaatgcgtagatattaggaggaacaccagtggcgaaggcgacttactggacgataactgacgttgaggctcgaaagcgtggggagcaaacaggattagataccctggtagtccacgccgtaaacgatgaatactaggtgttggggagcaaagctcttcggtgccgtcgcaaacgcagtaagtattccacctggggagtacgttcgcaagaatgaaactcaaaggaattgacggggacccgcacaagcggtggagcatgtggtttaattcgaagcaacgcgaagaaccttaccaggtcttgacatcgatccgacgggggagtaacgtccccttcccttcggggcggagaagacaggtggtgcatggttgtcgtcagctcgtgtcgtgagatgttgggttaagtcccgcaacgagcgcaacccttattctaagtagccagcggttcggccgggaactcttgggagactgccagggataacctggaggaaggtggggatgacgtcaaatcatcatgccccttatgatctgggctacacacgtgctacaatggcgtaaacaaagagaagcaagaccgcgaggtggagcaaatctcaaaaataacgtctcagttcggactgcaggctgcaactcgcctgcacgaagctggaatcgctagtaatcgcgaatcagaatgtcgcggtgaatacgttcccgggtcttgtacacaccgcccgtcacaccatgggagtcagtaacgcccgaagtcagtgacccaaccgcaaggaggga

SEQ ID NO: 16 - DNA, 1402 bp, Unknown
  K16
agtcgaacgaagcaatactgtgtgaagagattagcttgctaagatcagaactttgtattgactgagtggcggacgggtgagtaacgcgtgggcaacctgccttacacagggggataacagctagaaatggctgctaataccgcataagacctcagtaccgcatggtagaggggtaaaaactccggtggtgtaagatgggcccgcgtctgattaggtagttggtagggtaacggcctaccaagccgacgatcagtagccgacctgagagggtgaccggccacattgggactgagacacggcccaaactcctacgggaggcagcagtggggaatattgcacaatgggggaaaccctgatgcagcgacgccgcgtgaaggatgaagtatttcggtatgtaaacttctatcagcagggaagaagatgacggtacctgactaagaagccccggctaactacgtgccagcagccgcggtaatacgtagggggcaagcgttatccggatttactgggtgtaaagggagcgtagacggcatggcaagtctgaagtgaaagcccggggctcaaccccgggactgctttggaaactgtcaggctagagtgtcggagaggcaagtggaattcctagtgtagcggtgaaatgcgtagatattaggaggaacaccagtggcgaaggcggcttgctggacgatgactgacgttgaggctcgaaagcgtggggagcaaacaggattagataccctggtagtccacgccgtaaacgatgattactaggtgtcgggaagcaaagcttttcggtgccgcagccaacgcaataagtaatccacctggggagtacgttcgcaagaatgaaactcaaaggaattgacggggacccgcacaagcggtggagcatgtggtttaattcgaagcaacgcgaagaaccttacctgatcttgacatcccggtgacaaagtatgtaatgtactctttcttcggaacaccggtgacaggtggtgcatggttgtcgtcagctcgtgtcgtgagatgttgggttaagtcccgcaacgagcgcaacccttatctttagtagccagcatttgaggtgggcactctagagagactgccagggataacctggaggaaggtggggatgacgtcaaatcatcatgccccttatgaccagggctacacacgtgctacaatggcgtaaacaaagggaagcgaccctgtgaaggcaagcaaatcccaaaaataacgtctcagttcggattgtagtctgcaactcgactacatgaagctggaatcgctagtaatcgcgaatcagaatgtcgcggtgaatacgttcccgggtcttgtacacaccgcccgtcacaccatgggagtcagtaacgcccgaagccggtgacctaaccgaaaggaagga

SEQ ID NO: 17 - DNA, 1393 bp, Unknown
  K17
  misc_feature (942)..(945): n is a, c, g, or t
  misc_feature (953)..(956): n is a, c, g, or t
  misc_feature (1067)..(1069): n is a, c, g, or t
gcaagtcgagcgaagcggtttcgatgaagttttcggatggatttgaaattgacttagcggcggacgggtgagtaacgcgtgggtaacctgccttacactgggggataacagttagaaatgactgctaataccgcataagcgcacagggccgcatggtctggtgtgaaaaactccggtggtgtaagatggacccgcgtctgattaggtagttggtggggtaacggcccaccaagccgacgatcagtagccgacctgagagggtgaccggccacattgggactgagacacggcccaaactcctacgggaggcagcagtggggaatattggacaatgggcgaaagcctgatccagcgacgccgcgtgagtgaagaagtatttcggtatgtaaagctctatcagcagggaagaaaatgacggtacctgactaagaagccccggctaactacgtgccagcagccgcggtaatacgtagggggcaagcgttatccggatttactgggtgtaaagggagcgtagacggttaagcaagtctgaagtgaaagcccggggctcaaccccggtactgctttggaaactgtttgacttgagtgcaggagaggtaagtggaattcctagtgtagcggtgaaatgcgtagatattaggaggaacaccagtggcgaaggcggcttactggactgtaactgacgttgaggctcgaaagcgtggggagcaaacaggattagataccctggtagtccacgccgtaaacgatgaatactaggtgtcgggggacaaagtccttcggtgccgccgctaacgcaataagtattccacctggggagtacgttcgcaagaatgaaactcaaaggaattgacggggacccgcacaagcggtggagcatgtggtttaattcgaagcaacgcgaagaaccttaccaagtcttgacatcccattgaaaannnnttaaccgnnnnccctcttcggagcaatggagacaggtggtgcatggttgtcgtcagctcgtgtcgtgagatgttgggttaagtcccgcaacgagcgcaacccttatccttagtagccagcannnaatggtgggcactctggggagactgccagggataacctggaggaaggtggggatgacgtcaaatcatcatgccccttatgatttgggctacacacgtgctacaatggcgtaaacaaagggaagcaaaggagcgatctggagcaaaccccaaaaataacgtctcagttcggattgcaggctgcaactcgcctgcatgaagctggaatcgctagtaatcgcgaatcagaatgtcgcggtgaatacgttcccgggtcttgtacacaccgcccgtcacaccatgggagttggtaacgcccgaagtcagtgacccaaccgcaaggaggg

SEQ ID NO: 18 - DNA, 1389 bp, Unknown
  K18
gtcgaggggcagcatggtcttagcttgctaaggctgatggcgaccggcgcacgggtgagtaacacgtatccaacctgccgtctactcttggccagccttctgaaaggaagattaatccaggatggcatcatgagttcacatgtccgcatgattaaaggtattttccggtagacgatggggatgcgttccattagatagtaggcggggtaacggcccacctagtcaacgatggataggggttctgagaggaaggtcccccacattggaactgagacacggtccaaactcctacgggaggcagcagtgaggaatattggtcaatgggcgatggcctgaaccagccaagtagcgtgaaggatgactgccctatgggttgtaaacttcttttataaaggaataaagtcgggtatgcatacccgtttgcatgtactttatgaataaggatcggctaactccgtgccagcagccgcggtaatacggaggatccgagcgttatccggatttattgggtttaaagggagcgtagatggatgtttaagtcagttgtgaaagtttgcggctcaaccgtaaaattgcagttgatactggatgtcttgagtgcagttgaggcaggcggaattcgtggtgtagcggtgaaatgcttagatatcacgaagaactccgattgcgaaggcagcctgctaagctgcaactgacattgaggctcgaaagtgtgggtatcaaacaggattagataccctggtagtccacacggtaaacgatgaatactcgctgtttgcgatatacggcaagcggccaagcgaaagcgttaagtattccacctggggagtacgccggcaacggtgaaactcaaaggaattgacgggggcccgcacaagcggaggaacatgtggtttaattcgatgatacgcgaggaaccttacccgggcttaaattgcactcgaatgatccggaaacggttcagctagcaatagcgagtgtgaaggtgctgcatggttgtcgtcagctcgtgccgtgaggtgtcggcttaagtgccataacgagcgcaacccttgttgtcagttactaacaggtgatgctgaggactctgacaagactgccatcgtaagatgtgaggaaggtggggatgacgtcaaatcagcacggcccttacgtccggggctacacacgtgttacaatggggggtacagagggccgctaccacgcgagtggatgccaatccctaaaacccctctcagttcggactggagtctgcaacccgactccacgaagctggattcgctagtaatcgcgcatcagccacggcgcggtgaatacgttcccgggccttgtacacaccgcccgtcaagccatgggagccgggggtacctgaagtgcgtaaccgcgagg

SEQ ID NO: 19 - DNA, 1393 bp, Unknown
  K19
  misc_feature (1205)..(1206): n is a, c, g, or t
gcagtcgaacgaagcaattaagatgaagttttcggatggaatcttgattgactgagtggcggacgggtgagtaacgcgtggataacctgcctcacactgggggataacagttagaaatgactgctaataccgcataagcgcacagtgccgcatggcagtgtgtgaaaaactccggtggtgtgagatggatccgcgtctgattagccagttggcggggtaacggcccaccaaagcgacgatcagtagccgacctgagagggtgaccggccacattgggactgagacacggcccaaactcctacgggaggcagcagtggggaatattgcacaatgggcgaaagcctgatgcagcgacgccgcgtgagtgaagaagtatttcggtatgtaaagctctatcagcagggaagaaaatgacggtacctgactaagaagccccggctaactacgtgccagcagccgcggtaatacgtagggggcaagcgttatccggatttactgggtgtaaagggagcgtagacggcgaagcaagtctgaagtgaaaacccagggctcaaccctgggactgctttggaaactgttttgctagagtgtcggagaggtaagtggaattcctagtgtagcggtgaaatgcgtagatattaggaggaacaccagtggcgaaggcggcttactggacgataactgacgttgaggctcgaaagcgtggggagcaaacaggattagataccctggtagtccacgccgtaaacgatgaatgctaggtgttggggggcaaagcccttcggtgccgccgcaaacgcagtaagcattccacctggggagtacgttcgcaagaatgaaactcaaaggaattgacggggacccgcacaagcggtggagcatgtggtttaattcgaagcaacgcgaagaaccttaccaagtcttgacatccccctgacgggccggtaacgcggcctttccttcgggacaggggagacaggtggtgcatggttgtcgtcagctcgtgtcgtgagatgttgggttaagtcccgcaacgagcgcaacccttatccttagtagccagcacgtgaaggtgggcactctagggagactgccagggataacctggaggaaggtggggatgacgtcaaatcatcatgccccttatgatttgggctacacacgtgctacaatggcgtaaacaaagggaagcgagacagtgatgnngagcaaatcccaaaaataacgtcccagttcggactgtagtctgcaacccgactacacgaagctggaatcgctagtaatcgcgaatcagaatgtcgcggtgaatacgttcccgggtcttgtacacaccgcccgtcacaccatgggagtcagcaacgcccgaagtcagtgacccaaccgaaaggaggga

SEQ ID NO: 20 - DNA, 1394 bp, Unknown
  K20
tgcaagtcgaacggggtgctcatgacggaggattcgtccaacggattgagttacctagtggcggacgggtgagtaacgcgtgaggaacctgccttggagaggggaataacactccgaaaggagtgctaataccgcatgatgcagttgggtcgcatggctctgactgccaaagatttatcgctctgagatggcctcgcgtctgattagctagtaggcggggtaacggcccacctaggcgacgatcagtagccggactgagaggttgaccggccacattgggactgagacacggcccagactcctacgggaggcagcagtggggaatattgggcaatgggcgcaagcctgacccagcaacgccgcgtgaaggaagaaggctttcgggttgtaaacttcttttgtcggggacgaaacaaatgacggtacccgacgaataagccacggctaactacgtgccagcagccgcggtaatacgtaggtggcaagcgttatccggatttactgggtgtaaagggcgtgtaggcgggattgcaagtcagatgtgaaaactgggggctcaacctccagcctgcatttgaaactgtagttcttgagtgctggagaggcaatcggaattccgtgtgtagcggtgaaatgcgtagatatacggaggaacaccagtggcgaaggcggattgctggacagtaactgacgctgaggcgcgaaagcgtggggagcaaacaggattagataccctggtagtccacgccgtaaacgatggatactaggtgtggggggtctgaccccctccgtgccgcagttaacacaataagtatcccacctggggagtacgatcgcaaggttgaaactcaaaggaattgacgggggcccgcacaagcggtggagtatgtggtttaattcgaagcaacgcgaagaaccttaccagggcttgacatcccactaacgaagcagagatgcattaggtgcccttcggggaaagtggagacaggtggtgcatggttgtcgtcagctcgtgtcgtgagatgttgggttaagtcccgcaacgagcgcaacccttattgttagttgctacgcaagagcactctagcgagactgccgttgacaaaacggaggaaggtggggacgacgtcaaatcatcatgccccttatgtcctgggccacacacgtactacaatggtggttaacagagggaggcaataccgcgaggtggagcaaatccctaaaagccatcccagttcggattgcaggctgaaacccgcctgtatgaagttggaatcgctagtaatcgcggatcagcatgccgcggtgaatacgttcccgggccttgtacacaccgcccgtcacaccatgagagtcgggaacacccgaagtccgtagcctaaccgcaaggaggg

SEQ ID NO: 21 - DNA, 1385 bp, Unknown
  K21
agtcgaggggcagcattttagtttgcttgcaaactaaagatggcgaccggcgcacgggtgagtaacacgtatccaacctgccgataactcggggatagcctttcgaaagaaagattaatatccgatggtatattaaaaccgcatggttttactattaaagaatttcggttatcgatggggatgcgttccattagtttgttggcggggtaacggcccaccaagactacgatggataggggttctgagaggaaggtcccccacattggaactgagacacggtccaaactcctacgggaggcagcagtgaggaatattggtcaatggacgagagtctgaaccagccaagtagcgtgaaggatgactgccctatgggttgtaaacttcttttatatgggaataaagtattccacgtgtgggattttgtatgtaccatatgaataaggatcggctaactccgtgccagcagccgcggtaatacggaggatccgagcgttatccggatttattgggtttaaagggagcgtaggtggattgttaagtcagttgtgaaagtttgcggctcaaccgtaaaattgcagttgaaactggcagtcttgagtacagtagaggtgggcggaattcgtggtgtagcggtgaaatgcttagatatcacgaagaactccgattgcgaaggcagctcactagactgcaactgacactgatgctcgaaagtgtgggtatcaaacaggattagataccctggtagtccacacagtaaacgatgaatactcgctgtttgcgatatacagtaagcggccaagcgaaagcattaagtattccacctggggagtacgccggcaacggtgaaactcaaaggaattgacgggggcccgcacaagcggaggaacatgtggtttaattcgatgatacgcgaggaaccttacccgggcttaaattgcatttgaataatctggaaacaggttagccgcaaggcaaatgtgaaggtgctgcatggttgtcgtcagctcgtgccgtgaggtgtcggcttaagtgccataacgagcgcaacccttatctttagttactaacaggtcatgctgaggactctagagagactgccgtcgtaagatgtgaggaaggtggggatgacgtcaaatcagcacggcccttacgtccggggctacacacgtgttacaatggggggtacagaaggcagctacctggcgacaggatgctaatcccaaaaacctctctcagttcggatcgaagtctgcaacccgacttcgtgaagctggattcgctagtaatcgcgcatcagccatggcgcggtgaatacgttcccgggccttgtacacaccgcccgtcaagccatgaaagccgggggtacctgaagtacgtaaccgcaa

SEQ ID NO: 22 - DNA, 1385 bp, Unknown
  K22
agtcgaggggcagcatttcagtttgcttgcaaactggagatggcgaccggcgcacgggtgagtaacacgtatccaacctgccgataactcggggatagcctttcgaaagaaagattaatacccgatggtataattagaccgcatggtcttgttattaaagaatttcggttatcgatggggatgcgttccattaggcagttggtgaggtaacggctcaccaaaccttcgatggataggggttctgagaggaaggtcccccacattggaactgagacacggtccaaactcctacgggaggcagcagtgaggaatattggtcaatgggcgcaggcctgaaccagccaagtagcgtgaaggatgactgccctatgggttgtaaacttcttttatatgggaataaagttttccacgtgtggaattttgtatgtaccatatgaataaggatcggctaactccgtgccagcagccgcggtaatacggaggatccgagcgttatccggatttattgggtttaaagggagcgtaggtggacagttaagtcagttgtgaaagtttgcggctcaaccgtaaaattgcagttgatactggctgtcttgagtacagtagaggtgggcggaattcgtggtgtagcggtgaaatgcttagatatcacgaagaactccgattgcgaaggcagctcactggactgcaactgacactgatgctcgaaagtgtgggtatcaaacaggattagataccctggtagtccacacagtaaacgatgaatactcgctgtttgcgatatacagtaagcggccaagcgaaagcattaagtattccacctggggagtacgccggcaacggtgaaactcaaaggaattgacgggggcccgcacaagcggaggaacatgtggtttaattcgatgatacgcgaggaaccttacccgggcttaaattgcatttgaatatattggaaacagtatagccgtaaggcaaatgtgaaggtgctgcatggttgtcgtcagctcgtgccgtgaggtgtcggcttaagtgccataacgagcgcaacccttatctttagttactaacaggtcatgctgaggactctagagagactgccgtcgtaagatgtgaggaaggtggggatgacgtcaaatcagcacggcccttacgtccggggctacacacgtgttacaatggggggtacagaaggcagctacctggtgacaggatgctaatcccaaaagcctctctcagttcggatcgaagtctgcaacccgacttcgtgaagctggattcgctagtaatcgcgcatcagccatggcgcggtgaatacgttcccgggccttgtacacaccgcccgtcaagccatgaaagccgggggtacctgaagtacgtaaccgcaa

SEQ ID NO: 23 - DNA, 1387 bp, Unknown
  K23
agtcgaggggcagcatgatttgtagcaatacagattgatggcgaccggcgcacgggtgagtaacgcgtatgcaacttacctatcagagggggatagcccggcgaaagtcggattaataccccataaaacaggggtcccgcatgggaatatttgttaaagattcatcgctgatagataggcatgcgttccattaggcagttggcggggtaacggcccaccaaaccgacgatggataggggttctgagaggaaggtcccccacattggtactgagacacggaccaaactcctacgggaggcagcagtgaggaatattggtcaatggccgagaggctgaaccagccaagtcgcgtgaaggaagaaggatctatggtttgtaaacttcttttataggggaataaagtggaggacgtgtccttttttgtatgtaccctatgaataagcatcggctaactccgtgccagcagccgcggtaatacggaggatgcgagcgttatccggatttattgggtttaaagggtgcgtaggtggtgatttaagtcagcggtgaaagtttgtggctcaaccataaaattgccgttgaaactgggttacttgagtgtgtttgaggtaggcggaatgcgtggtgtagcggtgaaatgcatagatatcacgcagaactccgattgcgaaggcagcttactaaaccataactgacactgaagcacgaaagcgtggggatcaaacaggattagataccctggtagtccacgcagtaaacgatgattactaggagtttgcgatacaatgtaagctctacagcgaaagcgttaagtaatccacctggggagtacgccggcaacggtgaaactcaaaggaattgacgggggcccgcacagcggaggaacatgtggtttaattcgatgatacgcgaggaaccttacccgggtttgaacgtagtctgaccggagtggaaacactctttctagcaatagcagattacgaggtgctgcatggttgtcgtcagctcgtgccgtgaggtgtcggcttaagtgccataacgagcgcaacccttatcactagttactaacaggtgaagctgaggactctggtgagactgccagcgtaagctgtgaggaaggtggggatgacgtcaaatcagcacggcccttacatccggggcgacacacgtgttacaatggcatggacaaagggcagctacctggtgacaggatgctaatctccaaaccatgtctcagttcggatcggagtctgcaactcgactccgtgaagctggattcgctagtaatcgcgcatcagccatggcgcggtgaatacgttcccgggccttgtacacaccgcccgtcaagccatgggagccgggggtacctgaagtccgtaaccgcaag

SEQ ID NO: 24 - DNA, 1384 bp, Unknown
  K24
gtcgaggggcagcatggtcttagcttgctaaggccgatggcgaccggcgcacgggtgagtaacacgtatccaacctgccgtctactcttggacagccttctgaaaggaagattaatacaagatggcatcatgagtccgcatgttcacatgattaaaggtattccggtagacgatggggatgcgttccattagatagtaggcggggtaacggcccacctagtcttcgatggataggggttctgagaggaaggtcccccacattggaactgagacacggtccaaactcctacgggaggcagcagtgaggaatattggtcaatgggcgagagcctgaaccagccaagtagcgtgaaggatgactgccctatgggttgtaaacttcttttataaaggaataaagtcgggtatggatacccgtttgcatgtactttatgaataaggatcggctaactccgtgccagcagccgcggtaatacggaggatccgagcgttatccggatttattgggtttaaagggagcgtagatggatgtttaagtcagttgtgaaagtttgcggctcaaccgtaaaattgcagttgatactggatatcttgagtgcagttgaggcaggcggaattcgtggtgtagcggtgaaatgcttagatatcacgaagaactccgattgcgaaggcagcctgctaagctgcaactgacattgaggctcgaaagtgtgggtatcaaacaggattagataccctggtagtccacacggtaaacgatgaatactcgctgtttgcgatatactgcaagcggccaagcgaaagcgttaagtattccacctggggagtacgccggcaacggtgaaactcaaaggaattgacgggggcccgcacaagcggaggaacatgtggtttaattcgatgatacgcgaggaaccttacccgggcttaaattgcagatgaattacggtgaaagccgtaagccgcaaggcatctgtgaaggtgctgcatggttgtcgtcagctcgtgccgtgaggtgtcggcttaagtgccataacgagcgcaacccttgttgtcagttactaacaggttccgctgaggactctgacaagactgccatcgtaagatgtgaggaaggtggggatgacgtcaaatcagcacggcccttacgtccggggctacacacgtgttacaatggggggtacagagggccgctaccacgcgagtggatgccaatccccaaaacctctctcagttcggactggagtctgcaacccgactccacgaagctggattcgctagtaatcgcgcatcagccacggcgcggtgaatacgttcccgggccttgtacacaccgcccgtcaagccatgggagccgggggtacctgaagtgcgtaaccgcgag

SEQ ID NO: 25 - DNA, 1396 bp, Unknown
  K25
  misc_feature (943)..(944): n is a, c, g, or t
  misc_feature (1072)..(1072): n is a, c, g, or t
  misc_feature (1290)..(1290): n is a, c, g, or t
gcagtcgaacgaagcgatctgggatgaagttttcggatggattcctggttgactgagtggcggacgggtgagtaacgcgtggataacctgcctcacactgggggataacagttagaaatggctgctaataccgcataagcgcacagtaccgcatggtacggtgtgaaaaacccaggtggtgtgagatggatccgcgtctgattagccagttggcggggtaacggcccaccaaagcgacgatcagtagccgacctgagagggtgaccggccacattgggactgagacacggcccaaactcctacgggaggcagcagtggggaatattgcacaatgggcgaaagcctgatgcagcgacgccgcgtgagtgaagaagtatctcggtatgtaaagctctatcagcagggaagaaaatgacggtacctgactaagaagccccggctaactacgtgccagcagccgcggtaatacgtagggggcaagcgttatccggatttactgggtgtaaagggagcgtagacggcgacgcaagtctggagtgaaagcccggggcccaaccccgggactgctttggaaactgtgctgctggagtgcaggagaggtaagtggaattcctagtgtagcggtgaaatgcgtagatattaggaggaacaccagtggcgaaggcggcttactggactgtaactgacgttgaggctcgaaagcgtggggagcaaacaggattagataccctggtagtccacgccgtaaacgatgaatgctaggtgtcggggggcaaagcccttcggtgccgccgctaacgcaataagcattccacctggggagtacgttcgcaagaatgaaactcaaaggaattgacggggacccgcacaagcggtggagcatgtggtttaattcgaagcaacgcgaagaaccttaccaagtcttgacatccccctgaccggnncgtaacggtgcccttccttcgggacaggggagacaggtggtgcatggttgtcgtcagctcgtgtcgtgagatgttgggttaagtcccgcaacgagcgcaacccttatccttagtagccagcacgtganggtgggcactctagggagactgccagggataacctggaggaaggtggggatgacgtcaaatcatcatgccccttatgatttgggctacacacgtgctacaatggcgtaaacaaagggaggcgaccctgcgaaggcaagcaaatcccaaaaataacgtcccagttcggactgtagtctgcaacccgactacacgaagctggaatcgctagtaatcgcgnatcagaatgccgcggtgaatacgttcccgggtcttgtacacaccgcccgtcacaccatgggagtcagcaacgcccgaagtcagtgacccaaccttaacaggaggga

SEQ ID NO: 26 - DNA, 1382 bp, Unknown
  K26
gtcgaggggcatcaggaagaaagcttgctttctttgctggcgaccggcgcacgggtgagtaacacgtatccaacctgccgatgactcggggatagcctttcgaaagaaagattaatacccgatggtatatctgaaaggcatctttcagctattaaagaatttcggtcattgatggggatgcgttccattaggttgttggcggggtaacggcccaccaagccgtcgatggataggggttctgagaggaaggtcccccacattggaactgagacacggtccaaactcctacgggaggcagcagtgaggaatattggtcaatggacgagagtctgaaccagccaagtagcgtgaaggatgactgccctatgggttgtaaacttcttttatacgggaataaagttaggcacgtgtgcctttttgtatgtaccgtatgaataaggatcggctaactccgtgccagcagccgcggtaatacggaggatccgagcgttatccggatttattgggtttaaagggagcgtaggcggatgcttaagtcagttgtgaaagtttgcggctcaaccgtaaaattgcagttgatactgggtgtcttgagtacagtagaggcaggcggaattcgtggtgtagcggtgaaatgcttagatatcacgaagaactccgattgcgaaggcagcttgctggactgtaactgacgctgatgctcgaaagtgtgggtatcaaacaggattagataccctggtagtccacacagtaaacgatgaatactcgctgtttgcgatatacagtaagcggccaagcgaaagcgttaagtattccacctggggagtacgccggcaacggtgaaactcaaaggaattgacgggggcccgcacaagcggaggaacatgtggtttaattcgatgatacgcgaggaaccttacccgggcttaaattgcaaatgaatgttctggaaacagatcagccgcaaggcatttgtgaaggtgctgcatggttgtcgtcagctcgtgccgtgaggtgtcggcttaagtgccataacgagcgcaacccttatcgatagttaccatcaggttatgctggggactctgtcgagactgccgtcgtaagatgtgaggaaggtggggatgacgtcaaatcagcacggcccttacgtccggggctacacacgtgttacaatggggggtacagaaggcagctacacggtgacgtgatgctaatccctaaaacctctctcagttcggattggagtctgcaacccgactccatgaagctggattcgctagtaatcgcgcatcagccacggcgcggtgaatacgttcccgggccttgtacacaccgcccgtcaagccatgaaagccgggggtacctgaagtgcgtaaccgcga

SEQ ID NO: 27 - DNA, 1370 bp, Unknown
  K27
  misc_feature (916)..(917): n is a, c, g, or t
tgcaagtcgaacggttaaggcgccttcgggcgcgaatagagtggcgaacgggtgagtaacacgtgaccaacctgcccccctccccgggataacgcgaggaaacccgcgctaataccggatactccgcccctcccgcatgggaggggcgggaaagccccgacggagggggatggggtcgcggcccattaggtagacggcggggcaacggcccaccgtgcctgcgatgggtagccgggttgagagaccgaccggccacattgggactgagatacggcccagactcctacgggaggcagcagtggggaattttgcgcaatggggggaaccctgacgcagcaacgccgcgtgcgggacgaaggccttcgggttgtaaaccgctttcagcagggaagaagttgacggtacctgcagaagaagccccggctaactacgtgccagcagccgcggtaatacgtagggggcgagcgttatccggattcattgggcgtaaagcgcgcgtaggcggcccgtcaagcggaacctctaacccgagggctcaacccccggtcgggttccgaactggcaggctcgagtttggtagaggaagatggaattcccggtgtagcggtggaatgcgcagatatcgggaagaacaccgatggcgaaggcagtcttctgggccatcaactgacgctgaggcgcgaaagctgggggagcgaacaggattagataccctggtagtcccagccgtaaacgatgggcgctaggtgtggggggatcatccctccgtgccgcagccaacgcattaagcgccccgcctggggagtacggccgcaaggctaaaactcaaaggaattgacgggggcccgcacaagcagcggagcatgtggcttaattcgaagcaacgcgaagaaccttaccagggcttgacatgctnntgaagccggggaaacccggtggccgagaggagccagcgcaggtggtgcatggctgtcgtcagctcgtgtcgtgagatgttgggttaagtcccgcaacgagcgcaacccctgccatatgttgccagcattcagttggggactcatatgggactgccggcgtcaagccggaggaaggtggggacgacgtcaagtcatcatgccctttatgccctgggctgcacacgtgctacaatggccggtacaacgggccgcgacctggcgacaggaagcgaatccctcaaagccggccccagttcggatcggaggctgcaacccgcctccgtgaagtcggagttgctagtaatcgcggatcagcatgccgcggtgaatacgttcccgggccttgtacacaccgcccgtcacaccacccgagtcgtctgcacccgaagccgccggccgaacccgcaaggggcg

SEQ ID NO: 28 - DNA, 1394 bp, Unknown
  K28
  misc_feature (909)..(911): n is a, c, g, or t
caagtcgaacgaagcacttacttccaaatcttcggaagaggaggtatttgactgagtggcggacgggtgagtaacgcgtggggaacctgccccgtaccgggggataacagtcagaaatgactgctaataccgcataagcgcacgaaggcgcatgcttttgtgtgaaaaactccggtggtacgggatggtcccgcgtctgattagccagttggcggggtaacggcccaccaaagcgacgatcagtagccggcctgagagggtggacggccacattgggactgagacacggcccagactcctacgggaggcagcagtggggaatattgcacaatgggggaaaccctgatgcagcgacgccgcgtgagcgaagaagtatttcggtatgtaaagctctgtcagcagggaagaaaatgacggtacctgaccaagaagcaccggctaaatacgtgccagcagccgcggtaatacgtatggtgcaagcgttatccggatttactgggtgtaaagggagcgtagacggaggggcaagtctgaagtgaaagcccggggcccaaccccgggactgctttggaaactgtccgtctggagtgccggagaggtaagcggaattcccagtgtagcggtgaaatgcgtagatattgggaggaacaccagtggcgaaggcggcttactggacggtcactgacgttgaggctcgaaagcgtggggagcaaacaggattagataccctggtagtccacgccgtaaacgatgactactaggtgtcgggtggcagagccattcggtgccgcagccaacgcagtaagtagtccacctggggagtacgttcgcaagaatgaaactcaaaggaattgacggggacccgcacaagcggtggagcatgtggtttaattcgaagcaacgcgaagnnncttacctggccttgacatccccctgaccggcgcgtaatggtgcctttccttcgggacaggggagacaggtggtgcatggttgtcgtcagctcgtgtcgtgagatgttgggttaagtcccgcaacgagcgcaacccttatcttcagtagccagcattcaggatgggcactctggagagactgccagggacaacctggaggaaggtggggatgacgtcaaatcatcatgccccttatggccagggctacacacgtgctacaatggcgtaaacagagggaagcgagcccgcgagggggagcaaatcccaaaaataacgtcccagttcggactgcaggctgcaacccgcctgcacgaagctggaatcgctagtaatcgcgaatcagcatgtcgcggtgaatacgttcccgggtcttgtacacaccgcccgtcacaccatgggagtcggtaacgcccgaagtcagtgacccaacctccgggagggagc

SEQ ID NO: 29 - DNA, 1387 bp, Unknown
  K29
  misc_feature (895)..(896): n is a, c, g, or t
  misc_feature (910)..(912): n is a, c, g, or t
  misc_feature (942)..(946): n is a, c, g, or t
  misc_feature (953)..(954): n is a, c, g, or t
agtcgaacgaagcatttaggattgaagttttcggatggatttcctttatgactgagtggcggacgggtgagtaacgcgtggggaacctgccctatacagggggataacagctggaaacggctgctaataccgcataagcgcacagaatcgcatgattcagtgtgaaaagccctggcagtataggatggtcccgcgtctgattagctggttggtgaggtaacggctcaccaaggcgacgatcagtagccggcttgagagagtgaacggccacattgggactgagacacggcccaaactcctacgggaggcagcagtggggaatattgcacaatgggggaaaccctgatgcagcgacgccgcgtgagtgaagaagtatttcggtatgtaaagctctatcagcagggaagaaaacagacggtacctgactaagaagccccggctaactacgtgccagcagccgcggtaatacgtagggggcaagcgttatccggaattactgggtgtaaagggtgcgtaggtggcatggtaagtcagaagtgaaagcccggggcttaaccccgggactgcttttgaaactgtcatgctggagtgcaggagaggtaagcggaattcctagtgtagcggtgaaatgcgtagatattaggaggaacaccagtggcgaaggcggcttactggactgtcactgacactgatgcacgaaagcgtggggagcaaacaggattagataccctggtagtccacgccgtaaacgatgaatactaggtgtcggggccgtagaggcttcggtgccgcagcaaacgcagtaagtattccacctggggagtacgttcgcaagaatgaaactcaaaggaattgacggggacccgcacaagcggtggagcatgtggtttaattnnaagcaacgcgaagnnncttacctggtcttgacatcccaatgaccgnnnnntaaccgnntttttctttcgagacattggagacaggtggtgcatggttgtcgtcagctcgtgtcgtgagatgttgggttaagtcccgcaacgagcgcaacccctatctttagtagccagcattagaggtgggcactctagagagactgccagggataacctggaggaaggtggggaggacgtcaaatcatcatgccccttatggccagggctacacacgtgctacaatggcgtaaacaaagggaagcgaagtcgtgaggcgaagcaaatcccagaaataacgtctcagttcggattgtagtctgcaactcgactacatgaagctggaatcgctagtaatcgtgaatcagaatgtcacggtgaatacgttcccgggtcttgtacacaccgcccgtcacaccatgggagtcagtaacgcccgaagtcagtgacccaaccgcaag

SEQ ID NO: 30 - DNA, 1392 bp, Unknown
  K30
gcaagtcgagcgaagcaccttgacggatttcttcggattgaagccttggtgactgagcggcggacgggtgagtaacgcgtgggtaacctgcctcatacagggggataacagttggaaacggctgctaataccgcataagcgcacagtaccgcatggtacggtgtgaaaaactccggtggtatgagatggacccgcgtctgattaggtagttggtggggtaacggcctaccaagccgacgatcagtagccgacctgagagggtgaccggccacattgggactgagacacggcccaaactcctacgggaggcagcagtggggaatattgcacaatgggggaaaccctgatgcagcgacgccgcgtgagcgatgaagtatttcggtatgtaaagctctatcagcagggaagaaaatgacggtacctgactaagaagccccggctaactacgtgccagcagccgcggtaatacgtagggggcaagcgttatccggatttactgggtgtaaagggagcgtagacggcatggcaagccagatgtgaaagcccggggctcaaccccgggactgcatttggaactgtcaggctagagtgtcggagaggaaagcggaattcctagtgtagcggtgaaatgcgtagatattaggaggaacaccagtggcgaaggcggctttctggacgatgactgacgttgaggctcgaaagcgtggggagcaaacaggattagataccctggtagtccacgccgtaaacgatgaatactaggtgtcgggtggcaaagccattcggtgccgcagcaaacgcaataagtattccacctggggagtacgttcgcaagaatgaaactcaaaggaattgacggggacccgcacaagcggtggagcatgtggtttaattcgaagcaacgcgaagaaccttacctggtcttgacatccctctgaccgctctttaatcggagctttccttcgggacagaggagacaggtggtgcatggttgtcgtcagctcgtgtcgtgagatgttgggttaagtcccgcaacgagcgcaacccctatctttagtagccagcattttggatgggcactctagagagactgccagggataacctggaggaaggtggggatgacgtcaaatcatcatgccccttatgaccagggctacacacgtgctacaatggcgtaaacaaagggaagcgagcccgcgagggggagcaaatcccaaaaataacgtctcagttcggattgtagtctgcaactcgactacatgaagctggaatcgctagtaatcgcgaatcagaatgtcgcggtgaatacgttcccgggtcttgtacacaccgcccgtcacaccatgggagtcagtaacgcccgaagtcagtgacccaaccgcaaggaggg

SEQ ID NO: 31 - DNA, 1394 bp, Unknown
  K31
  misc_feature (1073)..(1074): n is a, c, g, or t
cagtcgagcgaagcgctttgtgcggatttcttcggattgaagcaactgtgactgagcggcggacgggtgagtaacgcgtgggtaacctgcctcatacagggggataacagttggaaacggctgctaataccgcataagcgcacagtaccgcatggtacggtgtgaaaaactccggtggtatgagatggacccgcgtctgattaggtagttggtggggtaacggcctaccaaggcgacgatcagtagccgacctgagagggtgaccggccacattgggactgagacacggcccaaactcctacgggaggcagcagtggggaatattgcacaatgggggaaaccctgatgcagcgacgccgcgtgagcgatgaagtatttcggtatgtaaagctctatcagcagggaagaaaatgacggtacctgactaagaagccccggctaactacgtgccagcagccgcggtaatacgtagggggcaagcgttatccggatttactgggtgtaaagggagcgtagacggcatggcaagccagatgtgaaagcccggggctcaaccccgggactgcatttggaactgtcaggctagagtgtcggagaggaaagcggaattcctagtgtagcggtgaaatgcgtagatattaggaggaacaccagtggcgaaggcggctttctggacgatgactgacgttgaggctcgaaagcgtggggagcaaacaggattagataccctggtagtccacgccgtaaacgatgaatactaggtgtcgggtggcaaagccattcggtgccgcagcaaacgcaataagtattccacctgggggagtacgttcgcaagaatgaaactcaaaggaattgacggggacccgcacaagcggtggagcatgtggtttaattcgaagcaacgcgaagaaccttacctggtcttgacatccctctgaccgctctttaatcggagctttctttcgggacagaggagacaggtggtgcatggttgtcgtcagctcgtgtcgtgagatgttgggttaagtcccgcaacgagcgcaacccctatctttagtagccagcatttaagnngggcactctagagagactgccagggataacctggaggaaggtggggatgacgtcaaatcatcatgccccttatgaccagggctacacacgtgctacaatggcgtaaacaaagggaagcgagcccgcgagggggagcaaatcccaaaaataacgtctcagttcggattgtagtctgcaactcgactacatgaagctggaatcgctagtaatcgcgaatcagaatgtcgcggtgaatacgttcccgggtcttgtacacaccgcccgtcacaccatgggagtcagtaacgcccgaagtcagtgacccaaccgcaaggagggag

SEQ ID NO: 32 - DNA, 1383 bp, Unknown
  K32
aagtcgaggggcagcacggtgtagcaatacactggtggcgaccggcgcacgggtgcgtaacgcgtatgcaacctacccataacagggggataacactgagaaattggtactaataccccataacatcaggaccggcatcggttctggttgaaaactccggtggttatggatgggcatgcgttgtattagctggttggtgaggtaacggctcaccaaggcaacgatacatagggggactgagaggttaaccccccacattggtactgagacacggaccaaactcctacgggaggcagcagtgaggaatattggtcaatggacgcaagtctgaaccagccatgccgcgtgcaggaagacggctctatgagttgtaaactgcttttgtacgagggtaaacgctcttacgtgtaagagcctgaaagtatcgtacgaataaggatcggctaactccgtgccagcagccgcggtaatacggaggatccaagcgttatccggatttattgggtttaaagggtgcgtaggcggtttgataagttagaggtgaaataccggtgcttaacaccggaactgcctctaatactgttgaactagagagtagttgcggtaggcggaatgtatggtgtagcggtgaaatgcttagagatcatacagaacaccgattgcgaaggcagcttaccaaactatatctgacgttgaggcacgaaagcgtggggagcaaacaggattagataccctggtagtccacgcagtaaacgatgataactcgctgtcggcgatacacagtcggcggctaagcgaaagcgataagttatccacctggggagtacgttcgcaagaatgaaactcaaaggaattgacgggggcccgcacaagcggaggaacatgtggtttaattcgatgatacgcgaggaaccttacccgggcttgaaagttactgacgattctggaaacaggatttcccttcggggcaggaaactaggtgctgcatggttgtcgtcagctcgtgccgtgaggtgtcgggttaagtcccataacgagcgcaacccctaccgttagttgccatcaggtcaagctgggcactctggcgggactgccggtgtaagccgagaggaaggtggggatgacgtcaaatcagcacggcccttacgtccggggctacacacgtgttacaatggtaggtacagagggcagctacccagtgatgggatgcgaatctcgaaagcctatctcagttcggatcggaggctgaaacccgcctccgtgaagttggattcgctagtaatcgcgcatcagccatggcgcggtgaatacgttcccgggccttgtacacaccgcccgtcaagccatggaagctgggggtgcctgaagttcgtgaccgcaagg

SEQ ID NO: 33 - DNA, 1378 bp, Unknown
  K33
gaggggcagcatcattaaagcttgctttgatggatggcgaccggcgcacgggtgagtaacacgtatccaacctgccgacaacactgggatagcctttcgaaagaaagattaataccggatggcatagttttcccgcatgggataattattaaagaatttcggttgtcgatggggatgcgttccattaggcagttggcggggtaacggcccaccaaaccaacgatggataggggttctgagaggaaggtcccccacattggaactgagacacggtccaaactcctacgggaggcagcagtgaggaatattggtcaatggacgagagtctgaaccagccaagtagcgtgaaggatgactgccctatgggttgtaaacttcttttatacgggaataaagttagccacgtgtggctttttgtatgtaccgtatgaataaggatcggctaactccgtgccagcagccgcggtaatacggaggatccgagcgttatccggatttattgggtttaaagggagcgtaggcgggttgttaagtcagttgtgaaagtttgcggctcaaccgtaaaattgcagttgatactggcgaccttgagtgcaacagaggtaggcggaattcgtggtgtagcggtgaaatgcttagatatcacgaagaactccgattgcgaaggcagcttactggattgtaactgacgctgatgctcgaaagtgtgggtatcaaacaggattagataccctggtagtccacacagtaaacgatgaatactcgctgttggcgatatacggtcagcggccaagcgaaagcattaagtattccacctggggagtacgccggcaacggtgaaactcaaaggaattgacgggggcccgcacaagcggaggaacatgtggtttaattcgatgatacgcgaggaaccttacccgggcttaaattgcaactgactgaaccggaaacggttctttcttcggacagttgtgaaggtgctgcatggttgtcgtcagctcgtgccgtgaggtgtcggcttaagtgccataacgagcgcaacccttatcgatagttactagcaggtcatgctgaggactctattgagactgccgtcgtaagatgtgaggaaggtggggatgacgtcaaatcagcacggcccttacgtccggggctacacacgtgttacaatggggggtacagaaggcagctacacggcgacgtggtgctaatcccgaaagcctctctcagttcggattggagtctgcaacccgactccatgaagctggattcgctagtaatcgcgcatcagccacggcgcggtgaatacgttcccgggccttgtacacaccgcccgtcaagccatgaaagccgggggtacctgaagtacgtaaccgcg

SEQ ID NO: 34 - DNA, 1394 bp, Unknown
  K34
cagtcgagcgaagcacttaagtggatctcttcggattgaaacttattgtgactgagcggcggacgggtgagtaacgcgtgggtaacctgcctcatacagggggataacagttagaaatggctgctaataccgcataagcgcacaggaccgcatggtctggtgtgaaaaactccggtggtatgagatggacccgcgtctgattagctagttggaggggtaacggcccaccaaggcgacgatcagtagccggcctgagagggtgaacggccacattgggactgagacacggcccagactcctacgggaggcagcagtggggaatattgcacaatgggggaaaccctgatgcagcgacgccgcgtgaaggaagaagtatctcggtatgtaaacttctatcagcagggaagaaaatgacggtacctgactaagaagccccggctaactacgtgccagcagccgcggtaatacgtagggggcaagcgttatccggatttactgggtgtaaagggagcgtagacggaagagcaagtctgatgtgaaaggctggggcttaaccccaggactgcattggaaactgtttttctagagtgccggagaggtaagcggaattcctagtgtagcggtgaaatgcgtagatattaggaggaacaccagtggcgaaggcggcttactggacggtaactgacgttgaggctcgaaagcgtggggagcaaacaggattagataccctggtagtccacgccgtaaacgatgaatactaggtgtcgggtggcaaagccattcggtgccgcagcaaacgcaataagtattccacctggggagtacgttcgcaagaatgaaactcaaaggaattgacggggacccgcacaagcggtggagcatgtggtttaattcgaagcaacgcgaagaaccttaccaagtcttgacatccctctgaccggcccgtaacggggccttcccttcggggcagaggagacaggtggtgcatggttgtcgtcagctcgtgtcgtgagatgttgggttaagtcccgcaacgagcgcaacccctatccttagtagccagcaggtgaagctgggcactctagggagactgccggggataacccggaggaaggcggggacgacgtcaaatcatcatgccccttatgatttgggctacacacgtgctacaatggcgtaaacaaagggaagcgagacagcgatgttgagcaaatcccaaaaataacgtcccagttcggactgcagtctgcaactcgactgcacgaagctggaatcgctagtaatcgcgaatcagaatgtcgcggtgaatacgttcccgggtcttgtacacaccgcccgtcacaccatgggagtcagtaacgcccgaagtcagtgacccaaccttacaggaggga

SEQ ID NO: 35 - DNA, 1392 bp, Unknown
  K35
  misc_feature (901)..(901): n is a, c, g, or t
cagtcgaacggagctcagttttggaaactttcttcgggagtggaattctcgacttagtggcggacgggtgagtaacgcgtgagcaatctgcctttaagagggggataacagtcggaaacggctgctaataccgcataaagcattgaattcgcatgttttcgatgccaaaggagcaatccgcttttagatgagctcgcgtctgattagctagttggcggggtaacggcccaccaaggcgacgatcagtagccggactgagaggttgaacggccacattgggactgagacacggcccagactcctacgggaggcagcagtggggaatattgcgcaatgggggaaaccctgacgcagcaacgccgcgtgattgaagaaggccttcgggttgtaaagatctttaatcagggacgaaacaaatgacggtacctgaagaataagctccggctaactacgtgccagcagccgcggtaatacgtagggagcaagcgttatccggatttactgggtgtaaagggcgcgcaggcgggccggcaagttggaagtgaaatctatgggcttaacccataaactgctttcaaaactgctggtcttgagtgatggagaggcaggcggaattccgtgtgtagcggtgaaatgcgtagatatacggaggaacaccagtggcgaaggcggcctgctggacattaactgacgctgaggcgcgaaagcgtggggagcaaacaggattagataccctggtagtccacgccgtaaacgatggatactaggtgtgggaggtattgaccccttccgtgccgcagttaacacaataagtatcccacctggggagtacggccgcaaggttgaaactcaaaggaattgacgggggcccgcacaagcagtggagtatgtggtttaattngaagcaacgcgaagaaccttaccaggtcttgacatcccgatgaccgccttagagataaggctttttttcggaacatcggtgacaggtggtgcatggttgtcgtcagctcgtgtcgtgagatgttgggttaagtcccgcaacgagcgcaacccttacggttagttgatacgcaagatcactctagccggactgccgttgacaaaacggaggaaggtggggacgacgtcaaatcatcatgccccttatgacctgggctacacacgtactacaatggcagtcatacagagggaagcaaaaccgcgaggtggagcaaatccctaaaagctgtcccagttcagattgcaggctgcaacccgcctgcatgaagtcggaattgctagtaatcgcggatcagcatgccgcggtgaatacgttcccgggccttgtacacaccgcccgtcacaccatgagagccgtcaatacccgaagtccgtagcctaaccttcttggag

SEQ ID NO: 36 - DNA, 1394 bp, Unknown
  K36
  misc_feature (1068)..(1069): n is a, c, g, or t
agtcgaacgaagcaattaaaatgaagttttcggatggatttttgattgactgagtggcggacgggtgagtaacgcgtggataacctgcctcacactgggggataacagttagaaatgactgctaataccgcataagcgcacagtaccgcatggtacggtgtgaaaaactccggtggtgtgagatggatccgcgtctgattagccagttggcggggtaacggcccaccaaagcgacgatcagtagccgacctgagagggtgaccggccacattgggactgagacacggcccaaactcctacgggaggcagcagtggggaatattgcacaatgggcgaaagcctgatgcagcgacgccgcgtgagtgaagaagtatttcggtatgtaaagctctatcagcagggaagaaaatgacggtacctgactaagaagccccggctaactacgtgccagcagccgcggtaatacgtagggggcaagcgttatccggatttactgggtgtaaagggagcgtagacggcgaagcaagtctgaagtgaaaacccagggctcaaccctgggactgctttggaaactgttttgctagagtgtcggagaggtaagtggaattcctagtgtagcggtgaaatgcgtagatattaggaggaacaccagtggcgaaggcggcttactggacgataactgacgttgaggctcgaaagcgtggggagcaaacaggattagataccctggtagtccacgccgtaaacgatgaatgctaggtgttggggggcaaagcccttcggtgccgtcgcaaacgcagtaagcattccacctggggagtacgttcgcaagaatgaaactcaaaggaattgacggggacccgcacaagcggtggagcatgtggtttaattcgaagcaacgcgaagaaccttaccaagtcttgacatcctcttgaccggcgtgtaacggcgccttcccttcggggcaagagagacaggtggtgcatggttgtcgtcagctcgtgtcgtgagatgttgggttaagtcccgcaacgagcgcaacccttatccttagtagccagcaggtanngctgggcactctagggagactgccagggataacctggaggaaggtggggatgacgtcaaatcatcatgccccttatgatttgggctacacacgtgctacaatggcgtaaacaaagggaagcaagacagtgatgtggagcaaatcccaaaaataacgtcccagttcggactgtagtctgcaacccgactacacgaagctggaatcgctagtaatcgcgaatcagaatgtcgcggtgaatacgttcccgggtcttgtacacaccgcccgtcacaccatgggagtcagcaacgcccgaagtcagtgacccaactcgcaagagagggag

SEQ ID NO: 37 - DNA, 1371 bp, Unknown
  K37
cagtcgaacgagccgaggggagcttgctccccagagctagtggcggacgggtgagtaacacgtgagcaacctgcctttcagagggggataacgtttggaaacgaacgctaataccgcataacataccgggaccgcatgattctggtatcaaaggagcaatccgctgaaagatgggctcgcgtccgattagctagttggcggggtaacggcccaccaaggcgacgatcggtagccggactgagaggttgatcggccacattgggactgagacacggcccagactcctacgggaggcagcagtgggggatattgcacaatggaggaaactctgatgcagcgacgccgcgtgagggaagacggtcttcggattgtaaacctctgtctttggggacgataatgacggtacccaaggaggaagctccggctaactacgtgccagcagccgcggtaatacgtagggagcgagcgttgtccggaattactgggtgtaaagggagcgtaggcggggtctcaagtcgaatgttaaatctaccggctcaactggtagctgcgttcgaaactggggctcttgagtgaagtagaggcaggcggaattcctagtgtagcggtgaaatgcgtagatattaggaggaacaccagtggcgaaggcggcctgctgggcttttactgacgctgaggctcgaaagcgtggggagcaaacaggattagataccctggtagtccacgccgtaaacgatgattactaggtgtggggggactgaccccttccgtgccggagttaacacaataagtaatccacctggggagtacgaccgcaaggttgaaactcaaaggaattgacgggggcccgcacaagcagtggattatgtggtttaattcgaagcaacgcgaagaaccttaccaggtcttgacatcgagtgacggctctagagatagagctttccttcgggacacaaagacaggtggtgcatggttgtcgtcagctcgtgtcgtgagatgttgggttaagtcccgcaacgagcgcaacccttattattagttgctacattcagttgagcactctaatgagactgccgttgacaaaacggaggaaggtggggatgacgtcaaatcatcatgccccttatgacctgggctacacacgtaatacaatggcgatcaacagagggaagcaagaccgcgaggtggagcaaacccctaaaagtcgtctcagttcggattgcaggctgcaactcgcctgcatgaagtcggaattgctagtaatcgcggatcagcatgccgcggtgaatacgttcccgggccttgtacacaccgcccgtcacaccatgggagtcggtaacacccgaagtcagtagcctaaccgcaaggagg

SEQ ID NO: 38 - DNA, 1396 bp, Unknown
  K38
tgcagtcgaacgctttgtaaaggagcttgcttctttacgaggagtggcgaacgggtgagtaatacataagcaatctgcccatcggcctgggataacagttggaaacgactgctaataccggataggttagtttctggcatcagggactaattaaagttgggatacaacacggatggatgagcttatggcgtattagctagtaggtgaggtaacggcccacctaggcgatgatacgtagccgacctgagagggtgaccggccacattgggactgagacacggcccaaactcctacgggaggcagcagtagggaattttcggcaatgggcgaaagcctgaccgagcaacgccgcgtgagtgaagaaggccttcgggttgtaaagctctgttgtgaaggaagaacggctcatagagggaatgctatgggagtgacggtactttaccagaaagccacggctaactacgtgccagcagccgcggtaatacgtaggtggcgagcgttatccggaattattgggcgtaaagggtgcgcaggcggtttgaaaagtttaaggtgaaagcgtggggcttaaccccatacagccttagaaactgtcagactagagtacaggagagggcaatggaattccatgtgtagcggtaaaatgcgtagatatatggaggaacaccagtggcgaaggcggttgcctggcctgtaactgacgctcatgcacgaaagcgtggggagcaaataggattagataccctagtagtccacgccgtaaacgatgagaactaagtgttggggaaactcagtgctgcagttaacgcaataagttctccgcctggggagtatgcacgcaagtgtgaaactcaaaggaattgacgggggcccgcacaagcggtggagtatgtggtttaattcgacgcaacgcgaagaaccttaccaggtcttgacataccaggcaaagctatagagatatagtggaggatatcctggatacaggtggtgcatggttgtcgtcagctcgtgtcgtgagatgttgggttaagtcccgcaacgagcgcaacccttgtctttagttactaacattaagttgaggactctagagagactgccggtgacaaaccggaggaaggtggggatgacgtcaaatcatcatgccccttatgacctgggctacacacgtactacaatggcggatacaacgagaagcaagacagcaatgtggagcaaacctcagaaagtccgtctcagttcggattgaagtctgcaacccgacttcatgaagccggaatcgctagtaatcgcggatcagcatgccgcggtgaatacgttctcgggccttgtacacaccgcccgtcaaaccatgagagttggcaatacccgaagccggtggcctaaccctgcaaaggga

SEQ ID NO: 39 - DNA, 1399 bp, Unknown
  K39
cagtcgaacggtaacaggaagcagcttgctgctttgctgacgagtggcggacgggtgagtaatgtctgggaaactgcctgatggagggggataactactggaaacggtagctaataccgcataacgtcgcaagaccaaagagggggaccttagggcctcttgccatcggatgtgcccagatgggattagctagtaggtggggtaacggctcacctaggcgacgatccctagctggtctgagaggatgaccagccacactggaactgagacacggtccagactcctacgggaggcagcagtggggaatattgcacaatgggcgcaagcctgatgcagccatgccgcgtgtatgaagaaggccttcgggttgtaaagtactttcagcggggaggaagggagtaaagttaatacctttgctcattgacgttacccgcagaagaagcaccggctaactccgtgccagcagccgcggtaatacggagggtgcaagcgttaatcggaattactgggcgtaaagcgcacgcaggcggtttgttaagtcagatgtgaaatccccgggctcaacctgggaactgcatctgatactggcaagcttgagtctcgtagaggggggtagaattccaggtgtagcggtgaaatgcgtagagatctggaggaataccggtggcgaaggcggccccctggacgaagactgacgctcaggtgcgaaagcgtggggagcaaacaggattagataccctggtagtccacgccgtaaacgatgtcgacttggaggttgtgcccttgaggcgtggcttccggagctaacgcgttaagtcgaccgcctggggagtacggccgcaaggttaaaactcaaatgaattgacgggggcccgcacaagcggtggagcatgtggtttaattcgatgcaacgcgaagaaccttacctggtcttgacatccacggaagttttcagagatgagaatgtgccttcgggaaccgtgagacaggtgctgcatggctgtcgtcagctcgtgttgtgaaatgttgggttaagtcccgcaacgagcgcaacccttatcctttgttgccagcggtccggccgggaactcaaaggagactgccagtgataaactggaggaaggtggggatgacgtcaagtcatcatggcccttacgaccagggctacacacgtgctacaatggcgcatacaaagagaagcgacctcgcgagagcaagcggacctcataaagtgcgtcgtagtccggattggagtctgcaactcgactccatgaagtcggaatcgctagtaatcgtggatcagaatgccacggtgaatacgttcccgggccttgtacacaccgcccgtcacaccatgggagtgggttgcaaaagaagtaggtagcttaaccttcgggag

SEQ ID NO: 40 - DNA, 1384 bp, Unknown
  K40
agtcgaacggggttattttggaaatctcttcggagatggaattcttaacctagtggcggacgggtgagtaacgcgtgagcaatctgcctttaggagggggataacagtcggaaacggctgctaataccgcataatacgtttgggaggcatctcttgaacgtcaaagattttatcgcctttagatgagctcgcgtctgattagctggttggcggggtaacggcccaccaaggcgacgatcagtagccggactgagaggttgaacggccacattgggactgagacacggcccagactcctacgggaggcagcagtggggaatattgcgcaatgggggaaaccctgacgcagcaacgccgcgtgattgaagaaggccttcgggttgtaaagatctttaatcagggacgaaaaatgacggtacctgaagaataagctccggctaactacgtgccagcagccgcggtaatacgtagggagcaagcgttatccggatttactgggtgtaaagggcgcgcaggcgggccggcaagttgggagtgaaatcccggggcttaaccccggaactgctttcaaaactgctggtcttgagtgatggagaggcaggcggaattccgtgtgtagcggtgaaatgcgtagatatacggaggaacaccagtggcgaaggcggcctgctggacattaactgacgctgaggcgcgaaagcgtggggagcaaacaggattagataccctggtagtccacgccgtaaacgatggatactaggtgtgggaggtattgaccccttccgtgccgcagttaacacaataagtatcccacctggggagtacggccgcaaggttgaaactcaaaggaattgacgggggcccgcacaagcagtggagtatgtggtttaattcgaagcaacgcgaagaaccttaccaggtcttgacatcccgatgaccggcgtagagatacgccctctcttcggagcatcggtgacaggtggtgcatggttgtcgtcagctcgtgtcgtgagatgttgggttaagtcccgcaacgagcgcaacccttacggttagttgatacgcaagatcactctagccggactgccgttgacaaaacggaggaaggtggggacgacgtcaaatcatcatgccccttatgacctgggctacacacgtactacaatggcagtcatacagagggaagcaataccgcgaggtggagcaaatccctaaaagctgtcccagttcagattgcaggctgcaacccgcctgcatgaagtcggaattgctagtaatcgcggatcagcatgccgcggtgaatacgttcccgggccttgtacacaccgcccgtcacaccatgagagccgtcaatacccgaagtccgtagcctaaccgcaagggg

SEQ ID NO: 41 - DNA, 1392 bp, Unknown
  K41
agtcgaacgaagcactttatttgatttccttcgggactgattattttgtgactgagtggcggacgggtgagtaacgcgtgggtaacctgccttgtacagggggataacagttggaaacggctgctaataccgcataagcgcacggcatcgcatgatgcagtgtgaaaaactccggtggtataagatggacccgcgttggattagctagttggtgaggtaacggcccaccaaggcgacgatccatagccgacctgagagggtgaccggccacattgggactgagacacggcccaaactcctacgggaggcagcagtggggaatattgcacaatgggcgaaagcctgatgcagcgacgccgcgtgagcgaagaagtatttcggtatgtaaagctctatcagcagggaagataatgacggtacctgactaagaagcaccggctaaatacgtgccagcagccgcggtaatacgtatggtgcaagcgttatccggatttactgggtgtaaagggagcgcaggcggtgcggcaagtctgatgtgaaagcccggggctcaaccccggtactgcattggaaactgtcgtactagagtgtcggaggggtaagcggaattcctagtgtagcggtgaaatgcgtagatattaggaggaacaccagtggcgaaggcggcttactggacgataactgacgctgaggctcgaaagcgtggggagcaaacaggattagataccctggtagtccacgccgtaaacgatgaatactaggtgttgggaagcattgcttctcggtgccgtcgcaaacgcagtaagtattccacctggggagtacgttcgcaagaatgaaactcaaaggaattgacggggacccgcacaagcggtggagcatgtggtttaattcgaagcaacgcgaagaaccttaccaagtcttgacatccttctgaccggtacttaaccgtaccttctcttcggagcaggagtgacaggtggtgcatggttgtcgtcagctcgtgtcgtgagatgttgggttaagtcccgcaacgagcgcaacccttatctttagtagccagcggttcggccgggcactctagagagactgccagggataacctggaggaaggcggggatgacgtcaaatcatcatgccccttatgacttgggctacacacgtgctacaatggcgtaaacaaagggaagcaaagctgtgaagccgagcaaatctcaaaaataacgtctcagttcggactgtagtctgcaacccgactacacgaagctggaatcgctagtaatcgcagatcagaatgctgcggtgaatacgttcccgggtcttgtacacaccgcccgtcacaccatgggagttgggaatgcccgaagccagtgacctaaccgaaaggaagga

SEQ ID NO: 42 - DNA, 1397 bp, Unknown
  K42
cagtcgaacgaagcatatagagacgagtatttcggtatgagtaactatatgactgagtggcggacgggtgagtaacgcgtggataacctgcctcatacagggggataacagttagaaatgactgctaataccgcataagcgcacagtgctgcatggcacagtgtgaaaagctccggcggtatgagatggatccgcgtttgattagctagttggtggggtaaaggcctaccaaggcgacgatcaatagccgacctgagagggtgaccggccacattgggactgagacacggcccaaactcctacgggaggcagcagtggggaatattgcacaatgggggaaaccctgatgcagcgacgccgcgtgaaggaagaagtatttcggtatgtaaacttctatcagcagggaagaaaatgacggtacctgactaagaagccccggctaattacgtgccagcagccgcggtaatacgtaaggggcaagcgttatccggatttactgggtgtaaagggagcgtagacggcagtgcaagtctgatgtgaaagcccggggctcaaccccgggactgcattggaaactgtgcagctagagtgtcggagaggtaagtggaattcctagtgtagcggtgaaatgcgtagatattaggaggaacaccagtggcgaaggcggcttactggacgataactgacgttgaggctcgaaagcgtggggagcaaacaggattagataccctggtagtccacgccgtaaacgatgaatactaggtgtcgggcgccaaaggcgttcggtgccgcagcaaacgcaataagtattccacctggggagtacgttcgcaagaatgaaactcaaaggaattgacggggacccgcacaagcggtggagcatgtggtttaattcgaagcaacgcgaagaaccttaccaagtcttgacatctgcctgaccggtccgtaacaggacccttccttcgggacaggcaagacaggtggtgcatggttgtcgtcagctcgtgtcgtgagatgttgggttaagtcccgcaacgagcgcaacccttatccttagtagccagcaggtagagctgggcactctagggagactgccagggacaacctggaggaaggtggggatgacgtcaaatcatcatgccccttatgatttgggctacacacgtgctacaatggcgtaaacaaagggaagcgaaggggtgacctgaagcaaatcccaaaaataacgtctcagttcggattgtagtctgcaactcgactacatgaagctggaatcgctagtaatcgcgaatcagaatgtcgcggtgaatacgttcccgggtcttgtacacaccgcccgtcacaccatgggagtcggatatgcccgaagccggtgaccgaacccgaaagggaaggag

SEQ ID NO: 43 - DNA, 1388 bp, Unknown
  K43
agtcgaacggagcacccttgactgaggtttcggccaaatgataggaatgcttagtggcggactggtgagtaacgcgtgaggaacctgccttccagagggggacaacagttggaaacgactgctaataccgcatgacgcatgaccggggcatcccgggcatgtcaaagattttatcgctggaagatggcctcgcgtctgattagctagatggtggggtaacggcccaccatggcgacgatcagtagccggactgagaggttgaccggccacattgggactgagatacggcccagactcctacgggaggcagcagtggggaatattgggcaatggacgcaagtctgacccagcaacgccgcgtgaaggaagaaggctttcgggttgtaaacttcttttgtcagggaagagtagaagacggtacctgacgaataagccacggctaactacgtgccagcagccgcggtaatacgtaggtggcaagcgttgtccggatttactgggtgtaaagggcgtgcagccgggccggcaagtcagatgtgaaatctggaggcttaacctccaaactgcatttgaaactgtaggtcttgagtaccggagaggttatcggaattccttgtgtagcggtgaaatgcgtagatataaggaagaacaccagtggcgaaggcggataactggacggcaactgacggtgaggcgcgaaagcgtggggagcaaacaggattagataccctggtagtccacgctgtaaacgatggatactaggtgtgcggggactgaccccctgcgtgccgcagttaacacaataagtatcccacctggggagtacgatcgcaaggttgaaactcaaaggaattgacgggggcccgcacaagcggtggattatgtggtttaattcgaagcaacgcgaagaaccttaccagggcttgacatcctactaacgaagtagagatacatcaggtgcccttcggggaaagtagagacaggtggtgcatggttgtcgtcagctcgtgtcgtgagatgttgggttaagtcccgcaacgagcgcaacccctattgttagttgctacgcaagagcactctagcgagactgccgttgacaaaacggaggaaggtggggacgacgtcaaatcatcatgccccttatgtcctgggctacacacgtaatacaatggcggtcaacagagggaggcaaagccgcgaggcagagcaaacccccaaaagccgtcccagttcggatcgcaggctgcaacccgcctgcgtgaagtcggaatcgctagtaatcgcggatcagcatgccgcggtgaatacgttcccgggccttgtacacaccgcccgtcacaccatgagagtcgggaacacccgaagtccgtagcctaaccgcaaggagg

SEQ ID NO: 44 - DNA, 1393 bp, Unknown
  K44
tgcagtcgaacggagtgccttagaaagaggattcgtccaattgataaggttacttagtggcggacgggtgagtaacgcgtgaggaacctgcctcggagtggggaataacagaccgaaaggcctgctaataccgcatgatgcagttggaccgcatggtcctgactgccaaagatttatcgctctgagatggcctcgcgtctgattagcttgttggcggggtaatggcccaccaaggcgacgatcagtagccggactgagaggttggccggccacattgggactgagacacggcccagactcctacgggaggcagcagtggggaatattgggcaatgggcgcaagcctgacccagcaacgccgcgtgaaggaagaaggctttcgggttgtaaacttcttttctcagggacgaacaaatgacggtacctgaggaataagccacggctaactacgtgccagcagccgcggtaatacgtaggtggcaagcgttatccggatttactgggtgtaaagggcgtgtaggcgggaaggcaagtcagatgtgaaaactatgggctcaacccatagcctgcatttgaaactgtttttcttgagtgctggagaggcaatcggaattccgtgtgtagcggtgaaatgcgtagatatacggaggaacaccagtggcgaaggcggattgctggacagtaactgacgctgaggcgcgaaagcgtggggagcaaacaggattagataccctggtagtccacgctgtaaacgatggatactaggtgtgggggggtctgaccccctccgtgccgcagttaacacaataagtatcccacctggggagtacgatcgcaaggttgaaactcaaaggaattgacgggggcccgcacaagcggtggagtatgtggtttaattcgaagcaacgcgaagaaccttaccagggcttgacatcctactaacgaagcagagatgcattaggtgcccttcggggaaagtagagacaggtggtgcatggttgtcgtcagctcgtgtcgtgagatgttgggttaagtcccgcaacgagcgcaacccttattgttagttgctacgcaagagcactctagcgagactgccgttgacaaaacggaggaaggcggggacgacgtcaaatcatcatgccccttatgtcctgggctacacacgtactacaatggtggtaaacagagggaagcaagaccgcgaggtggagcaaatccctaaaagccatcccagttcggattgcaggctgaaacccgcctgtatgaagttggaatcgctagtaatcgcggatcagcatgccgcggtgaatacgttcccgggccttgtacacaccgcccgtcacaccatgagagtcgggaacacccgaagtccgtagtctaaccgcaaggggga

SEQ ID NO: 45 - DNA, 1409 bp, Unknown
  K45
caagtagaacgctgactactttagcttgctagagtagaaggagttgcgaacgggtgagtaacgcgtaggtaacctgcctactagcgggggataactattggaaacgatagctaataccgcataacagtgtttaacacatgttagatgcttgaaagatgcaattgcatcactagtagatggacctgcgttgtattagctagttggtggggtaacggcccaccaaggcgacgatacatagccgacctgagagggtgatcggccacactgggactgagacacggcccagactcctacgggaggcagcagtagggaatcttcggcaatgggggcaaccctgaccgagcaacgccgcgtgagtgaagaaggttttcggatcgtaaagctctgttgtaagagaagaacgtgtgtgagagtggaaagttcacacagtgacggtaacttaccagaaagggacggctaactacgtgccagcagccgcggtaatacgtaggtcccgagcgttgtccggatttattgggcgtaaagcgagcgcaggcggtttaataagtctgaagttaaaggcagtggcttaaccattgttcgctttggaaactgttaaacttgagtgcagaaggggagagtggaattccatgtgtagcggtgaaatgcgtagatatatggaggaacaccggtggcgaaagcggctctctggtctgtaactgacgctgaggctcgaaagcgtggggagcaaacaggattagataccctggtagtccacgccgtaaacgatgagtgctaggtgttaggccctttccggggcttagtgccgcagctaacgcattaagcactccgcctggggagtacgaccgcaaggttgaaactcaaaggaattgacgggggcccgcacaagcggtggagcatgtggtttaattcgaagcaacgcgaagaaccttaccaggtcttgacatcccgatgctatttctagagatagaaagtttcttcggaacatcggtgacaggtggtgcatggttgtcgtcagctcgtgtcgtgagatgttgggttaagtcccgcaacgagcgcaacccctattgttagttgccatcatttagttgggcactctagcgagactgccggtaataaaccggaggaaggtggggatgacgtcaaatcatcatgccccttatgacctgggctacacacgtgctacaatggttggtacaacgagtcgcaagtcggtgacggcaagcaaatctcttaaagccaatctcagttcggattgtaggctgcaactcgcctacatgaagtcggaatcgctagtaatcgcggatcagcacgccgcggtgaatacgttcccgggccttgtacacaccgcccgtcacaccacgagagtttgtaacacccgaagtcggtgaggtaaccatttaggagcc

SEQ ID NO: 46 - DNA, 1395 bp, Unknown
  K46
caagtcgaacggcagcgcggggagcttgctccctggcggcgagtggcgcacgggtgagtaatacatcggaacgtgtcttctagtgggggataactgcccgaaagggcagctaataccgcatgagacctgagggtgaaagcgggggatcgcaagacctcgcgctggaagagcggccgatgtccgattagctagttggtgaggtaaaggctcaccaaggcgacgatcggtagctggtctgagaggacgaccagccacactgggactgagacacggcccagactcctacgggaggcagcagtggggaattttggacaatgggggcaaccctgatccagccatgccgcgtgcaggatgaaggtcttcggattgtaaactgcttttgtcagggacgaaaagggatgcgataacaccgcattccgctgacggtacctgaagaataagcaccggctaactacgtgccagcagccgcggtaatacgtagggtgcaagcgttaatcggaattactgggcgtaaagcgtgcgcaggcggttctgtaagatagatgtgaaatccccgggctcaacctgggaattgcatatatgactgcaggacttgagtttgtcagaggagggtggaattccacgtgtagcagtgaaatgcgtagatatgtggaagaacaccgatggcgaaggcagccctctgggacatgactgacgctcatgcacgaaagcgtggggagcaaacaggattagataccctggtagtccacgccctaaacgatgtctactagttgttggggacgatagtccttggtaacgcagctaacgcgtgaagtagaccgcctggggagtacggtcgcaagattaaaactcaaaggaattgacggggacccgcacaagcggtggatgatgtggattaattcgatgcaacgcgaaaaaccttacctagccttgacatgccaggaaggcctgagagatcaggccgtgcccgcaagggaatctggacacaggtgctgcatggctgtcgtcagctcgtgtcgtgagatgttgggttaagtcccgcaacgagcgcaacccttgtcattagttgctacgaaagggcactctaatgagactgccggtgacaaaccggaggaaggtggggatgacgtcaagtcctcatggcccttatggctagggcctcacacgtcatacaatggtcggaacagagggaagcgaagccgcgaggtgaagccaatcccagaaaaccgatcgtagtccggattgcagtctgcaactcgactgcatgaagtcggaatcgctagtaatcgcggatcagcatgccgcggtgaatacgttcccgggtcttgtacacaccgcccgtcacaccatgggagtggggttcaccagaagacgtttgcccaaccgaaaggaagg

SEQ ID NO: 47 - DNA, 1384 bp, Unknown
  K47
agtcgaacgggatcccaggagcttgctcctgggtgagagtggcgaacgggtgagtaatgcgtgaccgacctgccccatacaccggaatagctcctggaaacgggtggtaatgccggatgctccagttgaccgcatggtcctctgggaaagattctatcggtatgggatggggtcgcgtcctatcagcttgatggcggggtaacggcccaccatggcttcgacgggtagccggcctgagagggcgaccggccacattgggactgagatacggcccagactcctacgggaggcagcagtggggaatattgcacaatgggcgcaagcctgatgcagcgacgccgcgtgcgggatgacggccttcgggttgtaaaccgcttttgactgggagcaagcccttcggggtgagtgtacctttcgaataagcaccggctaactacgtgccagcagccgcggtaatacgtagggtgcaagcgttatccggaattattgggcgtaaagggctcgtaggcggttcgtcgcgtccggtgtgaaagtccatcgcttaacggtggatccgcgccgggtacgggcgggcttgagtgcggtaggggagactggaattcccggtgtaacggtggaatgtgtagatatcgggaagaacaccaatggcgaaggcaggtctctgggccgtcactgacgctgaggagcgaaagcgtggggagcgaacaggattagataccctggtagtccacgccgtaaacggtggatgctggatgtggggaccattccacggtctccgtgtcggagccaacgcgttaagcatcccgcctggggagtacggccgcaaggctaaaactcaaagaaattgacgggggcccgcacaagcggcggagcatgcggattaattcgatgcaacgcgaagaaccttacctgggcttgacatgttcccgacagccgtagagatacggtctcccttcggggcgggttcacaggtggtgcatggtcgtcgtcagctcgtgtcgtgagatgttgggttaagtcccgcaacgagcgcaaccctcgccctgtgttgccagcacgtcgtggtgggaactcacgggggaccgccggggtcaactcggaggaaggtggggatgacgtcagatcatcatgccccttacgtccagggcttcacgcatgctacaatggccggtacaacgggatgcgacatcgtgagggggagcggatcccttaaaaccggtctcagttcggattggagtctgcaacccgactccatgaaggcggagtcgctagtaatcgcggatcagcaacgccgcggtgaatgcgttcccgggccttgtacacaccgcccgtcaagtcatgaaagtgggtagcacccgaagccggtggcccaaccttttggggg

SEQ ID NO: 48 - DNA, 1387 bp, Unknown
  K48
gtcgaacggagctgctttgatgaagttttcggatggatttaaaacagcttagtggcggacgggtgagtaacgcgtgggtaacctgcctcacactgggggataacagttagaaatagctgctaataccgcataagcgcacagttccgcatggaacagtgtgaaaaactccggtggtgtgagatggacccgcgtctgattagccagttggcggggtaacggcccaccaaagcgacgatcagtagccggcctgagagggtgaacggccacattgggactgagacacggcccaaactcctacgggaggcagcagtggggaatattgcacaatgggggaaaccctgatgcagcgacgccgcgtgagtgaagaagtatttcggtatgtaaagctctatcagcagggaagaaagtgacggtacctgaataagaagccccggctaactacgtgccagcagccgcggtaatacgtagggggcaagcgttatccggatttactgggtgtaaagggagcgtagacggcaaggcaagtctgaagtgaaagcccggtgcttaacgccgggactgctttggaaactgtttggctggagtgccggagaggtaagcggaattcctagtgtagcggtgaaatgcgtagatattaggaagaacaccagtggcgaaggcggcttactggacggtaactgacgttgaggctcgaaagcgtggggagcaaacaggattagataccctggtagtccacgccgtaaacgatgattgctaggtgtaggtgggtatggacccatcggtgccgcagctaacgcaataagcaatccacctgggggagtacgttcgcaagaatgaaactcaaaggaattgacggggacccgcacaagcggtggagcatgtggtttaattcgaagcaacgcgaagaaccttaccaggtcttgacatcccgatgaaaaacccgtaacggggttccctcttcggagcatcggagacaggtggtgcatggttgtcgtcagctcgtgtcgtgagatgttgggttaagtcccgcaacgagcgcaacccttattcttagtagccagcaggtaaagctgggcactctaaggagactgccggggataacccggaggaaggtggggatgacgtcaaatcatcatgccccttatgatctgggctacacacgtgctacaatggcgtaacaaagggaagcgagcctgcgagggtgagcgaatcccaaaaataacgtcccagttcggactgtagtctgcaacccgactacacgaagctggaatcgctagtaatcgcgaatcagaatgtcgcggtgaatacgttcccgggtcttgtacacaccgcccgtcacaccatgggagtcggaaatgcccgaagtctgtgactcaaccgcaaggag

SEQ ID NO: 49 - DNA, 1368 bp, Unknown
  K49
ttaaggagattcttcggatgattcttgactgactgagcggcggacgggtgagtaacgcgtgggtgacctgccccataccgggggataacagctggaaacggctgctaataccgcataagcgcacagagctgcatggctcggtgtgaaaaactccggtggtatgggatgggcccgcgtctgattaggcagttggcggggtaacggcccaccaaaccgacgatcagtagccggcctgagagggcgaccggccacattgggactgagacacggcccaaactcctacgggaggcagcagtggggaatattgcacaatgggggaaaccctgatgcagcgacgccgcgtgagcgaagaagtatttcggtatgtaaagctctatcagcagggaagataatgacggtacctgactaagaagccccggctaactacgtgccagcagccgcggtaatacgtagggggcaagcgttatccggatttactgggtgtaaagggagcgtagacggcaaggcaagtctgatgtgaaaacccagggcttaaccctgggactgcattggaaactgtctggctcgagtgccggagaggtaagcggaattcctagtgtagcggtgaaatgcgtagatattaggaagaacaccagtggcgaaggcggcttactggacggtaactgacgttgaggctcgaaagcgtggggagcaaacaggattagataccctggtagtccacgccgtaaacgatgaatgctaggtgttggggagcaaagctcttcggtgccgccgcaaacgcattaagcattccacctggggagtacgttcgcaagaatgaaactcaaaggaattgacggggacccgcacaagcggtggagcatgtggtttaattcgaagcaacgcgaagaaccttaccaggtcttgacatcccgatgaccggcccgtaacggggccttctcttcggagcattggagacaggtggtgcatggttgtcgtcagctcgtgtcgtgagatgttgggttaagtcccgcaacgagcgcaacccttatcctcagtagccagcaggtcaagctgggcactctgtggagactgccagggataacctggaggaaggtggggatgacgtcaaatcatcatgccccttatgatctgggctacacacgtgctacaatggcgtaaacaaagggaggcaaagccgcgaggtggagcaaatcccaaaaataacgtctcagttcggactgcagtctgcaactcgactgcacgaagctggaatcgctagtaatcgcgaatcagaatgtcgcggtgaatacgttcccgggtcttgtacacaccgcccgtcacaccatgggagttggtaacgcccgaagtcagtgacccaaccttcag

SEQ ID NO: 50 - DNA, 1390 bp, Unknown
  K50
gtcgagcgaagcacttatgatgattcttcggatgaatcatttgtgactgagcggcggacgggtgagtaacgcgtgagtaacctgcctcatacaggggaataacagttagaaatgactgctaatgccgcataagcgcacagggccgcatggcccggtgtgaaaaactccggtggtatgagatggactcgcgtctgattagctagttggcagggtaacggcctaccaaggcgacgatcagtagccggcctgagagggtgaacggccacattgggactgagacacggcccaaactcctacgggaggcagcagtggggaatattgcacaatgggggaaaccctgatgcagcgacgccgcgtgagtgaagaagtatttcggtatgtaaagctctatcagcagggaagaaaatgacggtacctgactaagaagccccggctaactacgtgccagcagccgcggtaatacgtagggggcaagcgttatccggatttactgggtgtaaagggagcgtagacggctttgcaagtctgacgtgaaactccggggctcaactccggaactgcgttggaaactgtaaggcttgagtgccggagaggtaagcggaattcctagtgtagcggtgaaatgcgtagatattaggaggaacaccagtggcgaaggcggcttactggacggcaactgacgttgaggctcgaaagcgtggggagcaaacaggattagataccctggtagtccacgcggtaaacgatgaatactaggtgttgggggacaaagtccttcggtgccgccgcaaacgcattaagtattccacctgggggagtacgttcgcaagaatgaaactcaaaggaattgacggggacccgcacaagcggtggagcatgtggtttaattcgaagcaacgcgaagaaccttaccaagtcttgacatcgattcgacgggagtgtaatgactcctttcccttcggggacgaagaagacaggtggtgcatggttgtcgtcagctcgtgtcgtgagatgttgggttaagtcccgcaacgagcgcaacccttatcttcagtagccagcgagtaaggtcgggcactctggagagactgccagggacaacctggaggaaggtggggatgacgtcaaatcatcatgccccttatgacttgggctacacacgtgctacaatggcgtaaacaaagggaagcgaacctgtgagggtgggcaaatcccaaaaataacgtctcagttcggattgtagtctgcaactcgactacatgaagctggaatcgctagtaatcgcgaatcagcatgtcgcggtgaatacgttcccgggtcttgtacacaccgcccgtcacaccatgggagtcggtaacgcccgaagtcagtgacccaaccgcaaggaggg

SEQ ID NO: 51 - DNA, 1382 bp, Unknown
  K51
gcagtcggacgcaatgcttcggcattgagtggcgaacgggtgagtaagacataagcaacctgcccctgtgagggggataactgctggaaacggcagctaagaccgcataggcatagaggacgcatgtcgactatgttaaatatcccacgggatagcacagggatgggcttatgacgcattagccagctggtgaggtaacggctcaccagggcgacgatgcgtagccggcctgagagggtggacggccacactgggactgagacacggcccagactcctacgggaggcagcagtagggaattttcggcaatgggcgaaagcctgaccgagcaacgccgcgtgaaggaagaagtcattcgtgatgtaaacttctgttatgaaggaagaacggcagatggagggaatgccatgtgcgtgacggtacttcatgaggaagccacggctaactacgtgccagcagccgcggtaatacgtaggtggcgagcgttatccggaatcattgggcgtaaagagggagcaggcggcagtgcaggtctgcggtgaaagaccggagctaaacttcggtaagccgtggaaaccgcacagctagagagcatcagaggatcgcggaattccatgtgtagcggtgaaatgcgtagatatatggaggaacaccagtggcgaaggcggcggtctggggtgcagctgacgctcagtcccgaaagcgtggggagcaaataggattagataccctagtagtccacgccgtaaacgatgagtgctaagtgttgggggtcagacctcagtgctggagttaacgcaataagcactccgcctgagtagtacgttcgcaagaatgaaactcaaaggaattgacgggggcccgcacaaagcggtggagcatgtggtttaattcgaagcaacgcgaagaaccttaccaggtcttgacatggagataaaggccctggagacagggagatagatatatctcacacaggtggtgcatggttgtcgtcagctcgtgtcgtgagatgttgggttaagtcccgcaacgagcgcaacccctgttgccagttgccagcattaggttggggactctggcgagactgcctctgcaaggaggaggaaggcggggatgacgtcaaatcatcatgccccttatgacctgggctacacacgtgctacaatggacggatcagagggaggcgaagccgcgaggtggagcgaaacccagaaacccgttcacagttcggactgcagtctgcaactcgactgcacgaagctggaatcgctagtaatcgcgaatcagcatgtcgcggtgaatacgttctcgggccttgtacacaccgcccgtcacaccatgagagttggtaacacccgaagccggtggcccaaccgcaagga

SEQ ID NO: 52 - DNA, 1388 bp, Unknown
  K52
agtcgaacgggaaatattttattgaaacttcggtggatttaatttatttctagtggcggacgggtgagtaacgcgtgggtaacctgccttatactgggggataacagccagaaatgactgctaataccgcataagcgcacagaaccgcatggttcggtgtgaaaaactccggtggtataagatggacccgcgttggattagctagttggcagggcagcggcctaccaaggcgacgatccatagccggcctgagagggtgaacggccacattgggactgagacacggcccagactcctacgggaggcagcagtggggaatattgcacaatgggggaaaccctgatgcagcgacgccgcgtgaaggaagaagtatctcggtatgtaaacttctatcagcagggaagataatgacggtacctgactaagaagccccggctaactacgtgccagcagccgcggtaatacgtagggggcaagcgttatccggatttactgggtgtaaagggagcgtagacggcgcagcaagtctgatgtgaaaggcaggggcttaacccctggactgcattggaaactgctgtgcttgagtgccggaggggtaagcggaattcctagtgtagcggtgaaatgcgtagatattaggaggaacaccagtggcgaaggcggcttactggacggtaactgacgttgaggctcgaaagcgtggggagcaaacaggattagataccctggtagtccacgccgtaaacgatgaatactaggtgtcagggagcacagctctttggtgccgccgcaaacgcattaagtattccacctggggagtacgttcgcaagaatgaaactcaaaggaattgacggggacccgcacaagcggtggagcatgtggtttaattcgaagcaacgcgaagaaccttaccaaatcttgacatccctctgaccgggacttaaccgtccctttccttcgggacaggggagacaggtggtgcatggttgtcgtcagctcgtgtcgtgagatgttgggttaagtcccgcaacgagcgcaacccctatccttagtagccagcacgcagtggtgggcactctgaggagactgccagggataacctggaggaaggcggggatgacgtcaaatcatcatgccccttatgatttgggctacacacgtgctacaatggcgtaaacaaagggaagcgaacccgcgagggtgggcaaatctcaaaaataacgtcccagttcggactgcagtctgcaactcgactgcacgaagctggaatcgctagtaatcgcggatcagaatgccgcggtgaatacgttcccgggtcttgtacacaccgcccgtcacaccatgggagtcagtaacgcccgaagtcagtgacctaaccgcaagggag

SEQ ID NO: 53 - DNA, 1385 bp, Unknown
  K53
cgaacgggaattatttcattgagacttcggtggatttgatctatttctagtggcggacgggtgagtaacgcgtgggtaacctgccttatacagggggataacagtcagaaatggctgctaataccgcataagcgcacagagctgcatggctcagtgtgaaaaactccggtggtataagatggacccgcgttggattagcttgttggtggggtaacggcccaccaaggcgacgatccatagccggcctgagagggtgaacggccacattgggactgagacacggcccagactcctacgggaggcagcagtggggaatattgcacaatgggggaaaccctgatgcagcgacgccgcgtgaaggaagaagtatctcggtatgtaaacttctatcagcagggaagatagtgacggtacctgactaagaagccccggctaactacgtgccagcagccgcggtaatacgtagggggcaagcgttatccggatttactgggtgtaaagggagcgtagacggtgtggcaagtctgatgtgaaaggcatgggctcaacctgtggactgcattggaaactgtcatacttgagtgccggaggggtaagcggaattcctagtgtagcggtgaaatgcgtagatattaggaggaacaccagtggcgaaggcggcttactggacggtaactgacgttgaggctcgaaagcgtggggagcaaacaggattagataccctggtagtccacgccgtaaacgatgaatactaggtgtcggggagcatggctcttcggtgccgtcgcaaacgcagtaagtattccacctgggggagtacgttcgcaagaatgaaactcaaaggaattgacggggacccgcacaagcggtggagcatgtggtttaattcgaagcaacgcgaagaaccttaccaagtcttgacatccgcctgaccgatccttaatcggatcttttcttcgggacagacgagacaggtggtgcatggttgtcgtcagctcgtgtcgtgagatgttgggttaagtcccgcaacgagcgcaacccctatcctcagtagccagcatttaaggtgggcactctggggagactgccagggataacctggaggaaggcggggatgacgtcaaatcatcatgccccttatgatttgggctacacacgtgctacaatggcgtaaacaaagggaagcgagatcgtgagatggagcaaatcccaaaaataacgtcccagttcggactgtagtctgcaacccgactacacgaagctggaatcgctagtaatcgcggatcagaatgccgcggtgaatacgttcccgggtcttgtacacaccgcccgtcacaccatgggagtcagtaacgcccgaagtcagtgacctaactgcaaagaag

SEQ ID NO: 54 - DNA, 1415 bp, Unknown
  K54
gtcgaacggagaattttatttcggtagaattcttagtggcgaacgggtgagtaacgcgtaggcaacctgccctttagacggggacaacattccgaaaggagtgctaataccggatgtgatcatcgtgccgcatggcaggatgaagaaagatggcctctacaagtaagctatcgctaaaggatgggcctgcgtctgattagctagttggtagtgtaacggactaccaaggcgatgatcagtagccggtctgagaggatgaacggccacattgggactgagacacggcccaaactcctacgggaggcagcagtggggaatcttccgcaatggacgaaagtctgacggagcaacgccgcgtgagtgatgaaggatttcggtctgtaaagctctgttgtttatgacgaacgtgcagtgtgtgaacaatgcattgcaatgacggtagtaaacgaggaagccacggctaactacgtgccagcagccgcggtaatacgtaggtggcgagcgttgtccggaattattgggcgtaaagagcatgtaggcggcttaataagtcgagcgtgaaaatgcggggctcaaccccgtatggcgctggaaactgttaggcttgagtgcaggagaggaaaggggaattcccagtgtagcggtgaaatgcgtagatattgggaggaacaccagtggcgaaggcgcctttctggactgtgtctgacgctgagatgcgaaagccagggtagcgaacgggattagataccccggtagtcctggccgtaaacgatgggtactaggtgtaggaggtatcgaccccttctgtgccggagttaacgcaataagtaccccgcctggggagtacggccgcaaggttgaaactcaaaggaattgacgggggcccgcacaagcggtggagtatgtggtttaattcgacgcaacgcgaagaaccttaccaaggcttgacattgattgaacgctctagagatagagctttcccttcggggacaagaaaacaggtggtgcatggctgtcgtcagctcgtgtcgtgagatgttgggttaagtcccgcaacgagcgcaacccctatcctatgttaccagcaagtaaagttggggactcatgggagactgccagggacaacctggaggaaggcggggatgacgtcaagtcatcatgccccttatgtcttgggctacacacgtactacaatggtcggaaacagagggaagcgaagccgcgaggcagagcaaaccccagaaacccgatctcagttcggatcgcaggctgcaacccgcctgcgtgaagtcggaatcgctagtaatcgcaggtcagcatactgcggtgaatacgttcccgggccttgtacacaccgcccgtcacaccacgaaagttggtaacacccgaagccggtgaggtaacctattaggagc

SEQ ID NO: 55 - DNA, 1366 bp, Unknown
  K55
atgaggtagcaataccttgatggcgaccggcgcacgggtgagtaacgcgtatgcaacctgcctgataccggggtatagcccatggaaacgtggattaacaccccatagtacttttatcctgcatgggatgtgagttaaatgttcaaggtatcggatgggcatgcgtcctattagttagttggcggggtaacagcccaccaagacgatgataggtaggggttctgagaggaaggtcccccacattggaactgagacacggtccaaactcctacgggaggcagcagtgaggaatattggtcaatggacgagagtctgaaccagccaagtcgcgtgagggaagactgccctatgggttgtaaacctcttttataagggaagaataagttctacgtgtagaatgatgcctgtaccttatgaataagcatcggctaactccgtgccagcagccgcggtaatacggaggatgcgagcgttatccggatttattgggtttaaagggtgcgtaggcggtttattaagttagtggttaaatatttgagctaaactcaattgtgccattaatactggtaaactggagtacagacgaggtaggcggaataagttaagtagcggtgaaatgcatagatataacttagaactccgatagcgaaggcagcttaccagactgtaactgacgctgatgcacgagagcgtgggtagcgaacaggattagataccctggtagtccacgccgtaaacgatgctcactggttctgtgcgatatattgtacgggattaagcgaaagtattaagtgagccacctggggagtacgtcggcaacgatgaaactcaaaggaattgacgggggcccgcacaagcggaggaacatgtggtttaattcgatgatacgcgaggaaccttacctgggtttaaatgggaaatgtcgtatttggaaacagatattctcttcggagcgtttttcaaggtgctgcatggttgtcgtcagctcgtgccgtgaggtgtcgggttaagtcccataacgagcgcaacccttaccgttagttgctagcatgtaatgatgagcactctaacgggactgccaccgtaaggtgagaggaaggcggggatgacgtcaaatcagcacggcccttacacccagggctacacacgtgttacaatggccggtacagagggccgctaccaggtgactggatgccaatctcaaaagccggtcgtagttcggattggagtctgtaacccgactccatgaagttggattcgctagtaatcgcgcatcagccatggcgcggtgaatacgttcccgggccttgtacacaccgcccgtcaagccatggaagccgggggtgcctgaagtccgtaaccgcga

SEQ ID NO: 56 - DNA, 1364 bp, Unknown
  K56
  misc_feature (923)..(924): n is a, c, g, or t
  misc_feature (1349)..(1349): n is a, c, g, or t
  misc_feature (1351)..(1352): n is a, c, g, or t
tcgaacgagcgagagagagcttgctttctcgagcgagtggcgaacgggtgagtaacgcgtgaggaacctgcctcaaagagggggacaacagttggaaacgactgctaataccgcataagcccacgggtcggcatcgaccagagggaaaaggagcaatccgctttgagatggcctcgcgtccgattagctagttggtgaggtaacggcccaccaaggcgacgatcggtagccggactgagaggttgaacggccacattgggactgagacacggcccagactcctacgggaggcagcagtggggaatattgcacaatgggggaaaccctgatgcagcgacgccgcgtggaggaagaaggtcttcggattgtaaactcctgttgttggggaagataatgacggtacccaacaaggaagtgacggctaactacgtgccagcagccgcggtaaaacgtaggtcacaagcgttgtccggaattactgggtgtaaagggagcgcaggcgggaagacaagttggaagtgaaatctatgggctcaacccataaactgctttcaaaactgtttttcttgagtagtgcagaggtaggcggaattcccggtgtagcggtggaatgcgtagatatcgggaggaacaccagtggcgaaggcggcctactgggcaccaactgacgctgaggctcgaaagtgtgggtagcaaacaggattagataccctggtagtccacaccgtaaacgatgattactaggtgttggaggattgaccccttcagtgccgcagttaacacaataagtaatccacctggggagtacgaccgcaaggttgaaactcaaaggaattgacgggggcccgcacaagcagtggagtatgtggtttaattcgacgcaacgcgaagaaccttaccaagtcttgacatcccttgacagnnatagaaatatgttttctcttcggagcaaggagacaggtggtgcatggttgtcgtcagctcgtgtcgtgagatgttgggttaagtcccgcaacgagcgcaacccttatggtcagttactacgcaagaggactctggccagactgccgttgacaaaacggaggaaggtggggatgacgtcaaatcatcatgccctttatgacttgggctacacacgtactacaatggcgttaaacaaagagaagcaagaccgcgaggtggagcaaaactcagaaacaacgtcccagttcggactgcaggctgcaactcgcctgcacgaagtcggaattgctagtaatcgtggatcagcatgccacggtgaatacgttcccgggccttgtacacaccgcccgtcacaccatgagagccggggggacccgaagtcggtngnntaaccgcaagga

SEQ ID NO: 57 - DNA, 1391 bp, Unknown
  K57
tgcagtcgaacggagtgctcatgacagaggattcgtccaatggagtgagttacttagtggcggacgggtgagtaacgcgtgagtaacctgccttggagtggggaataacaggtggaaacatctgctaataccgcatgatgcagttgggtcgcatggctctgactgccaaagatttatcgctctgagatggactcgcgtctgattagctggttggcggggtaacggcccaccaaggcgacgatcagtagccggactgagaggttggccggccacattgggactgagacacggcccagactcctacgggaggcagcagtggggaatattgggcaatgggcgcaagcctgacccagcaacgccgcgtgaaggaagaaggctttcgggttgtaaacttcttttctcagggacgaagcaagtgacggtacctgaggaataagccacggctaactacgtgccagcagccgcggtaatacgtaggtggcgagcgttatccggatttactgggtgtaaagggcgtgtaggcgggactgcaagtcagatgtgaaaaccatgggctcaacctgtggcctgcatttgaaactgtagttcttgagtactggagaggcagacggaattcctagtgtagcggtgaaatgcgtagatattaggaggaacaccagtggcgaaggcggtctgctggacagcaactgacgctgaggcgcgaaagcgtggggagcaaacaggattagataccctggtagtccacgctgtaaacgatggatactaggtgtggggggtctgaccccctccgtgccgcagttaacacaataagtatcccacctggggagtacgatcgcaaggttgaaactcaaaggaattgacgggggcccgcacaagcggtggagtatgtggtttaattcgaagcaacgcgaagaaccttaccagggcttgacatcccggtgaccggtgtagagatacaccttcttcttcggaagcgccggtgacaggtggtgcatggttgtcgtcagctcgtgtcgtgagatgttgggttaagtcccgcaacgagcgcaacccttattgttagttgctacgcaagagcactctagcgagactgccgttgacaaaacggaggaaggtggggacgacgtcaaatcatcatgccccttatgtcctgggccacacacgtactacaatggtggtcaacagagggaagcaagaccgcgaggtggagcaaacccctaaaagccatcccagttcggattgcaggctgcaactcgcctgtatgaagttggaatcgctagtaatcgcggatcagcatgccgcggtgaatacgttcccgggccttgtacacaccgcccgtcacaccatgagagtcgggaacacccgaagtccgtagcctaaccgcaaggggg

SEQ ID NO: 58 - DNA, 1377 bp, Unknown
  K58
gcaagtcgagcgagaagctttgaactgacgcttcggttgatgatcaaagtggaaagcggcggacgggtgagtaacgcgtaggcaacctgccctttgcagagggatagcctcgggaaaccgggattaaaacctcataacgcacaactgagacatcttggatgtgccaaagatttatcggcagaggatgggcctgcgtctgattagttagttggtggggtaacggcctaccaaggcgacgatcagtagccgacctgagagggtgatcggccacattggaactgagacacggtccaaactcctacgggaggcagcagtggggaatattgcacaatgggggaaaccctgatgcagcaacgccgcgtgaaggatgaaggcccttgggtcgtaaacttctgttctaggggaagatagtgacggtaccttaggagcaagtcccggctaactacgtgccagcagccgcggtaatacgtagggggcaagcgttatccggaattattgggcgtaaagagtacgtaggtggttacctaagcaaggggtttaaggcaatggcttaactattgttcgccccttgaactgggctacttgagtgcaggagaggaaagcggaattcctagtgtagcggtgaaatgcgtagatattaggaggaacaccagtggcgaaggcggctttctggactgtaactgacactgaggtacgaaagcgtggggagcaaacaggattagataccctggtagtccacgccgtaaacgatgagcactaggtgtcggggtcgcaagacttcggtgccgcagttaacgcaataagtgctccgcctggggagtacgttcgcaagaatgaaactcaaaggaattgacggggacccgcacaagcagcggagcatgtggtttaattcgaagcaacgcgaagaaccttaccagggcttgacatcttcctgacagacccttaaacgggtccttcttcggacaggaaagacaggtggtgcatggttgtcgtcagctcgtgtcgtgagatgttgggttaagtcccgcaacgagcgcaacccttgctgttagttgccatcattaagttgggcactctaacgggactgccggggataactcggaggaaggtggggatgacgtcaaatcatcatgccccttatgttctgggctacacacgtgctacaatggccggtacaaagaggaagcgagaccgcgaggtggagcgaatctcaaaagccggtcccagttcggattgcaggctgcaactcgcctgcatgaagtcggagttgctagtaatcgcgaatcagaatgtcgcggtgaatgcgttcccgggtcttgtacacaccgcccgtcacaccatggaagttgggggcgcccgaagttggcaggcaaatat

SEQ ID NO: 59 - DNA, 1373 bp, Unknown
  K59
cgaggggcagcgcggagagtagcaatactttggaggcgaccggcgcacgggtgcgtaacgcgtatgcaacctacctttaacaggggcataacactgagaaattggtactaattccccataacattcgagaaggcatcttcttgggttaaaaactccggtggttaaagatgggcatgcgttgtattagctagttggtgaggtaacggctcaccaaggcgacgatacatagggggactgagaggttaaccccccacattggtactgagacacggaccaaactcctacgggaggcagcagtgaggaatattggtcaatggacgcaagtctgaaccagccatgccgcgtgcaggaagacggctctatgagttgtaaactgcttttgtactagggtaaacgcttctacgtgtaggagtctgaaagtatagtacgaataaggatcggctaactccgtgccagcagccgcggtaatacggaggatccaagcgttatccggatttattgggtttaaagggtgcgtaggcggtttgataagttagaggtgaaataccggggctcaactccggaactgcctctaatactgttgaactagagagtagttgcggtaggcggaatgtatggtgtagcggtgaaatgcttagagatcatacagaacaccgattgcgaaggcagcttaccaaactatatctgacgttgaggcacgaaagcgtggggagcaaacaggattagataccctggtagtccacgcagtaaacgatgataactcgttgtcggcgatacacagtcggtgactaagcgaaagcgataagttatccacctggggagtacgttcgcaagaatgaaactcaaaggaattgacgggggcccgcacaagcggaggaacatgtggtttaattcgatgatacgcgaggaaccttacccgggcttgaaagttagtgacgattctggaaacaggatttcccttcggggcacgaaactaggtgctgcatggttgtcgtcagctcgtgccgtgaggtgtcgggttaagtcccataacgagcgcaacccctaccgttagttgccatcaggtcaagctgggcactctggcgggactgccggtgtaagccgagaggaaggtggggatgacgtcaaatcagcacggcccttacgtccggggctacacacgtgttacaatggtaggtacagagggccgctaccccgcgaggggatgccaatctcgaaagcctatctcagttcggatcggaggctgaaacccgcctccgtgaagttggattcgctagtaatcgcgcatcagccatggcgcggtgaatacgttcccgggccttgtacacaccgcccgtcaagccatggaagctgggggtgcctgaagttcgtga

SEQ ID NO: 60 - DNA, 1384 bp, Unknown
  K60
gtcgaacggagctgttttctctgaagttttcggatggaagagagttcagcttagtggcgaacgggtgagtaacacgtgagcaacctgcctttcagtgggggacaacatttggaaacgaatgctaataccgcataagaccacagtgtcgcatggcacaggggtcaaaggatttatccgctgaaagatgggctcgcgtccgattagctagatggtgaggtaacggcccaccatggcgacgatcggtagccggactgagaggttgaacggccacattgggactgagacacggcccagactcctacgggaggcagcagtggggaatattgcacaatgggggaaaccctgatgcagcgacgccgcgtggaggaagaaggtcttcggattgtaaactcctgtcccaggggacgataatgacggtaccctgggaggaagcaccggctaactacgtgccagcagccgcggtaaaacgtagggtgcaagcgttgtccggaattactgggtgtaaagggagcgcaggcggattggcaagttgggagtgaaatctatgggctcaacccataaattgctttcaaaactgtcagtcttgagtggtgtagaggtaggcggaattcccggtgtagcggtggaatgcgtagatatcgggaggaacaccagtggcgaaggcggcctactgggcactaactgacgctgaggctcgaaagcatgggtagcaaacaggattagataccctggtagtccatgccgtaaacgatgattactaggtgtgggaggattgaccccttccgtgccgcagttaacacaataagtaatccacctggggagtacgaccgcaaggttgaaactcaaaggaattgacgggggcccgcacaagcagtggagtatgtggtttaattcgaagcaacgcgaagaaccttaccaggtcttgacatcggatgcatacctaagagattagggaagtccttcgggacatccagacaggtggtgcatggttgtcgtcagctcgtgtcgtgagatgttgggttaagtcccgcaacgagcgcaacccttatcgttagttactacgcaagaggactctagcgagactgccgttgacaaaacggaggaaggtggggatgacgtcaaatcatcatgccctttatgacctgggctacacacgtactacaatggctattaacagagagaagcgataccgcgaggtggagcaaacctcacaaaaatagtctcagttcggatcgcaggctgcaacccgcctgcgtgaagccggaattgctagtaatcgcggatcagcatgccgcggtgaatacgttcccgggccttgtacacaccgcccgtcacaccatgagagccggggggacccgaagtcggtagtctaaccgcaaggagg

SEQ ID NO: 61 - DNA, 1394 bp, Unknown
  K61
agtcgaacgaagttgctctttgtgaagccctcgggtggaactgcgagtatacttagtggcggacgggtgagtaacgcgtgagcaatctgccctgcaatgggggacaacagttggaaacgactgctaataccgcatgagaccacgaaaccgcatggttttgaggtaaaaggatttattcgatgcaggatgagctcgcgtcccattagatagttggtgaggtaacggcccaccaagtcaacgatgggtagccgacctgagagggtgatcggccacactggaactgagacacggtccagactcctacgggaggcagcagtggggaatattgggcaatgggggaaaccctgacccagcaacgccgcgtgagggaagaaggtcttcggattgtaaacctttgtcctatgggacgaaacaaatgacggtaccataggaggaagctccggctaactacgtgccagcagccgcggtaatacgtagggagcaagcgttgtccggaattactgggcgtaaagggtgcgtaggtggctatgtaagtcagatgtgaaagaccggggcttaaccccggggttgcatttgaaactgtgtggcttgagtacaggagagggaagtggaattcctagtgtagcggtgaaatgcgtagatattaggaggaacaccagtggcgaaggcgactttctggactgtaactgacactgaagcacgaaagcgtggggagcaaacaggattagataccctggtagtccacgccgtaaacgatggatactaggtgtggggcccgatagggttccgtgccgaagctaacgcattaagtatcccgcctggggagtacgatcgcaaggttgaaactcaaaggaattgacgggggcccgcacaagcagcggagcatgtggtttaattcgaagcaacgcgaagaaccttaccaaggcttgacatcctctgacgactgtagagatacagtttcccttcggggcagagagacaggtggtgcatggttgtcgtcagctcgtgtcgtgagatgttgggttaagtcccgcaacgagcgcaacccttattgctagttgccagcgcgtaaaggcgggaactctagtgagactgccggggacaactcggaggaaggtggggacgacgtcaaatcatcatgccccttatgtcttgggctacacacgtgctacaatggccggtacaaagggcagcgaacccgtaaggggaagcgaatctcaaaaagccggtcccagttcggattgtgggctgcaacccgcccacatgaagtcggagttgctagtaatcgcgaatcagcatgtcgcggtgaatgcgttcccgggccttgtacacaccgcccgtcacaccacggaagttgggagcacccgaagccagtggcttaaccgtaaggagag

SEQ ID NO: 62 - DNA, 1388 bp, Unknown
  K62
aacgaagcgcttccgcctgattttcttcggagatgaaggcggctgcgactgagtggcggacgggtgagtaacgcgtgggcaacctgccttgcactgggggataacagccagaaatggctgctaataccgcataagaccgaagcgccgcatggcgctgcggccaaagccccggcggtgcaagatgggcccgcgtctgattaggtagttggcggggtaacggcccaccaagccgacgatcagtagccgacctgagagggtgaccggccacattgggactgagacacggcccagactcctacgggaggcagcagtggggaatattgcacaatgggggaaaccctgatgcagcgacgccgcgtgaaggatgaagtatttcggtatgtaaacttctatcagcagggaagaagatgacggtacctgactaagaagccccggctaactacgtgccagcagccgcggtaatacgtagggggcaagcgttatccggatttactgggtgtaaagggagcgtagacggcgatgcaagccagatgtgaaagcccggggctcaaccccgggactgcatttggaactgcgtggctggagtgtcggagaggcaggcggaattcctagtgtagcggtgaaatgcgtagaatattaggaggaacaccagtggcgaaggcggcctgctggacgatgactgacgttgaggctcgaaagcgtggggagcaaacaggattagataccctggtagtccacgccgtaaacgatgactactaggtgtcgggtggcaaggccattcggtgccgcagcaaacgcaataagtagtccacctgggggagtacgttcgcaagaatgaaactcaaaggaattgacggggacccgcacaagcggtggagcatgtggtttaattcgaagcaacgcgaagaaccttacctgatcttgacatcccgatgccaaagcgcgtaacgcgctctttcttcggaacatcggtgacaggtggtgcatggttgtcgtcagctcgtgtcgtgagatgttgggttaagtcccgcaacgagcgcaacccctatcttcagtagccagcattccggatgggcactctggagagactgccagggacaacctggaggaaggtggggatgacgtcaaatcatcatgccccttatgaccagggctacacacgtgctacaatggcgtaaacaaagggaggcgaacccgcgagggtgggcaaatcccaaaaataacgtctcagttcggattgtagtctgcaactcgactacatgaagctggaatcgctagtaatcgcgaatcagaatgtcgcggtgaatacgttcccgggtcttgtacacaccgcccgtcacaccatgggagtcagtaacgcccgaagccggtgacccaacccgcaaggg

SEQ ID NO: 63 - DNA, 1415 bp, Unknown
  K63
agtcgaacgcttctttcctcccgagtgcttgcactcaattggaaagaggagtggcggacgggtgagtaacacgtgggtaacctacccatcagagggggataacacttggaaacaggtgctaataccgcataacagtttatgccgcatggcataagagtgaaaggcgctttcgggtgtcgctgatggatggacccgcggtgcattagctagttggtgaggtaacggctcaccaaggccacgatgcatagccgacctgagagggtgatcggccacactgggactgagacacggcccagactcctacgggaggcagcagtagggaatcttcggcaatggacgaaagtctgaccgagcaacgccgcgtgagtgaagaaggttttcggatcgtaaaactctgttgttagagaagaacaaggacgttagtaactgaacgtcccctgacggtatctaaccagaaagccacggctaactacgtgccagcagccgcggtaatacgtaggtggcaagcgttgtccggatttattgggcgtaaagcgagcgcaggcggtttcttaagtctgatgtgaaagcccccggctcaaccggggagggtcattggaaactgggagacttgagtgcagaagaggagagtggaattccatgtgtagcggtgaaatgcgtagatatatggaggaacaccagtggcgaaggcggctctctggtctgtaactgacgctgaggctcgaaagcgtggggagcaaacaggattagataccctggtagtccacgccgtaaacgatgagtgctaagtgttggagggtttccgcccttcagtgctgcagcaaacgcattaagcactccgcctggggagtacgaccgcaaggttgaaactcaaaggaattgacgggggcccgcacaagcggtggagcatgtggtttaattcgaagcaacgcgaagaaccttaccaggtcttgacatcctttgaccactctagagatagagctttcccttcggggacaaagtgacaggtggtgcatggttgtcgtcagctcgtgtcgtgagatgttgggttaagtcccgcaacgagcgcaacccttattgttagttgccatcatttagttgggcactctagcgagactgccggtgacaaaccggaggaaggtggggatgacgtcaaatcatcatgccccttatgacctgggctacacacgtgctacaatgggaagtacaacgagtcgctagaccgcgaggtcatgcaaatctcttaaagcttctctcagttcggattgcaggctgcaactcgcctgcatgaagccggaatcgctagtaatcgcggatcagcacgccgcggtgaatacgttcccgggccttgtacacaccgcccgtcacaccacgagagtttgtaacacccgaagtcggtgaggtaacctttttgg

SEQ ID NO: 64 - DNA, 1392 bp, Unknown
  K64
agtcgagcgaagcgctaagacaggatttcttcggattgaagtctttgtgactgagcggcggacgggtgagtaacgcgtgggtaacctgcctcatacagggggataacagttagaaatgactgctaataccgcataagcgcacaggaccgcatggtctggtgtgaaaaactccggtggtatgagatggacccgcgtctgattagctagttggaggggtaacggcccaccaaggcgacgatcagtagccggcctgagagggtgaacggccacattgggactgagacacggcccagactcctacgggaggcagcagtggggaatattgcacaatgggggaaaccctgatgcagcgacgccgcgtgaaggaagaagtatctcggtatgtaaacttctatcagcagggaagaaaatgacggtacctgactaagaagccccggctaactacgtgccagcagccgcggtaatacgtagggggcaagcgttatccggatttactgggtgtaaagggagcgtagacggaagagcaagtctgatgtgaaaggctggggcttaaccccaggactgcattggaaactgttgttctagagtgccggagaggtaagcggaattcctagtgtagcggtgaaatgcgtagatattaggaggaacaccagtggcgaaggcggcttactggacggtaactgacgttgaggctcgaaagcgtggggagcaaacaggattagataccctggtagtccacgccgtaaacgatgaatactaggtgtcgggtggcaaagccattcggtgccgcagcaaacgcaataagtattccacctggggagtacgttcgcaagaatgaaactcaaaggaattgacggggacccgcacaagcggtggagcatgtggtttaattcgaagcaacgcgaagaaccttaccaagtcttgacatccctctgaccgtcccgtaacgggggcttcccttcggggcagaggagacaggtggtgcatggttgtcgtcagctcgtgtcgtgagatgttgggttaagtcccgcaacgagcgcaacccttatccttagtagccagcacatgatggtgggcactctagggagactgccggggataacccggaggaaggcggggacgacgtcaaatcatcatgccccttatgatttgggctacacacgtgctacaatggcgtaaacaaagggaagcgagacagcgatgttgagcgaatcccaaaaataacgtcccagttcggactgcagtctgcaactcgactgcacgaagctggaatcgctagtaatcgcggatcagaatgccgcggtgaatacgttcccgggtcttgtacacaccgcccgtcacaccatgggagtcagtaacgcccgaagtcagtgacctaaccgaaaggaagga

SEQ ID NO: 65 - DNA, 1388 bp, Unknown
  K65
aagtcgaggggcagcggatggagtgcttcggtactcctgccggcgaccggcggacgggtgcgtaacgcgtatgcaacctgccttcaacagggggataatccgaagaaatttggtctaataccccataatattccgacaggcatctgtcggagttgaaagcttcggtggttggagatgggcatgcgttgtattagctggatggtgaggtaacggctcaccatggcgatgatacatagggggactgagaggttttccccccacactggtactgagacacggaccagactcctacgggaggcagcagtgaggaatattggtcaatggacggaagtctgaaccagccatgccgcgtgcaggatgaatgtgctatgcattgtaaactgcttttgtacgagggtaaacccagatacgcgtatctgcttgaaagtatcgtacgaataaggatcggctaactccgtgccagcagccgcggtaatacggaggatccgagcgttatccggatttattgggtttaaagggtgcgtaggctgttttttaagttagaggtgaaagctcgacgctcaacgtcgaaattgcctctgatactgagagactagagtgtagttgcggaaggcggaatgtgtggtgtagcggtgaaatgcttagatatcacacagaacaccgattgcgaaggcagctttccaagctattactgacgctgaggcacgaaagcgtggggagcgaacaggattagataccctggtagtccacgcagtaaacgatgataactcgttgccggcgatacacagtcggtgacttagcgaaagcgttaagttatccacctgggggagtacgttcgcaagaatgaaactcaaaggaattgacgggggcccgcacaagcggaggaacatgtggtttaattcgatgatacgcgaggaaccttacccgggcttgaaagttagcgacggatcgagaaatcggtcttccctacggggcgcgaaactaggtgctgcatggttgtcgtcagctcgtgccgtgaggtgtcgggttaagtcccataacgagcgcaacccctaccgttagttgccatcaggtcaagctgggcactctagcgggactgccggtgtaagccgagaggaaggtggggatgacgtcaaatcagcacggcccttacgtccggggcgacacacgtgttacaatggccggtacagagggtagctacctggtgacaggatgccaatctcgaaagccggtctcagttcggattggaggctgaaactcgcctccatgaagttggattcgctagtaatcgcgcatcagccatggcgcggtgaatacgttcccgggccttgtacacaccgcccgtcaagccatgggagttgggggtgcctgaagtacgtgaccgcaag

SEQ ID NO: 66 - DNA, 1388 bp, Unknown
  K66
gtcgaacggagcacccctgacggagttttcggacaacgaaagggaatgcttagtggcggacgggtgagtaacgcgtgagtaacctgccttggagtggggaataacagccggaaacggctgctaataccgcatgatgtatctggatcgcatggttctggataccaaagatttatcgctctgagatggactcgcgtctgattagctagttggtgaggtaatggctcaccaaggcgacgatcagtagccggactgagaggttggccggccacattgggactgagacacggcccagactcctacgggaggcagcagtggggaatattgggcaatgggcgaaagcctgacccagcaacgccgcgtgaaggaagaaggccctcgggttgtaaacttcttttgtcagggacgaagcaagtgacggtacctgacgaataagccacggctaactacgtgccagcagccgcggtaatacgtaggtggcaagcgttatccggatttactgggtgtaaagggcgtgtaggcgggagtgcaagtcagatgtgaaaactatgggctcaacccatagcctgcatttgaaactgtacttcttgagtgatggagaggcaggcggaattccctgtgtagcggtgaaatgcgtagatatagggaggaacaccagtggcgaaggcggcctgctggacattaactgacgctgaggcgcgaaagcgtggggagcaaacaggattagataccctggtagtccacgccgtaaacgatggatactaggtgtggggggtctgaccccctccgtgccgcagttaacacaataagtatcccacctggggagtacgatcgcaaggttgaaactcaaaggaattgacgggggcccgcacaagcggtggagtatgtggtttaattcgaagcaacgcgaagaaccttaccaggacttgacatcctactaacgaagcagagatgcataaggtgcccttcggggaaagtagagacaggtggtgcatggttgtcgtcagctcgtgtcgtgagatgttgggttaagtcccgcaacgagcgcaacccttattgttagttgctacgcaagagcactctagcgagactgccgttgacaaaacggaggaaggtggggacgacgtcaaatcatcatgccccttatgtcctgggccacacacgtactacaatggcggtcaacagagggaagcaaagccgcgaggtggagcaaatccctaaaagccgtcccagttcggattgcaggctgaaactcgcctgtatgaagtcggaatcgctagtaatcgcggatcagcatgccgcggtgaatacgttcccgggccttgtacacaccgcccgtcacaccatgagagtcgggaacacccgaagtccgtagcctaacagcaatgggg

SEQ ID NO: 67 - DNA, 1380 bp, Unknown
  K67
tcgaggggcagcatgaacttagcttgctaagtttgatggcgaccggcgcacgggtgagtaacacgtatccaacctgccgatgactcggggatagcctttcgaaagaaagattaatacccgatggcataattcttccgcatggtagaactattaaagaatttcggtcatcgatggggatgcgttccattaggttgttggcggggtaacggcccaccaagccttcgatggataggggttctgagaggaaggtcccccacattggaactgagacacggtccaaactcctacgggaggcagcagtgaggaatattggtcaatggacgagagtctgaaccagccaagtagcgtgaaggatgactgccctatgggttgtaaacttcttttatacgggaataaagtgaggcacgtgtgcctttttgtatgtaccgtatgaataaggatcggctaactccgtgccagcagccgcggtaatacggaggatccgagcgttatccggatttattgggtttaaagggagcgtaggcggacgcttaagtcagttgtgaaagtttgcggctcaaccgtaaaattgcagttgatactgggtgtcttgagtacagtagaggcaggcggaattcgtggtgtagcggtgaaatgcttagatatcacgaagaactccgattgcgaaggcagcttgctggactgtaactgacgctgatgctcgaaagtgtgggtatcaaacaggattagataccctggtagtccacacagtaaacgatgaatactcgctgtttgcgatatacagtaagcggccaagcgaaagcgttaagtattccacctggggagtacgccggcaacggtgaaactcaaaggaattgacgggggcccgcacaagcggaggaacatgtggtttaattcgatgatacgcgaggaaccttacccgggcttgaattgcaactgaatgatgtggagacatgtcagccgcaaggcagttgtgaaggtgctgcatggttgtcgtcagctcgtgccgtgaggtgtcggcttaagtgccataacgagcgcaacccttatcgatagttaccatcaggttatgctggggactctgtcgagactgccgtcgtaagatgtgaggaaggtggggatgacgtcaaatcagcacggcccttacgtccggggctacacacgtgttacaatggggggtacagaaggcagctacacggcgacgtgatgctaatccctaaagcctctctcagttcggattggagtctgcaacccgactccatgaagctggattcgctagtaatcgcgcatcagccacggcgcggtgaatacgttcccgggccttgtacacaccgcccgtcaagccatgaaagccgggggtacctgaagtgcgtaaccgca

SEQ ID NO: 68 - DNA, 1370 bp, Unknown
  K68
  misc_feature (6)..(6): n is a, c, g, or t
  misc_feature (1352)..(1352): n is a, c, g, or t
agtcgnacgagagaattgctagcttgctaataattctctagtggcgcacgggtgagtaacacgtgagtaacctgcccccaagagtgggatagccccgggaaactgggattaataccgcataaaatcgcaagattaaagcagcaatgcgcttggggatgggctcgcgtcctattagttagttggtgaggtaacggctcaccaaggcgatgacgggtagccggtctgagaggatgtccggccacactggaactgagacacggtccagacacctacgggtggcagcagtcgagaatcattcacaatgggggaaaccctgatggtgcgacgccgcgtgggggaatgaaggtcttcggattgtaaacccctgtcatgtgggagcaaattaaaaagatagtaccacaagaggaagagacggctaactctgtgccagcagccgcggtaatacagaggtctcaagcgttgttcggaatcactgggcgtaaagcgtgcgtaggcggtttcgtaagtcgtgtgtgaaaggcgggggctcaacccccggactgcacatgatactgcgagactagagtaatggagggggaaccggaattctcggtgtagcagtgaaatgcgtagatatcgagaggaacactcgtggcgaaggcgggttcctggacattaactgacgctgaggcacgaaggccaggggagcgaaagggattagatacccctgtagtcctggcagtaaacggtgcacgcttggtgtgcggggaatcgaccccctgcgtgccggagctaacgcgttaagcgtgccgcctgggggagtacggtcgcaagattaaaactcaaagaaattgacggggacccgcacaagcggtggagtatgtggcttaattcgatgcaacgcgaagaaccttacctgggcttgacatgtaatgaacaacatgtgaaagcatgcgactcttcggaggcgttacacaggtgctgcatggccgtcgtcagctcgtgtcgtgagatgtttggttaagtccagcaacgagcgcaacccctgttgccagttaccagcacgtaaaggtggggactctggcgagactgcccagatcaactgggaggaaggtggggacgacgtcaggtcagtatggcccttatgcccagggctgcacacgtactacaatgcccagtacagagggggccgaagccgcgaggcggaggaaatcctaaaaactgggcccagttcggactgtaggctgcaacccgcctacacgaagccggaatcgctagtaatggcgcatcagctacggcgccgtgaatacgttcccgggtcttgtacacaccgcccgtcacatcatggaagccggtcgcacccgaagtatctnaagccaaccgcaaggagg

SEQ ID NO: 69 - DNA, 1514 bp, Unknown
  F01
agggttcgattctggctcaggatgaacgctggcggcgtgcttaacacatgcaagtcgaacgggatccatcaggctttgcttggtggtgagagtggcgaacgggtgagtaatgcgtgaccgacctgccccatacaccggaatagctcctggaaacgggtggtaatgccggatgctccagttgatcgcatggtcttctgggaaagctttcgcggtatgggatggggtcgcgtcctatcagcttgacggcggggtaacggcccaccgtggcttcgacgggtagccggcctgagagggcgaccggccacattgggactgagatacggcccagactcctacgggaggcagcagtggggaatattgcacaatgggcgcaagcctgatgcagcgacgccgcgtgagggatggaggccttcgggttgtaaacctcttttatcggggagcaagcgagagtgagtttacccgttgaataagcaccggctaactacgtgccagcagccgcggtaatacgtagggtgcaagcgttatccggaattattgggcgtaaagggctcgtaggcggttcgtcgcgtccggtgtgaaagtccatcgcttaacggtggatccgcgccgggtacgggcgggcttgagtgcggtaggggagactggaattcccggtgtaacggtggaatgtgtagatatcgggaagaacaccaatggcgaaggcaggtctctgggccgttactgacgctgaggagcgaaagcgtggggagcgaacaggattagataccctggtagtccacgccgtaaacggtggatgctggatgtggggcccgttccacgggttccgtgtcggagctaacgcgttaagcatcccgcctggggagtacggccgcaaggctaaaactcaaagaaattgacgggggcccgcacaagcggcggagcatgcggattaattcgatgcaacgcgaagaaccttacctgggcttgacatgttcccgacggtcgtagagatacggcttcccttcggggcgggttcacaggtggtgcatggtcgtcgtcagctcgtgtcgtgagatgttgggttaagtcccgcaacgagcgcaaccctcgccccgtgttgccagcggattatgccgggaactcacgggggaccgccggggttaactcggaggaaggtggggatgacgtcagatcatcatgccccttacgtccagggcttcacgcatgctacaatggccggtacaacgggatgcgacgcggcgacgcggagcggatccctgaaaaccggtctcagttcggatcgcagtctgcaactcgactgcgtgaaggcggagtcgctagtaatcgcgaatcagcaacgtcgcggtgaatgcgttcccgggccttgtacacaccgcccgtcaagtcatgaaagtgggcagcacccgaagccggtggcctaaccccttgtgggatggagccgtctaaggtgaggctcgtgattgggactaagtcgtaacaaggtagccgtaccggaaggtgcggctggatcacct

SEQ ID NO: 70 - DNA, 1517 bp, Unknown
  F02
agagtttgatcctggctcaggatgaacgctagctacaggcttaacacatgcaagtcgaggggcagcattttagtttgcttgcaaactaaagatggcgaccggcgcacgggtgagtaacacgtatccaacctgccgataactcggggatagcctttcgaaagaaagattaatatccgatagtatattaaaaccgcatggttttactattaaagaatttcggttatcgatggggatgcgttccattagtttgttggcggggtaacggcccaccaagactacgatggataggggttctgagaggaaggtcccccacattggaactgagacacggtccaaactcctacgggaggcagcagtgaggaatattggtcaatggacgagagtctgaaccagccaagtagcgtgaaggatgactgccctatgggttgtaaacttcttttatatgggaataaagtattccacgtgtgggattttgtatgtaccatatgaataaggatcggctaactccgtgccagcagccgcggtaatacggaggatccgagcgttatccggatttattgggtttaaagggagcgtaggtggattgttaagtcagttgtgaaagtttgcggctcaaccgtaaaattgcagttgaaactggcagtcttgagtacagtagaggtgggcggaattcgtggtgtagcggtgaaatgcttagatatcacgaagaactccgattgcgaaggcagctcactagactgcaactgacactgatgctcgaaagtgtgggtatcaaacaggattagataccctggtagtccacacagtaaacgatgaatactcgctgtttgcgatatacagtaagcggccaagcgaaagcattaagtattccacctggggagtacgccggcaacggtgaaactcaaaggaattgacgggggcccgcacaagcggaggaacatgtggtttaattcgatgatacgcgaggaaccttacccgggcttaaattgcatttgaataatctggaaacaggttagccgcaaggcaaatgtgaaggtgctgcatggttgtcgtcagctcgtgccgtgaggtgtcggcttaagtgccataacgagcgcaacccttatctttagttactaacaggtcatgctgaggactctagagagactgccgtcgtaagatgtgaggaaggtggggatgacgtcaaatcagcacggcccttacgtccggggctacacacgtgttacaatggggggtacagaaggcagctacctggcgacaggatgctaatcccaaaaacctctctcagttcggatcgaagtctgcaacccgacttcgtgaagctggattcgctagtaatcgcgcatcagccatggcgcggtgaatacgttcccgggccttgtacacaccgcccgtcaagccatgaaagccgggggtacctgaagtacgtaaccgcaaggagcgtcctagggtaaaactggtaattggggctaagtcgtaacaaggtagccgtaccggaaggtgcggctggaacacct

SEQ ID NO: 71 - DNA, 1517 bp, Unknown
  F03
agagtttgatcctggctcaggatgaacgctagctacaggcttaacacatgcaagtcgaggggcatcaggaagaaagcttgctttctttgctggcgaccggcgcacgggtgagtaacacgtatccaacctgccctttactcggggatagcctttcgaaagaaagattaatacccgatggtataattattccgcatggtttgattattaaaggattccggtaaaggatggggatgcgttccattaggttgttggtgaggtaacggctcaccaagccttcgatggataggggttctgagaggaaggtcccccacattggaactgagacacggtccaaactcctacgggaggcagcagtgaggaatattggtcaatgggcgatggcctgaaccagccaagtagcgtgaaggatgaaggctctatgggtcgtaaacttcttttatattagaataaagtgcagtatgtatactgttttgtatgtataatatgaataaggatcggctaactccgtgccagcagccgcggtaatacggaggatccgagcgttatccggatttattgggtttaaagggagcgtaggtggactggtaagtcagttgtgaaagtttgcggctcaaccgtaaaattgcagttgatactgtcagtcttgagtacagtagaggtgggcggaattcgtggtgtagcggtgaaatgcttagatatcacgaagaactccgattgcgaaggcagctcactggactgcaactgacactgatgctcgaaagtgtgggtatcaaacaggattagataccctggtagtccacacagtaaacgatgaatactcgctgtttgcgatatacagtaagcggccaagcgaaagcattaagtattccacctggggagtacgccggcaacggtgaaactcaaaggaattgacgggggcccgcacaagcggaggaacatgtggtttaattcgatgatacgcgaggaaccttacccgggcttaaattgcagtggaatgatgtggaaacatgtcagtgagcaatcaccgctgtgaaggtgctgcatggttgtcgtcagctcgtgccgtgaggtgtcggcttaagtgccataacgagcgcaacccttatctttagttactaacaggtcatgctgaggactctggagagactgccgtcgtaagatgtgaggaaggtggggatgacgtcaaatcagcacggcccttacgtccggggctacacacgtgttacaatggggggtacagaaggcagctacctggtgacaggatgctaatcccaaaagcctctctcagttcggatcgaagtctgcaacccgacttcgtgaagctggattcgctagtaatcgcgcatcagccacggcgcggtgaatacgttcccgggccttgtacacaccgcccgtcaagccatgggagccgggggtacctgaagtacgtaaccgcaaggagcgtcctagggtaaaactggtgactggggctaagtcgtaacaaggtagccgtaccggaaggtgcggctggaacacct

SEQ ID NO: 72 - DNA, 1515 bp, Unknown
  F04
agagtttgatcctggctcaggatgaacgctagctacaggcttaacacatgcaagtcgaggggcagcatgaacttagcttgctaagtttgatggcgaccggcgcacgggtgagtaacacgtatccaacctgccgatgactcggggatagcctttcgaaagaaagattaatacccgatggcatagttcttccgcatggtagaactattaaagaatttcggtcatcgatggggatgcgttccattaggttgttggcggggtaacggcccaccaagccttcgatggataggggttctgagaggaaggtcccccacattggaactgagacacggtccaaactcctacgggaggcagcagtgaggaatattggtcaatggacgagagtctgaaccagccaagtagcgtgaaggatgactgccctatgggttgtaaacttcttttatacgggaataaagtgaggcacgtgtgcctttttgtatgtaccgtatgaataaggatcggctaactccgtgccagcagccgcggtaatacggaggatccgagcgttatccggatttattgggtttaaagggagcgtaggcggacgcttaagtcagttgtgaaagtttgcggctcaaccgtaaaattgcagttgatactgggtgtcttgagtacagtagaggcaggcggaattcgtggtgtagcggtgaaatgcttagatatcacgaagaactccgattgcgaaggcagcttgctggactgtaactgacgctgatgctcgaaagtgtgggtatcaaacaggattagataccctggtagtccacacagtaaacgatgaatactcgctgtttgcgatatacagtaagcggccaagcgaaagcgttaagtattccacctggggagtacgccggcaacggtgaaactcaaaggaattgacgggggcccgcacaagcggaggaacatgtggtttaattcgatgatacgcgaggaaccttacccgggcttgaattgcaactgaatgatgtggagacatgtcagccgcaaggcagttgtgaaggtgctgcatggttgtcgtcagctcgtgccgtgaggtgtcggcttaagtgccataacgagcgcaacccttatcgatagttaccatcaggttatgctggggactctgtcgagactgccgtcgtaagatgtgaggaaggtggggatgacgtcaaatcagcacggcccttacgtccggggctacacacgtgttacaatggggggtacagaaggcagctacacggcgacgtgatgctaatcccgaaagcctctctcagttcggattggagtctgcaacccgactccatgaagctggattcgctagtaatcgcgcatcagccacggcgcggtgaatacgttcccgggccttgtacacaccgcccgtcaagccatgaaagccgggggtacctgaagtgcgtaaccgcaaggagcgccctagggtaaaactggtgattggggctaagtcgtaacaaggtagccgtaccggaaggtgcggctggaacacct

SEQ ID NO: 73 - DNA, 1517 bp, Unknown
  F05
agagtttgatcctggctcaggatgaacgctagctacaggcttaacacatgcaagtcgaggggcagcatttcagtttgcttgcaaactggagatggcgaccggcgcacgggtgagtaacacgtatccaacctgccgataactcggggatagcctttcgaaagaaagattaatacccgatggtataatcagaccgcatggtcttgttattaaagaatttcggttatcgatggggatgcgttccattaggcagttggtgaggtaacggctcaccaaaccttcgatggataggggttctgagaggaaggtcccccacattggaactgagacacggtccaaactcctacgggaggcagcagtgaggaatattggtcaatgggcgcaggcctgaaccagccaagtagcgtgaaggatgactgccctatgggttgtaaacttcttttatatgggaataaagttttccacgtgtggaattttgtatgtaccatatgaataaggatcggctaactccgtgccagcagccgcggtaatacggaggatccgagcgttatccggatttattgggtttaaagggagcgtaggtggacagttaagtcagttgtgaaagtttgcggctcaaccgtaaaattgcagttgatactggctgtcttgagtacagtagaggtgggcggaattcgtggtgtagcggtgaaatgcttagatatcacgaagaactccgattgcgaaggcagctcactggactgcaactgacactgatgctcgaaagtgtgggtatcaaacaggattagataccctggtagtccacacagtaaacgatgaatactcgctgtttgcgatatacagtaagcggccaagcgaaagcattaagtattccacctggggagtacgccggcaacggtgaaactcaaaggaattgacgggggcccgcacaagcggaggaacatgtggtttaattcgatgatacgcgaggaaccttacccgggcttaaattgcatttgaatatattggaaacagtatagccgtaaggcaaatgtgaaggtgctgcatggttgtcgtcagctcgtgccgtgaggtgtcggcttaagtgccataacgagcgcaacccttatctttagttactaacaggtcatgctgaggactctagagagactgccgtcgtaagatgtgaggaaggtggggatgacgtcaaatcagcacggcccttacgtccggggctacacacgtgttacaatggggggtacagaaggcagctacctggtgacaggatgctaatcccaaaagcctctctcagttcggatcgaagtctgcaacccgacttcgtgaagctggattcgctagtaatcgcgcatcagccatggcgcggtgaatacgttcccgggccttgtacacaccgcccgtcaagccatgaaagccgggggtacctgaagtacgtaaccgcaaggagcgtcctagggtaaaactggtaattggggctaagtcgtaacaaggtagccgtaccggaaggtgcggctggaacacct

SEQ ID NO: 74 - DNA, 1515 bp, Unknown; identical to SEQ ID NO: 72
  F06

SEQ ID NO: 75 - DNA, 1518 bp, Unknown
  F07
agagtttgatcctggctcaggatgaacgctagctacaggcttaacacatgcaagtcgaggggcagcatttcagtttgcttgcaaactggagatggcgaccggcgcacgggtgagtaacacgtatccaacctgccgataactcggggatagcctttcgaaagaaagattaatatccgatggtatatttctcccgcatgagagagatattaaagaatttcggttatcgatggggatgcgttccattagtttgttggcggggtaacggcccaccaagactacgatggataggggttctgagaggaaggtcccccacattggaactgagacacggtccaaactcctacgggaggcagcagtgaggaatattggtcaatggacgagagtctgaaccagccaagtagcgtgaaggatgactgccctatgggttgtaaacttcttttatatgggaataaaatgttccacgtgtgggattttgtatgtaccatatgaataaggatcggctaactccgtgccagcagccgcggtaatacggaggatccgagcgttatccggatttattgggtttaaagggagcgtaggtggattgttaagtcagttgtgaaagtttgcggctcaaccgtaaaattgcagttgaaactggcagtcttgagtacagtagaggtgggcggaattcgtggtgtagcggtgaaatgcttagatatcacgaagaactccgattgcgaaggcagctcactagactggtcactgacactgaggctcgaaagtgtgggtatcaaacaggattagataccctggtagtccacacagtaaacgatgaatactcgctgtttgcgatatacagcaagcggccaagcgaaagcattaagtattccacctggggagtacgccggcaacggtgaaactcaaaggaattgacgggggcccgcacaagcggaggaacatgtggtttaattcgatgatacgcgaggaaccttacccgggcttaaattgcatttgaatatagtggaaacattatagccgcaaggcaaatgtgaaggtgctgcatggttgtcgtcagctcgtgccgtgaggtgtcggcttaagtgccataacgagcgcaacccttatcttcagttactaacaggtcatgctgaggactctggagagactgccgtcgtaagatgtgaggaaggtggggatgacgtcaaatcagcacggcccttacgtccggggctacacacgtgttacaatggggggtacagaaggccgctacctggtgacaggatgccaatcccaaaaacctctctcagttcggatcgaagtctgcaacccgacttcgtgaagctggattcgctagtaatcgcgcatcagccatggcgcggtgaatacgttcccgggccttgtacacaccgcccgtcaagccatgaaagccgggggtacctgaagtacgtaaccgcaaggagcgtcctagggtaaaactggtaattggggctaagtcgtaacaaggtagccgtaccggaaggtgcggctggaacacct

SEQ ID NO: 76 - DNA, 1517 bp, Unknown; identical to SEQ ID NO: 71
  F08

SEQ ID NO: 77 - DNA, 1515 bp, Unknown
  F09
agagtttgatcctggctcaggatgaacgctagcgacaggcttaacacatgcaagtcgaggggcagcacgatgtagcaatacattggtggcgaccggcgcacgggtgagtaacgcgtatgcaacctacctatcagaggggaataacccggcgaaagtcggactaataccgcataaaacaggggttccacatggaaatatttgttaaagaattatcgctgatagatgggcatgcgttccattagatagttggtgaggtaacggctcaccaagtccacgatggataggggttctgagaggaaggtcccccacactggtactgagacacggaccagactcctacgggaggcagcagtgaggaatattggtcaatgggcgagagcctgaaccagccaagtcgcgtgaaggatgaaggatctatggtttgtaaacttcttttatatgggaataaagtgaggaacgtgttcctttttgtatgtaccatatgaataagcatcggctaactccgtgccagcagccgcggtaatacggaggatgcgagcgttatccggatttattgggtttaaagggtgcgtaggtggttaattaagtcagcggtgaaagtttgtggctcaaccataaaattgccgttgaaactggttgacttgagtatatttgaggtaggcggaatgcgtggtgtagcggtgaaatgcatagatatcacgcagaactccgattgcgaaggcagcttactaaactataactgacactgaagcacgaaagcgtggggatcaaacaggattagataccctggtagtccacgcagtaaacgatgattactagctgtttgcgatacacagtaagcggcacagcgaaagcgttaagtaatccacctggggagtacgccggcaacggtgaaactcaaaggaattgacgggggcccgcacaagcggaggaacatgtggtttaattcgatgatacgcgaggaaccttacccgggtttgaacgcattcggaccggagtggaaacacttcttctagcaatagccgtttgcgaggtgctgcatggttgtcgtcagctcgtgccgtgaggtgtcggcttaagtgccataacgagcgcaacccttatcactagttactaacaggtcatgctgaggactctagtgagactgccagcgtaagctgtgaggaaggtggggatgacgtcaaatcagcacggcccttacatccggggcgacacacgtgttacaatggtggggacaaagggcagctaccgtgtgagcggatgctaatctccaaaccccatctcagttcggatcgaagtctgcaacccgacttcgtgaagctggattcgctagtaatcgcgcatcagccatggcgcggtgaatacgttcccgggccttgtacacaccgcccgtcaagccatgggagttgggggtacctaaagtccgtaaccgcaaggatcggcctagggtaaaaccgatgactggggctaagtcgtaacaaggtagccgtaccggaaggtgcggctggaacacct

SEQ ID NO: 78 - DNA, 1519 bp, Unknown
  F10
agagtttgatcctggctcaggatgaacgctggcggcgtgcttaacacatgcaagtcgagcgaagcaccttgacggatttcttcggattgaagccttggtgactgagcggcggacgggtgagtaacgcgtgggtaacctgcctcatacagggggataacagttggaaacggctgctaataccgcataagcgcacagtaccgcatggtacggtgtgaaaaactccggtggtatgagatggacccgcgtctgattaggtagttggtggggtaacggcctaccaagccgacgatcagtagccgacctgagagggtgaccggccacattgggactgagacacggcccaaactcctacgggaggcagcagtggggaatattgcacaatgggggaaaccctgatgcagcgacgccgcgtgagcgatgaagtatttcggtatgtaaagctctatcagcagggaagaaaatgacggtacctgactaagaagccccggctaactacgtgccagcagccgcggtaatacgtagggggcaagcgttatccggatttactgggtgtaaagggagcgtagacggcatggcaagccagatgtgaaagcccggggctcaaccccgggactgcatttggaactgtcaggctagagtgtcggagaggaaagcggaattcctagtgtagcggtgaaatgcgtagatattaggaggaacaccagtggcgaaggcggctttctggacgatgactgacgttgaggctcgaaagcgtggggagcaaacaggattagataccctggtagtccacgccgtaaacgatgaatactaggtgtcgggtggcaaagccattcggtgccgcagcaaacgcaataagtattccacctggggagtacgttcgcaagaatgaaactcaaaggaattgacggggacccgcacaagcggtggagcatgtggtttaattcgaagcaacgcgaagaaccttacctggtcttgacatccctctgaccgctctttaatcggagctttccttcgggacagaggagacaggtggtgcatggttgtcgtcagctcgtgtcgtgagatgttgggttaagtcccgcaacgagcgcaacccctatctttagtagccagcattttggatgggcactctagagagactgccagggataacctggaggaaggtggggatgacgtcaaatcatcatgccccttatgaccagggctacacacgtgctacaatggcgtaaacaaagggaagcgagcccgcgagggggagcaaatcccaaaaataacgtctcagttcggattgtagtctgcaactcgactacatgaagctggaatcgctagtaatcgcgaatcagaatgtcgcggtgaatacgttcccgggtcttgtacacaccgcccgtcacaccatgggagtcagtaacgcccgaagtcagtgacccaaccgcaaggagggagctgccgaaggtgggaccgataactggggtgaagtcgtaacaaggtagccgtatcggaaggtgcggctggatcacct

SEQ ID NO: 79 - DNA, 1519 bp, Unknown
  F11
agagtttgatcctggctcaggatgaacgctggcggcgtgcttaacacatgcaagtcgaacgggaatcacttcattgagacttcggtggatttgatttgattctagtggcggacgggtgagtaacgcgtgggtaacctgccttatacagggggataacagtcagaaatgactgctaataccgcataagcgcacaggaccgcatggtccggtgtgaaaaactccggtggtataagatggacccgcgttggattagcttgttggtggggtaacggcccaccaaggcgacgatccatagccggcctgagagggtgaacggccacattgggactgagacacggcccagactcctacgggaggcagcagtggggaatattgcacaatgggggaaaccctgatgcagcgacgccgcgtgaaggaagaagtatctcggtatgtaaacttctatcagcagggaagatagtgacggtacctgactaagaagccccggctaactacgtgccagcagccgcggtaatacgtagggggcaagcgttatccggatttactgggtgtaaagggagcgtagacggtgtggcaagtctgatgtgaaaggcatgggctcaacctgtggactgcattggaaactgtcatacttgagtgccggaggggtaagcggaattcctagtgtagcggtgaaatgcgtagatattaggaggaacaccagtggcgaaggcggcttactggacggtaactgacgttgaggctcgaaagcgtggggagcaaacaggattagataccctggtagtccacgccgtaaacgatgaatactaggtgtcgggtggcatggccattcggtgccgtcgcaaacgcagtaagtattccacctggggagtacgttcgcaagaatgaaactcaaaggaattgacggggacccgcacaagcggtggagcatgtggtttaattcgaagcaacgcgaagaaccttaccaagtcttgacatccctctgaccgactcttaaccgagtctttccttcgggacagaggagacaggtggtgcatggttgtcgtcagctcgtgtcgtgagatgttgggttaagtcccgcaacgagcgcaacccctatcctcagtagccagcaagttaagttgggcactctgtggagactgccagggataacctggaggaaggcggggatgacgtcaaatcatcatgccccttatgatttgggctacacacgtgctacaatggcgtaaacaaagggaagcgagattgtgagatggagcaaatcccaaaaataacgtcccagttcggactgtagtctgcaacccgactacacgaagctggaatcgctagtaatcgcggatcagaatgccgcggtgaatacgttcccgggtcttgtacacaccgcccgtcacaccatgggagtcagtaacgcccgaagtcagtgacctaactgcaaagaaggagctgccgaaggcgggaccgatgactggggtgaagtcgtaacaaggtagccgtatcggaaggtgcggctggatcacct

SEQ ID NO: 80 - DNA, 1519 bp, Unknown
  F12
agagtttgatcctggctcaggatgaacgctggcggcgtgcttaacacatgcaagtcgaacgaagcacttgaatggaattcttcggaaggaagctcaagtgactgagtggcggacgggtgagtaacgcgtgggtaacctgcctcatacagggggataacagttagaaatgactgctaataccgcataagcacacgtgatcgcatgatcgagtgtgaaaaactccggtggtatgagatggacccgcgtctgattagctagttggtggggtaatggcccaccaaggcgacgatcagtagccggcctgagagggtgaacggccacattgggactgagacacggcccaaactcctacgggaggcagcagtggggaatattgcacaatgggggaaaccctgatgcagcgacgccgcgtgaaggatgaagtatttcggtatgtaaacttctatcagcagggaagaaaatgacggtacctgactaagaagccccggctaactacgtgccagcagccgcggtaatacgtagggggcaagcgttatccggatttactgggtgtaaagggagcgtagacggcagtgcaagtctgaagtgaaagcccggggctcaaccccgggactgctttggaaactgtgcagctagagtgtcggagaggcaagcggaattcctagtgtagcggtgaaatgcgtagatattaggaggaacaccagtggcgaaggcggcttgctggacgatgactgacgttgaggctcgaaagcgtggggagcaaacaggattagataccctggtagtccacgccgtaaacgatgactactaggtgtcggggagcaaagctcttcggtgccgcagccaacgcaataagtagtccacctggggagtacgttcgcaagaatgaaactcaaaggaattgacggggacccgcacaagcggtggagcatgtggtttaattcgaagcaacgcgaagaaccttacctgctcttgacatccctctgaccgctctttaatcggagctttccttcgggacagaggagacaggtggtgcatggttgtcgtcagctcgtgtcgtgagatgttgggttaagtcccgcaacgagcgcaacccctatcttcagtagccagcggcaaggccgggcactctggagagactgccagggataacctggaggaaggtggggatgacgtcaaatcatcatgccccttatgagcagggctacacacgtgctacaatggcgtaaacaaagggaagcagagtcgtgaggccgagcaaatcccaaaaataacgtctcagttcggattgtagtctgcaactcgactacatgaagctggaatcgctagtaatcgcgaatcagaatgtcgcggtgaatacgttcccgggtcttgtacacaccgcccgtcacaccatgggagtcagtaacgcccgaagtcagtgacccaaccgcaaggagggagctgccgaaggtgggaccgataactggggtgaagtcgtaacaaggtagccgtatcggaaggtgcggctggatcacct

SEQ ID NO: 81 - DNA, 1518 bp, Unknown
  F13
agagtttgatcctggctcaggatgaacgctggcggcgtgcctaacacatgcaagtcgagcgaagcggtctggaggaagttttcggatggaatccggattgactgagcggcggacgggtgagtaacgcgtgggtaacctgcctcatacagggggataacagttagaaatggctgctaataccgcataagcgcacagcttcgcatggagcagtgtgaaaaactccggtggtatgagatggacccgcgtctgattagctggttggtaaggtaacggcttaccaaggcgacgatcagtagccgacctgagagggtgaccggccacattgggactgagacacggcccaaactcctacgggaggcagcagtggggaatattgcacaatgggggaaaccctgatgcagcgacgccgcgtgagtgaagaagtatttcggtatgtaaagctctatcagcagggaagaaaatgacggtacctgactaagaagccccggctaactacgtgccagcagccgcggtaatacgtagggggcaagcgttatccggatttactgggtgtaaagggagcgtagacggcatagcaagtctggagtgaaagcccggggctcaaccccggtactgctttggaaactgttaagctagagtgctggagaggtaagtggaattcctagtgtagcggtgaaatgcgtagatattaggaggaacaccagtggcgaaggcggcttactggacagtaactgacgttgaggctcgaaagcgtggggagcaaacaggattagataccctggtagtccacgccgtaaacgatgaatactaggtgttggtgggcaaagcccatcggtgccgccgcaaacgcaataagtattccacctggggagtacgttcgcaagaatgaaactcaaaggaattgacggggacccgcacaagcggtggagcatgtggtttaattcgaagcaacgcgaagaaccttaccaagtcttgacatcggaatgaccgggaagtaatgttcccttctctacggagcattctagacaggtggtgcatggttgtcgtcagctcgtgtcgtgagatgttgggttaagtcccgcaacgagcgcaacccttatccttagtagccagcagtaagatgggcactctagggagactgccagggataacctggaggaaggtggggatgacgtcaaatcatcatgccccttatgatttgggctacacacgtgctacaatggcgtaaacaaagagaggcgagcctgcgagggggagcgaatctcaaaaataacgtcccagttcggactgtagtctgcaacccgactacacgaagctggaatcgctagtaatcgcgaatcagaatgtcgcggtgaatacgttcccgggtcttgtacacaccgcccgtcacaccatgggagtcagcaacgcccgaagtcagtgactcaaccgaaaggggagagctgccgaaggcggggcaggtaactggggtgaagtcgtaacaaggtagccgtatcggaaggtgcggctggatcacct

SEQ ID NO: 82 - DNA, 1519 bp, Unknown
  F14
agagtttgatcctggctcaggatgaacgctggcggcgtgcttaacacatgcaagtcgaacgaagcgcttaaacggatttcttcggattgaagtttttgtgactgagtggcggacgggtgagtaacgcgtgggtaacctgcctcatacagggggataacagttagaaatgactgctaataccgcataagcgcacagtgctgcatggcacagtgtgaaaaactccggtggtatgagatggacccgcgtctgattagctagttggtggggtaacggcctaccaaggcgacgatcagtagccggcctgagagggtgaacggccacattgggactgagacacggcccaaactcctacgggaggcagcagtggggaatattgcacaatgggggaaaccctgatgcagcgacgccgcgtgagcgaagaagtatttcggtatgtaaagctctatcagcagggaagaaaatgacggtacctgactaagaagcaccggctaaatacgtgccagcagccgcggtaatacgtatggtgcaagcgttatccggatttactgggtgtaaagggagcgtagacggttgtgtaagtctgatgtgaaagcccggggctcaaccccgggactgcattggaaactatgtaactagagtgtcggagaggtaagcggaattcctagtgtagcggtgaaatgcgtagatattaggaggaacaccagtggcgaaggcggcttactggacgatcactgacgttgaggctcgaaagcgtggggagcaaacaggattagataccctggtagtccacgccgtaaacgatgactactaggtgtcggggagcaaagctcttcggtgccgcagcaaacgcaataagtagtccacctggggagtacgttcgcaagaatgaaactcaaaggaattgacggggacccgcacaagcggtggagcatgtggtttaattcgaagcaacgcgaagaaccttacctggtcttgacatcccggtgaccggcaagtaatgttgcctttccttcgggacaccggtgacaggtggtgcatggttgtcgtcagctcgtgtcgtgagatgttgggttaagtcccgcaacgagcgcaacccctatcttcagtagccagcatttaaggtgggcactctggagagactgccagggataacctggaggaaggtggggatgacgtcaaatcatcatgccccttatgaccagggctacacacgtgctacaatggcgtaaacaaagggaagcgaacctgtgaggggaagcaaatctcaaaaataacgtctcagttcggattgtagtctgcaactcgactacatgaagctggaatcgctagtaatcgcgaatcagcatgtcgcggtgaatacgttcccgggtcttgtacacaccgcccgtcacaccatgggagtcagtaacgcccgaagtcagtgacccaaccgtaaggagggagctgccgaaggtgggaccgataactggggtgaagtcgtaacaaggtagccgtatcggaaggtgcggctggatcacct

SEQ ID NO: 83 - DNA, 1519 bp, Unknown; identical to SEQ ID NO: 78
  F15

SEQ ID NO: 84 - DNA, 1521 bp, Unknown
  F16
agagtttgatcctggctcaggatgaacgctggcggcgtgcttaacacatgcaagtcgaacgaaacaccttatttgattttcttcggaactgaagatttggtgattgagtggcggacgggtgagtaacgcgtgggtaacctgccctgtacagggggataacagtcagaaatgactgctaataccgcataagaccacagcaccgcatggtgcaggggtaaaaactccggtggtacaggatggacccgcgtctgattagctggttggtgaggtaacggctcaccaaggcgacgatcagtagccggcttgagagagtgaacggccacattgggactgagacacggcccaaactcctacgggaggcagcagtggggaatattgcacaatgggggaaaccctgatgcagcgacgccgcgtgagtgaagaagtatttcggtatgtaaagctctatcagcagggaagaaaatgacggtacctgactaagaagccccggctaactacgtgccagcagccgcggtaatacgtagggggcaagcgttatccggaattactgggtgtaaagggtgcgtaggtggtatggcaagtcagaagtgaaaacccagggcttaactctgggactgcttttgaaactgtcagactagagtgcaggagaggtaagcggaattcctagtgtagcggtgaaatgcgtagatattaggaggaacatcagtggcgaaggcggcttactggactgaaactgacactgaggcacgaaagcgtggggagcaaacaggattagataccctggtagtccacgccgtaaacgatgaatactaggtgtcggggccgtagaggcttcggtgccgcagccaacgcagtaagtattccacctggggagtacgttcgcaagaatgaaactcaaaggaattgacggggacccgcacaagcggtggagcatgtggtttaattcgaagcaacgcgaagaaccttacctggtcttgacatccttctgaccggtccttaaccggacctttccttcgggacaggagtgacaggtggtgcatggttgtcgtcagctcgtgtcgtgagatgttgggttaagtcccgcaacgagcgcaacccctatctttagtagccagcatataaggtgggcactctagagagactgccagggataacctggaggaaggtggggacgacgtcaaatcatcatgccccttatgaccagggctacacacgtgctacaatggcgtaaacagagggaagcagcctcgtgagagtgagcaaatcccaaaaataacgtctcagttcggattgtagtctgcaactcgactacatgaagctggaatcgctagtaatcgcgaatcagaatgtcgcggtgaatacgttcccgggtcttgtacacaccgcccgtcacaccatgggagtcagtaacgcccgaagtcagtgacccaaccgtaaggagggagctgccgaaggcgggaccgataactggggtgaagtcgtaacaaggtagccgtatcggaaggtgcggctggatcacct

SEQ ID NO: 85 - DNA, 1518 bp, Unknown
  F17
agagtttgatcctggctcaggatgaacgctggcggcgtgcttaacacatgcaagtcgaacggggaacattttatggaagcttcggtggaaatagcttgttcctagtggcggacgggtgagtaacgcgtgggtaacctgcctcacactgggggataacagtcagaaatgactgctaataccgcataagcgcacgggattgcatgatccagtgtgaaaaactccggtggtgtgagatggacccgcgttggattagccagttggcagggtaacggcctaccaaagcgacgatccatagccggcctgagagggtggacggccacattgggactgagacacggcccagactcctacgggaggcagcagtggggaatattgcacaatgggggaaaccctgatgcagcgacgccgcgtgaaggaagaagtatctcggtatgtaaacttctatcagcagggaagaaaatgacggtacctgactaagaagccccggctaactacgtgccagcagccgcggtaatacgtagggggcaagcgttatccggatttactgggtgtaaagggagcgtagacggagcagcaagtctgatgtgaaaggcgggggctcaacccccggactgcattggaaactgttgatcttgagtaccggagaggtaagcggaattcctagtgtagcggtgaaatgcgtagatattaggaggaacaccagtggcgaaggcggcttactggacggtaactgacgttgaggctcgaaagcgtggggagcaaacaggattagataccctggtagtccacgccgtaaacgatgaatactaggtgtcgggtggcagagccattcggtgccgcagcaaacgcagtaagtattccacctggggagtacgttcgcaagaatgaaactcaaaggaattgacggggacccgcacaagcggtggagcatgtggtttaattcgaagcaacgcgaagaaccttaccaagtcttgacatccctctgaccggtgagtaacgtcacctttccttcgggacagaggagacaggtggtgcatggttgtcgtcagctcgtgtcgtgagatgttgggttaagtcccgcaacgagcgcaacccctatccttagtagccagcggtttggccgggcactctgaggagactgccagggataacctggaggaaggcggggatgacgtcaaatcatcatgccccttatgatttgggctacacacgtgctacaatggcgtaaacaaagggaagcgagagtgtgagcttaagcaaatcccaaaaataacgtcccagttcggactgcagtctgcaactcgactgcacgaagctggaatcgctagtaatcgcggatcagaatgccgcggtgaatacgttcccgggtcttgtacacaccgcccgtcacaccatgggagtcagtaacgcccgaagtcagtgaccgaaccgaaaggacggagctgccgaaggcgggacggatgactggggtgaagtcgtaacaaggtagccgtatcggaaggtgcggctggatcacct

SEQ ID NO: 86 - DNA, 1522 bp, Unknown
  F18
agagtttgatcctggctcaggatgaacgctggcggcgtgcctaacacatgcaagtcgaacgaagcaattaaaatgaagttttcggatggatttttgattgactgagtggcggacgggtgagtaacgcgtggataacctgcctcacactgggggataacagttagaaatgactgctaataccgcataagcgcacagtaccgcatggtacggtgtgaaaaactccggtggtgtgagatggatccgcgtctgattagccagttggcggggtaacggcccaccaaagcgacgatcagtagccgacctgagagggtgaccggccacattgggactgagacacggcccaaactcctacgggaggcagcagtggggaatattgcacaatgggcgaaagcctgatgcagcgacgccgcgtgagtgaagaagtatttcggtatgtaaagctctatcagcagggaagaaaatgacggtacctgactaagaagccccggctaactacgtgccagcagccgcggtaatacgtagggggcaagcgttatccggatttactgggtgtaaagggagcgtagacggcgaagcaagtctgaagtgaaaacccagggctcaaccctgggactgctttggaaactgttttgctagagtgtcggagaggtaagtggaattcctagtgtagcggtgaaatgcgtagatattaggaggaacaccagtggcgaaggcggcttactggacgataactgacgttgaggctcgaaagcgtggggagcaaacaggattagataccctggtagtccacgccgtaaacgatgaatgctaggtgttggggggcaaagcccttcggtgccgtcgcaaacgcagtaagcattccacctggggagtacgttcgcaagaatgaaactcaaaggaattgacggggacccgcacaagcggtggagcatgtggtttaattcgaagcaacgcgaagaaccttaccaagtcttgacatcctcttgaccggcgtgtaacggcgccttcccttcggggcaagagagacaggtggtgcatggttgtcgtcagctcgtgtcgtgagatgttgggttaagtcccgcaacgagcgcaacccttatccttagtagccagcaggtagagctgggcactctagggagactgccagggataacctggaggaaggtggggatgacgtcaaatcatcatgccccttatgatttgggctacacacgtgctacaatggcgtaaacaaagggaagcaagacagtgatgtggagcaaatcccaaaaataacgtcccagttcggactgtagtctgcaacccgactacacgaagctggaatcgctagtaatcgcgaatcagaatgtcgcggtgaatacgttcccgggtcttgtacacaccgcccgtcacaccatgggagtcagcaacgcccgaagtcagtgacccaactcgcaagagagggagctgccgaaggcggggcaggtaactggggtgaagtcgtaacaaggtagccgtatcggaaggtgcggctggatcacct

SEQ ID NO: 97 - DNA, 1520 bp, Unknown
  F19
agagtttgatcctggctcaggatgaacgctggcggcgtgcttaacacatgcaagtcgaacggggattattttgacagagacttcggttgaagtcgttataatcctagtggcggacgggtgagtaacgcgtgggtaacctgcctcacactgggggataacagtcagaaatgactgctaataccgcataagcgcacgggattgcatgatccagtgtgaaaaactccggtggtgtgagatggacccgcgttggattagccagttggcagggtaacggcctaccaaagcgacgatccatagccggcctgagagggtggacggccacattgggactgagacacggcccagactcctacgggaggcagcagtggggaatattgcacaatgggggaaaccctgatgcagcgacgccgcgtgaaggaagaagtatctcggtatgtaaacttctatcagcagggaagaaaatgacggtacctgactaagaagccccggctaactacgtgccagcagccgcggtaatacgtagggggcaagcgttatccggatttactgggtgtaaagggagcgtagacggagcagcaagtctgatgtgaaaggcgggggctcaacccccggactgcattggaaactgttgatcttgagtaccggagaggtaagcggaattcctagtgtagcggtgaaatgcgtagatattaggaggaacaccagtggcgaaggcggcttactggacggtaactgacgttgaggctcgaaagcgtggggagcaaacaggattagataccctggtagtccacgccgtaaacgatgaatactaggtgtcgggtggcagagccattcggtgccgcagcaaacgcagtaagtattccacctggggagtacgttcgcaagaatgaaactcaaaggaattgacggggacccgcacaagcggtggagcatgtggtttaattcgaagcaacgcgaagaaccttaccaagtcttgacatccctctgaccggtgagtaacgtcacctttccttcgggacagaggagacaggtggtgcatggttgtcgtcagctcgtgtcgtgagatgttgggttaagtcccgcaacgagcgcaacccctatccttagtagccagcggtttggccgggcactctgaggagactgccagggataacctggaggaaggcggggatgacgtcaaatcatcatgccccttatgatttgggctacacacgtgctacaatggcgtaaacaaagggaagcgagagtgtgagcttaagcaaatcccaaaaataacgtcccagttcggactgcagtctgcaactcgactgcacgaagctggaatcgctagtaatcgcggatcagaatgccgcggtgaatacgttcccgggtcttgtacacaccgcccgtcacaccatgggagtcagtaacgcccgaagtcagtgaccgaaccgaaaggacggagctgccgaaggcgggacggatgactggggtgaagtcgtaacaaggtagccgtatcggaaggtgcggctggatcacct

SEQ ID NO: 88 - DNA, 1528 bp, Unknown
  F20
agagtttgatcctggctcaggatgaacgctggcggcatgcctaatacatgcaagtcgaacgaagtttcgaggaagcttgcttccaaagagacttagtggcgaacgggtgagtaacacgtaggtaacctgcccatgtgtccgggataactgctggaaacggtagctaaaaccggataggtatacagagcgcatgctcagtatattaaagcgcccatcaaggcgtgaacatggatggacctgcggcgcattagctagttggtgaggtaacggcccaccaaggcgatgatgcgtagccggcctgagagggtaaacggccacattgggactgagacacggcccaaactcctacgggaggcagcagtagggaattttcgtcaatgggggaaaccctgaacgagcaatgccgcgtgagtgaagaaggtcttcggatcgtaaagctctgttgtaagtgaagaacggctcatagaggaaatgctatgggagtgacggtagcttaccagaaagccacggctaactacgtgccagcagccgcggtaatacgtaggtggcaagcgttatccggaatcattgggcgtaaagggtgcgtaggtggcgtactaagtctgtagtaaaaggcaatggctcaaccattgtaagctatggaaactggtatgctggagtgcagaagagggcgatggaattccatgtgtagcggtaaaatgcgtagatatatggaggaacaccagtggcgaaggcggtcgcctggtctgtaactgacactgaggcacgaaagcgtggggagcaaataggattagataccctagtagtccacgccgtaaacgatgagaactaagtgttggaggaattcagtgctgcagttaacgcaataagttctccgcctggggagtatgcacgcaagtgtgaaactcaaaggaattgacgggggcccgcacaagcggtggagtatgtggtttaattcgaagcaacgcgaagaaccttaccaggccttgacatggaaacaaataccctagagatagggggataattatggatcacacaggtggtgcatggttgtcgtcagctcgtgtcgtgagatgttgggttaagtcccgcaacgagcgcaacccttgtcgcatgttaccagcatcaagttggggactcatgcgagactgccggtgacaaaccggaggaaggtggggatgacgtcaaatcatcatgccccttatggcctgggctacacacgtactacaatggcgaccacaaagagcagcgacacagtgatgtgaagcgaatctcataaaggtcgtctcagttcggattgaagtctgcaactcgacttcatgaagtcggaatcgctagtaatcgcagatcagcatgctgcggtgaatacgttctcgggccttgtacacaccgcccgtcaaaccatgggagtcagtaatacccgaagccggtggcataaccgtaaggagtgagccgtcgaaggtaggaccgatgactggggttaagtcgtaacaaggtatccctacgggaacgtggggatggatcacct

SEQ ID NO: 89 - DNA, 1521 bp, Unknown
  F21
agagtttgatcctggctcaggatgaacgctggcggcgtgcttaacacatgcaagtcgagcgaagcacttaagtggatctcttcggattgaaacttatttgactgagcggcggacgggtgagtaacgcgtgggtaacctgcctcatacagggggataacagttagaaatggctgctaataccgcataagcgcacaggaccgcatggtctggtgtgaaaaactccggtggtatgagatggacccgcgtctgattagctagttggaggggtaacggcccaccaaggcgacgatcagtagccggcctgagagggtgaacggccacattgggactgagacacggcccagactcctacgggaggcagcagtggggaatattgcacaatgggggaaaccctgatgcagcgacgccgcgtgaaggaagaagtatctcggtatgtaaacttctatcagcagggaagaaaatgacggtacctgactaagaagccccggctaactacgtgccagcagccgcggtaatacgtagggggcaagcgttatccggatttactgggtgtaaagggagcgtagacggaagagcaagtctgatgtgaaaggctggggcttaaccccaggactgcattggaaactgtttttctagagtgccggagaggtaagcggaattcctagtgtagcggtgaaatgcgtagatattaggaggaacaccagtggcgaaggcggcttactggacggtaactgacgttgaggctcgaaagcgtggggagcaaacaggattagataccctggtagtccacgccgtaaacgatgaatactaggtgtcgggtggcaaagccattcggtgccgcagcaaacgcaataagtattccacctggggagtacgttcgcaagaatgaaactcaaaggaattgacggggacccgcacaagcggtggagcatgtggtttaattcgaagcaacgcgaagaaccttaccaagtcttgacatccctctgaccggcccgtaacggggccttcccttcggggcagaggagacaggtggtgcatggttgtcgtcagctcgtgtcgtgagatgttgggttaagtcccgcaacgagcgcaacccctatccttagtagccagcaggtgaagctgggcactctagggagactgccggggataacccggaggaaggcggggacgacgtcaaatcatcatgccccttatgatttgggctacacacgtgctacaatggcgtaaacaaagggaagcgagacagcgatgttgagcaaatcccaaaaataacgtcccagttcggactgcagtctgcaactcgactgcacgaagctggaatcgctagtaatcgcgaatcagaatgtcgcggtgaatacgttcccgggtcttgtacacaccgcccgtcacaccatgggagtcagtaacgcccgaagtcagtgacccaaccttataggagggagctgccgaaggcgggaccgataactggggtgaagtcgtaacaaggtagccgtatcggaaggtgcggctggatcacct

SEQ ID NO: 90 - DNA, 1518 bp, Unknown
  F22
agagtttgatcctggctcaggatgaacgctggcggcgtgcctaacacatgcaagtcgaacgaagcattttagatgaagttttcggatggattctgagatgactgagtggcggacgggtgagtaacacgtggataacctgcctcacactgggggacaacagttagaaatgactgctaataccgcataagcgcacagtaccgcatggtacggtgtgaaaaactccggtggtgtgagatggatccgcgtctgattagccagttggcggggtaacggcccaccaaagcgacgatcagtagccgacctgagagggtgaccggccacattgggactgagacacggcccaaactcctacgggaggcagcagtggggaatattgcacaatgggcgaaagcctgatgcagcgacgccgcgtgagtgaagaagtatttcggtatgtaaagctctatcagcagggaagataatgacggtacctgactaagaagccccggctaactacgtgccagcagccgcggtaatacgtagggggcaagcgttatccggatttactgggtgtaaagggagcgtagacggcatggcaagtctgaagtgaaaacccagggctcaaccctgggactgctttggaaactgtcaagctagagtgcaggagaggtaagtggaattcctagtgtagcggtgaaatgcgtagatattaggaggaacaccagtggcgaaggcggcttactggactgtaactgacgttgaggctcgaaagcgtggggagcaaacaggattagataccctggtagtccacgccgtaaacgatgagtgctaggtgttggggggcaaagcccttcggtgccgtcgcaaacgcaataagcactccacctggggagtacgttcgcaagaatgaaactcaaaggaattgacggggacccgcacaagcggtggagcatgtggtttaattcgaagcaacgcgaagaaccttaccaagtcttgacatcctcttgaccggcgtgtaacggcgcctttccttcgggacaagagagacaggtggtgcatggttgtcgtcagctcgtgtcgtgagatgttgggttaagtcccgcaacgagcgcaacccttatccttagtagccagcattaagatgggcactctagggagactgccagggacaacctggaggaaggtggggatgacgtcaaatcatcatgccccttatgatttgggctacacacgtgctacaatggcgtaaacaaagggaagcgaccctgcgaaggtgagcaaatctcaaaaataacgtcccagttcggactgtagtctgcaacccgactacacgaagctggaatcgctagtaatcgcgaatcagaatgtcgcggtgaatacgttcccgggtcttgtacacaccgcccgtcacaccatgggagtcagcaacgcccgaagtcagtgacccaaccgaaaggagggagctgccgaaggcggggcaggtaactggggtgaagtcgtaacaaggtagccgtatcggaaggtgcggctggatcacct

SEQ ID NO: 91 - DNA, 1519 bp, Unknown
  F23
agagtttgatcctggctcaggatgaacgctggcggcgtgcttaacacatgcaagtcgaacgaagcactttaccggatttcttcgggatgaaagttttgtgactgagtggcggacgggtgagtaacgcgtgggtaacctgcctcatacagggggataacagttagaaatgactgctaataccgcataagaccacaggattgcatgatccggtggtaaaaactccggtggtatgagatggacccgcgtctgattaggtagttggtggggtaacggctcaccaagccgacgatcagtagccgacctgagagggtgaccggccacattgggactgagacacggcccaaactcctacgggaggcagcagtggggaatattgcacaatgggggaaaccctgatgcagcgacgccgcgtgagcgatgaagtatttcggtatgtaaagctctatcagcagggaagaaaatgacggtacctgactaagaagcaccggctaaatacgtgccagcagccgcggtaatacgtatggtgcaagcgttatccggatttactgggtgtaaagggagcgtagacggagaggcaagtctgatgtgaaaacccggggctcaaccccgggactgcattggaaactgtttttctagagtgtcggagaggtaagtggaattcctagtgtagcggtgaaatgcgtagatattaggaggaacaccagtggcgaaggcggcttactggacgatgactgacgttgaggctcgaaagcgtggggagcaaacaggattagataccctggtagtccacgccgtaaacgatgactgctaggtgtcgggaggcaaagcctttcggtgccgcagcaaacgcaataagcagtccacctggggagtacgttcgcaagaatgaaactcaaaggaattgacggggacccgcacaagcggtggagcatgtggtttaattcgaagcaacgcgaagaaccttacctgcccttgacatccggctgaccggcgagtaatgtcgcctttccttcgggacagccgagacaggtggtgcatggttgtcgtcagctcgtgtcgtgagatgttgggttaagtcccgcaacgagcgcaacccttatctttagtagccagcatttcggatgggcactctagagagactgccagggataacctggaggaaggtggggatgacgtcaaatcatcatgccccttatgggcagggctacacacgtgctacaatggcgtaaacaaagggaggcaagcctgcgagggtgagcaaatcccaaaaataacgtctcagttcggattgtagtctgcaactcgactacatgaagctggaatcgctagtaatcgcgaatcagaatgtcgcggtgaatacgttcccgggtcttgtacacaccgcccgtcacaccatgggagttggtaacgcccgaagtcagtgacccaaccgtaaggagggagctgccgaaggtgggaccgataactggggtgaagtcgtaacaaggtagccgtatcggaaggtgcggctggatcacct

SEQ ID NO: 92 - DNA, 1520 bp, Unknown
  F24
agagtttgatcctggctcaggatgaacgctggcggcgtgcctaacacatgcaagtcgaacgaagttacacagaggaagttttcggatggaatcggtataacttagtggcggacgggtgagtaacgcgtgggaaacctgccctgtaccgggggataacacttagaaataggtgctaataccgcataagcgcacggaaccgcatggttgtgtgtgaaaaactccggtggtacaggatggtcccgcgtctgattagccagttggcagggtaacggcctaccaaagcgacgatcagtagccggcctgagagggtgaacggccacattgggactgagacacggcccaaactcctacgggaggcagcagtggggaatattgcacaatgggggaaaccctgatgcagcgacgccgcgtgagtgaagaagtatttcggtatgtaaagctctatcagcagggaagaaaatgacggtacctgactaagaagccccggctaactacgtgccagcagccgcggtaatacgtagggggcaagcgttatccggatttactgggtgtaaagggagcgtagacggcatggcaagccagatgtgaaaacccagggctcaaccttgggattgcatttggaactgccaggctggagtgcaggagaggtaagcggaattcctagtgtagcggtgaaatgcgtagatattaggaggaacaccagtggcgaaggcggcttactggactgtaactgacgttgaggctcgaaagcgtggggagcaaacaggattagataccctggtagtccacgcggtaaacgatgattgctaggtgtaggtgggtatggacccatcggtgccgcagctaacgcaataagcaatccacctggggagtacgttcgcaagaatgaaactcaaaggaattgacggggacccgcacaagcggtggagcatgtggtttaattcgaagcaacgcgaagaaccttaccaagtcttgacatcccattgacgtgcctgtaaagaggcattcccttcggggcaatggagacaggtggtgcatggttgtcgtcagctcgtgtcgtgagatgttgggttaagtcccgcaacgagcgcaacccttattcttagtagccagcaggtaaagctgggcactctaaggagactgccggggataacccggaggaaggcggggatgacgtcaaatcatcatgccccttatgatttgggctacacacgtgctacaatggcgtaaacaaagggaagcgagacagtgatgtggagcaaatcccagaaataacgtctcagttcggattgtagtctgcaactcgactacatgaagctggaatcgctagtaatcgcgaatcagcatgtcgcggtgaatacgttcccgggtcttgtacacaccgcccgtcacaccatgggagttggaaatgcccgaagtctgtgacctaaccgaaagggaggagcagccgaaggcaggtctgataactggggtgaagtcgtaacaaggtagccgtatcggaaggtgcggctggatcacct

SEQ ID NO: 93 - DNA, 1519 bp, Unknown; identical to SEQ ID NO: 91
  F25

SEQ ID NO: 94 - DNA, 1520 bp, Unknown
  F26
agagtttgatcctggctcaggatgaacgctggcggcgtgcttaacacatgcaagtcgaacggggtgctcatgacggaggattcgtccaacggattgagttacctagtggcggacgggtgagtaacgcgtgaggaacctgccttggagaggggaataacactccgaaaggagtgctaataccgcatgatgcagttgggtcgcatggctctgactgccaaagatttatcgctctgagatggcctcgcgtctgattagctagtaggcggggtaacggcccacctaggcgacgatcagtagccggactgagaggttgaccggccacattgggactgagacacggcccagactcctacgggaggcagcagtggggaatattgggcaatgggcgcaagcctgacccagcaacgccgcgtgaaggaagaaggctttcgggttgtaaacttcttttgtcggggacgaaacaaatgacggtacccgacgaataagccacggctaactacgtgccagcagccgcggtaatacgtaggtggcaagcgttatccggatttactgggtgtaaagggcgtgtaggcgggattgcaagtcagatgtgaaaactgggggctcaacctccagcctgcatttgaaactgtagttcttgagtgctggagaggcaatcggaattccgtgtgtagcggtgaaatgcgtagatatacggaggaacaccagtggcgaaggcggattgctggacagtaactgacgctgaggcgcgaaagcgtggggagcaaacaggattagataccctggtagtccacgccgtaaacgatggatactaggtgtggggggtctgaccccctccgtgccgcagttaacacaataagtatcccacctggggagtacgatcgcaaggttgaaactcaaaggaattgacgggggcccgcacaagcggtggagtatgtggtttaattcgaagcaacgcgaagaaccttaccagggcttgacatcccactaacgaagcagagatgcattaggtgcccttcggggaaagtggagacaggtggtgcatggttgtcgtcagctcgtgtcgtgagatgttgggttaagtcccgcaacgagcgcaacccttattgttagttgctacgcaagagcactctagcgagactgccgttgacaaaacggaggaaggtggggacgacgtcaaatcatcatgccccttatgtcctgggccacacacgtactacaatggtggttaacagagggaggcaataccgcgaggtggagcaaatccctaaaagccatcccagttcggattgcaggctgaaacccgcctgtatgaagttggaatcgctagtaatcgcggatcagcatgccgcggtgaatacgttcccgggccttgtacacaccgcccgtcacaccatgagagtcgggaacacccgaagtccgtagcctaaccgcaaggagggcgcggccgaaggtgggttcgataattggggtgaagtcgtaacaaggtagccgtatcggaaggtgcggctggatcacct

SEQ ID NO: 95 - DNA, 1519 bp, Unknown; identical to SEQ ID NO: 79
  F27

SEQ ID NO: 96 - DNA, 1491 bp, Unknown
  F28
agagtttgatcctggctcaggatgaacgctggcggcgtgcctaacacatgcaagtcgagcgattctcttcggagaagagcggcggacgggtgagtaacgcgtgggtaacctgccctgtacacacggataacataccgaaaggtatgctaatacgggataacataagaaattcgcatgtttttcttatcaaagctccggcggtacaggatggacccgcgtctgattagctagttggtgaggtaacggctcaccaaggcgacgatcagtagccgacctgagagggtgatcggccacattggaactgagacacggtccaaactcctacgggaggcagcagtggggaatattgcacaatgggcgaaagcctgatgcagcaacgccgcgtgagcgatgaaggccttcgggtcgtaaagctctgtcctcaaggaagataatgacggtacttgaggaggaagccccggctaactacgtgccagcagccgcggtaatacgtagggggctagcgttatccggatttactgggcgtaaagggtgcgtaggcggtcttttaagtcaggagtgaaaggctacggctcaaccgtagtaagctcttgaaactggaggacttgagtgcaggagaggagagtggaattcctagtgtagcggtgaaatgcgtagatattaggaggaacaccagtagcgaaggcggctctctggactgtaactgacgctgaggcacgaaagcgtggggagcaaacaggattagataccctggtagtccacgccgtaaacgatgagtactagctgtcggaggttacccccttcggtggcgcagctaacgcattaagtactccgcctggggagtacgctcgcaagagtgaaactcaaaggaattgacggggacccgcacaagtagcggagcatgtggtttaattcgaagcaacgcgaagaaccttacctaagcttgacatccttttgaccgatgcctaatcgcatctttcccttcggggacagaagtgacaggtggtgcatggttgtcgtcagctcgtgtcgtgagatgttgggttaagtcccgcaacgagcgcaacccttgcctttagttgccatcattaagttgggcactctagagggactgccagggataacctggaggaaggtggggatgacgtcaaatcatcatgccccttatgcttagggctacacacgtgctacaatgggtggtacagagggcagcgaagtcgtgaggccaagctaatcccttaaagccattctcagttcggattgtaggctgaaactcgcctacatgaagctggagttactagtaatcgcagatcagaatgctgcggtgaatgcgttcccgggtcttgtacacaccgcccgtcacaccatgggagttgggggcgcccgaagccggctagctaaccttttggaagcggtcgtcgaaggtgaaaccaataactggggtgaagtcgtaacaaggtagccgtatcggaaggtgcggctggatcacct

SEQ ID NO: 97 - DNA, 1519 bp, Unknown
  F29
agagtttgatcctggctcaggatgaacgctggcggcgtgcttaacacatgcaagtcgagcgaagcacttttgcagatttcttcggattgaagcaattgtgactgagcggcggacgggtgagtaacgcgtgggtaacctgcctcatacagggggataacagttggaaacggctgctaataccgcataagcgcacagtaccgcatggtaccgtgtgaaaaactccggtggtatgagatggacccgcgtctgattagctagttggtggggtaacggcctaccaaggcgacgatcagtagccgacctgagagggtgaccggccacattgggactgagacacggcccaaactcctacgggaggcagcagtggggaatattgcacaatgggggaaaccctgatgcagcgacgccgcgtgagcgatgaagtatttcggtatgtaaagctctatcagcagggaagaaaatgacggtacctgactaagaagccccggctaactacgtgccagcagccgcggtaatacgtagggggcaagcgttatccggatttactgggtgtaaagggagcgtagacggcatggcaagccagatgtgaaagcccggggctcaaccccgggactgcatttggaactgtcaggctagagtgtcggagaggaaagcggaattcctagtgtagcggtgaaatgcgtagatattaggaggaacaccagtggcgaaggcggctttctggacgatgactgacgttgaggctcgaaagcgtggggagcaaacaggattagataccctggtagtccacgccgtaaacgatgaatactaggtgtcgggtggcaaagccattcggtgccgcagcaaacgcaataagtattccacctggggagtacgttcgcaagaatgaaactcaaaggaattgacggggacccgcacaagcggtggagcatgtggtttaattcgaagcaacgcgaagaaccttacctggtcttgacatccctctgaccgctctttaatcggagctttccttcgggacagaggagacaggtggtgcatggttgtcgtcagctcgtgtcgtgagatgttgggttaagtcccgcaacgagcgcaacccttatctttagtagccagcatttaaggtgggcactctagagagactgccagggataacctggaggaaggtggggatgacgtcaaatcatcatgccccttatgaccagggctacacacgtgctacaatggcgtaaacaaagggaagcgagcccgcgagggggagcaaatcccaaaaataacgtctcagttcggattgtagtctgcaactcgactacatgaagctggaatcgctagtaatcgcgaatcagaatgtcgcggtgaatacgttcccgggtcttgtacacaccgcccgtcacaccatgggagtcagtaacgcccgaagtcagtgacccaaccgcaaggagggagctgccgaaggtgggaccgataactggggtgaagtcgtaacaaggtagccgtatcggaaggtgcggctggatcacct

SEQ ID NO: 98 - DNA, 1512 bp, Unknown
  F30
agagtttgatcctggctcaggatgaacgctggcggcgtgcctaatacatgcaagtcggacgcaatgcttcggcattgagtggcgaacgggtgagtaagacataagcaacctgcccctgtgagggggataactgctggaaacggcagctaagaccgcataggcatagaggacgcatgtcgactatgttaaatatcccacgggatagcacagggatgggcttatgacgcattagccagctggtgaggtaacggctcaccagggcgacgatgcgtagccggcctgagagggtggacggccacactgggactgagacacggcccagactcctacgggaggcagcagtagggaattttcggcaatgggcgaaagcctgaccgagcaacgccgcgtgaaggaagaagtcattcgtgatgtaaacttctgttatgaaggaagaacggcagatggagggaatgccatgtgcgtgacggtacttcatgaggaagccacggctaactacgtgccagcagccgcggtaatacgtaggtggcgagcgttatccggaatcattgggcgtaaagagggagcaggcggcagtgcaggtctgcggtgaaagaccggagctaaacttcggtaagccgtggaaaccgcacagctagagagcatcagaggatcgcggaattccatgtgtagcggtgaaatgcgtagatatatggaggaacaccagtggcgaaggcggcggtctggggtgcagctgacgctcagtcccgaaagcgtggggagcaaataggattagataccctagtagtccacgccgtaaacgatgagtgctaagtgttgggggtcagacctcagtgctggagttaacgcaataagcactccgcctgagtagtacgttcgcaagaatgaaactcaaaggaattgacgggggcccgcacaagcggtggagcatgtggtttaattcgaagcaacgcgaagaaccttaccaggtcttgacatggagataaaggccctggagacagggagatagatatatctcacacaggtggtgcatggttgtcgtcagctcgtgtcgtgagatgttgggttaagtcccgcaacgagcgcaacccctgttgccagttgccagcattaggttggggactctggcgagactgcctctgcaaggaggaggaaggcggggatgacgtcaaatcatcatgccccttatgacctgggctacacacgtgctacaatggacggatcagagggaggcgaagccgcgaggtggagcgaaacccagaaacccgttcacagttcggactgcagtctgcaactcgactgcacgaagctggaatcgctagtaatcgcgaatcagcatgtcgcggtgaatacgttctcgggccttgtacacaccgcccgtcacaccatgagagttggtaacacccgaagccggtggcccaaccgcaaggagggagctgtctaaggtgggactgatgattggggtgaagtcgtaacaaggtatccctacgggaacgtggggatggatcacct

SEQ ID NO: 99 - DNA, 1523 bp, Unknown
  F31
agagtttgatcctggctcaggatgaacgctggcggcgtgcttaacacatgcaagtcgaacgaagcattttggaaggaagttttcggatggaattccttaatgactgagtggcggacgggtgagtaacgcgtggggaacctgccctatacagggggataacagctggaaacggctgctaataccgcataagcgcacagaatcgcatgattcggtgtgaaaagctccggcagtataggatggtcccgcgtctgattagctggttggcggggtaacggcccaccaaggcgacgatcagtagccggcttgagagagtggacggccacattgggactgagacacggcccaaactcctacgggaggcagcagtggggaatattgcacaatggggggaaccctgatgcagcgacgccgcgtgagtgaagaagtatttcggtatgtaaagctctatcagcagggaagaaaaaagacggtacctgactaagaagccccggctaactacgtgccagcagccgcggtaatacgtagggggcaagcgttatccggaattactgggtgtaaagggtgcgtaggtggcatggtaagtcagaagtgaaagcccggggcttaaccccgggactgcttttgaaactgtcatgctggagtgcaggagaggtaagcggaattcctagtgtagcggtgaaatgcgtagatattaggaggaacaccagtggcgaaggcggcttactggactgtcactgacactgatgcacgaaagcgtggggagcaaacaggattagataccctggtagtccacgccgtaaacgatgaatactaggtgtcggggccgtagaggcttcggtgccgcagcaaacgcagtaagtattccacctggggagtacgttcgcaagaatgaaactcaaaggaattgacggggacccgcacaagcggtggagcatgtggtttaattcgaagcaacgcgaagaaccttacctggtcttgacatctaactgaccggttcgtaatgggacctttccttcgggacagttaagacaggtggtgcatggttgtcgtcagctcgtgtcgtgagatgttgggttaagtcccgcaacgagcgcaacccctatctttagtagccagcatataaggtgggcactctagagagactgccagggataacctggaggaaggtggggacgacgtcaaatcatcatgccccttatggccagggctacacacgtgctacaatggcgtaaacaaagggaagcgaagtcgtgaggcgaagcaaatcccagaaataacgtctcagttcggattgtagtctgcaactcgactacatgaagctggaatcgctagtaatcgtgaatcagaatgtcacggtgaatacgttcccgggtcttgtacacaccgcccgtcacaccatgggagtcagtaacgcccgaagtcagtgacccaaccttataggagggagctgccgaaggtgggaccgataactggggtgaagtcgtaacaaggtagccgtatcggaaggtgcggctggatcacct

SEQ ID NO: 100 - DNA, 1520 bp, Unknown
  F32
agagtttgatcctggctcaggatgaacgctggcggcgtgcttaacacatgcaagtcgagcgaagcgctaagacggatttcttcggattgaagtctttgtgactgagcggcggacgggtgagtaacgcgtgggtaacctgcctcatacagggggataacagttagaaatgactgctaataccgcataagcgcacaggaccgcatggtctggtgtgaaaaactccggtggtatgagatggacccgcgtctgattagctagttggaggggtaacggcccaccaaggcgacgatcagtagccggcctgagagggtgaacggccacattgggactgagacacggcccagactcctacgggaggcagcagtggggaatattgcacaatgggggaaaccctgatgcagcgacgccgcgtgaaggaagaagtatctcggtatgtaaacttctatcagcagggaagaaaatgacggtacctgactaagaagccccggctaactacgtgccagcagccgcggtaatacgtagggggcaagcgttatccggatttactgggtgtaaagggagcgtagacggaagagcaagtctgatgtgaaaggctggggcttaaccccaggactgcattggaaactgttgttctagagtgccggagaggtaagcggaattcctagtgtagcggtgaaatgcgtagatattaggaggaacaccagtggcgaaggcggcttactggacggtaactgacgttgaggctcgaaagcgtggggagcaaacaggattagataccctggtagtccacgccgtaaacgatgaatactaggtgtcgggtggcaaagccattcggtgccgcagcaaacgcaataagtattccacctggggagtacgttcgcaagaatgaaactcaaaggaattgacggggacccgcacaagcggtggagcatgtggtttaattcgaagcaacgcgaagaaccttaccaagtcttgacatccctctgaccgtcccgtaacgggggcttcccttcggggcagaggagacaggtggtgcatggttgtcgtcagctcgtgtcgtgagatgttgggttaagtcccgcaacgagcgcaacccttatccttagtagccagcacatgatggtgggcactctagggagactgccggggataacccggaggaaggcggggacgacgtcaaatcatcatgccccttatgatttgggctacacacgtgctacaatggcgtaaacaaagggaagcgagacagcgatgttgagcgaatcccaaaaataacgtcccagttcggactgcagtctgcaactcgactgcacgaagctggaatcgctagtaatcgcggatcagaatgccgcggtgaatacgttcccgggtcttgtacacaccgcccgtcacaccatgggagtcagtaacgcccgaagtcagtgacctaaccgaaaggaaggagctgccgaaggcgggaccgataactggggtgaagtcgtaacaaggtagccgtatcggaaggtgcggctggatcacct

SEQ ID NO: 101 - DNA, 1515 bp, Unknown
  F33
agagtttgatcctggctcaggatgaacgctggcggcgtgcctaatacatgcaagtcgaacgcgagcacttgtgctcgagtggcgaacgggtgagtaatacataagtaacctgccctagacagggggataactattggaaacgatagctaagaccgcataggtacggacactgcatggtgaccgtattaaaagtgcctcaaagcactggtagaggatggacttatggcgcattagctggttggcggggtaacggcccaccaaggcgacgatgcgtagccgacctgagagggtgaccggccacactgggactgagacacggcccagactcctacgggaggcagcagtagggaattttcggcaatgggggaaaccctgaccgagcaacgccgcgtgaaggaagaaggttttcggattgtaaacttctgttataaaggaagaacggcggctacaggaaatggtagccgagtgacggtactttattagaaagccacggctaactacgtgccagcagccgcggtaatacgtaggtggcaagcgttatccggaattattgggcgtaaagagggagcaggcggcagcaagggtctgtggtgaaagcctgaagcttaacttcagtaagccatagaaaccaggcagctagagtgcaggagaggatcgtggaattccatgtgtagcggtgaaatgcgtagatatatggaggaacaccagtggcgaaggcgacgatctggcctgcaactgacgctcagtcccgaaagcgtggggagcaaataggattagataccctagtagtccacgccgtaaacgatgagtactaagtgttggatgtcaaagttcagtgctgcagttaacgcaataagtactccgcctgagtagtacgttcgcaagaatgaaactcaaaggaattgacgggggcccgcacaagcggtggagcatgtggtttaattcgaagcaacgcgaagaaccttaccaggtcttgacatactcataaaggctccagagatggagagatagctatatgagatacaggtggtgcatggttgtcgtcagctcgtgtcgtgagatgttgggttaagtcccgcaacgagcgcaacccttatcgttagttaccatcattaagttggggactctagcgagactgccagtgacaagctggaggaaggcggggatgacgtcaaatcatcatgccccttatgacctgggctacacacgtgctacaatggatggtgcagagggaagcgaagccgcgaggtgaagcaaaacccataaaaccattctcagttcggattgtagtctgcaactcgactacatgaagttggaatcgctagtaatcgcgaatcagcatgtcgcggtgaatacgttctcgggccttgtacacaccgcccgtcacaccacgagagttgataacacccgaagccggtggcctaaccgcaaggaaggagctgtctaaggtgggattgatgattggggtgaagtcgtaacaaggtatccctacgggaacgtggggatggatcacct

SEQ ID NO: 102 - DNA, 1552 bp, Unknown
  F34
agagtttgatcctggctcaggacgaacgctggcggcgtgcttaacacatgcaagtcgaacgaagagcgatggaagcttgcttctatcaatcttagtggcgaacgggtgagtaacgcgtaatcaacctgcccttcagagggggacaacagttggaaacgactgctaataccgcatacgatctaatctcggcatcgaggatagatgaaaggtggcctctacatgtaagctatcactgaaggaggggattgcgtctgattagctagttggaggggtaacggcccaccaaggcgatgatcagtagccggtctgagaggatgaacggccacattgggactgagacacggcccagactcctacgggaggcagcagtggggaatcttccgcaatggacgaaagtctgacggagcaacgccgcgtgagtgatgacggccttcgggttgtaaagctctgttaatcgggacgaaaggccttcttgcgaatagtgagaaggattgacggtaccggaatagaaagccacggctaactacgtgccagcagccgcggtaatacgtaggtggcaagcgttgtccggaattattgggcgtaaagcgcgcgcaggcggataggtcagtctgtcttaaaagttcggggcttaaccccgtgatgggatggaaactgccaatctagagtatcggagaggaaagtggaattcctagtgtagcggtgaaatgcgtagatattaggaagaacaccagtggcgaaggcgactttctggacgaaaactgacgctgaggcgcgaaagccaggggagcgaacgggattagataccccggtagtcctggccgtaaacgatgggtactaggtgtaggaggtatcgaccccttctgtgccggagttaacgcaataagtaccccgcctggggagtacgaccgcaaggttgaaactcaaaggaattgacgggggcccgcacaagcggtggagtatgtggtttaattcgacgcaacgcgaagaaccttaccaggtcttgacattgatggacagaaccagagatggttcctcttcttcggaagccagaaaacaggtggtgcacggttgtcgtcagctcgtgtcgtgagatgttgggttaagtcccgcaacgagcgcaacccctatcttatgttgccagcacgttagggtgggaactcatgagagactgccgcagacaatgcggaggaaggcggggatgacgtcaaatcatcatgccccttatgacctgggctacacacgtactacaatgggagttaatagacggaagcgagatcgcgagatggagcaaacccgagaaacactctctcagttcggatcgtaggctgcaactcgcctacgtgaagtcggaatcgctagtaatcgcaggtcagcatactgcggtgaatacgttcccgggccttgtacacaccgcccgtcacaccacgaaagtcggaagtgcccaaagccggtggggtaaccttcgggagccagccgtctaaggtaaagtcgatgattggggtgaagtcgtaacaaggtagccgtatcggaaggtgcggctggatcacct

SEQ ID NO: 103 - DNA, 1496 bp, Unknown
  F35
agagtttgatcctggctcaggatgaacgctgacagaatgcttaacacatgcaagtctacttgatccttcgggtgaaggtggcggacgggtgagtaacgcgtaaagaacttgccttacagactgggacaacatttggaaacgaatgctaataccggatattatgattgggtcgcatgatctggttatgaaagctatatgcgctgtgagagagctttgcgtcccattagttagttggtgaggtaacggctcaccaagacgatgatgggtagccggcctgagagggtgaacggccacaaggggactgagacacggcccttactcctacgggaggcagcagtggggaatattggacaatggaccaaaagtctgatccagcaattctgtgtgcacgatgaagtttttcggaatgtaaagtgctttcagttgggaagaagtcagtgacggtaccaacagaagaagcgacggctaaatacgtgccagcagccgcggtaatacgtatgtcgcaagcgttatccggatttattgggcgtaaagcgcgtctaggcggcttagtaagtctgatgtgaaaatgcggggctcaaccccgtattgcgttggaaactgctaaactagagtactggagaggtaggcggaactacaagtgtagaggtgaaattcgtagatatttgtaggaatgccgatggggaagccagcctactggacagatactgacgctaaagcgcgaaagcgtgggtagcaaacaggattagataccctggtagtccacgccgtaaacgatgattactaggtgttgggggtcgaacctcagcgcccaagctaacgcgataagtaatccgcctggggagtacgtacgcaagtatgaaactcaaaggaattgacggggacccgcacaagcggtggagcatgtggtttaattcgacgcaacgcgaggaaccttaccagcgtttgacatcccaagaagttaacagagatgttttcgtgcctcttcggaggaacttggtgacaggtggtgcatggctgtcgtcagctcgtgtcgtgagatgttgggttaagtcccgcaacgagcgcaacccctttcgtatgttaccatcattaagttggggactcatgcgagactgcctgcgatgagcaggaggaaggtggggatgacgtcaagtcatcatgccccttatacgctgggctacacacgtgctacaatgggtagtacagagagctgcaaacctgcgagggtaagctaatctcataaaactattcttagttcggattgtactctgcaactcgagtacatgaagttggaatcgctagtaatcgcaaatcagctatgttgcggtgaatacgttctcgggtcttgtacacaccgcccgtcacaccacgagagttggttgcacctgaagtaacaggcctaaccgtaaggagggatgttccgagggtgtgattagcgattggggtgaagtcgtaacaaggtatccgtacgggaacgtgcggatggatcacct

SEQ ID NO: 104 - DNA, 1496 bp, Unknown; identical to SEQ ID NO: 103
  F36

SEQ ID NO: 105 - DNA, 1530 bp, Unknown
  F37
agagtttgatcatggctcagattgaacgctggcggcaggcctaacacatgcaagtcgaacggtaacaggaagcagcttgctgctttgctgacgagtggcggacgggtgagtaatgtctgggaaactgcctgatggagggggataactactggaaacggtagctaataccgcataacgtcgcaagaccaaagagggggaccttcgggcctcttgccatcggatgtgcccagatgggattagctagtaggtggggtaacggctcacctaggcgacgatccctagctggtctgagaggatgaccagccacactggaactgagacacggtccagactcctacgggaggcagcagtggggaatattgcacaatgggcgcaagcctgatgcagccatgccgcgtgtatgaagaaggccttcgggttgtaaagtactttcagcggggaggaagggagtaaagttaatacctttgctcattgacgttacccgcagaagaagcaccggctaactccgtgccagcagccgcggtaatacggagggtgcaagcgttaatcggaattactgggcgtaaagcgcacgcaggcggtttgttaagtcagatgtgaaatccccgggctcaacctgggaactgcatctgatactggcaagcttgagtctcgtagaggggggtagaattccaggtgtagcggtgaaatgcgtagagatctggaggaataccggtggcgaaggcggccccctggacgaagactgacgctcaggtgcgaaagcgtggggagcaaacaggattagataccctggtagtccacgccgtaaacgatgtcgacttggaggttgtgcccttgaggcgtggcttccggagctaacgcgttaagtcgaccgcctggggagtacggccgcaaggttaaaactcaaatgaattgacgggggcccgcacaagcggtggagcatgtggtttaattcgatgcaacgcgaagaaccttacctggtcttgacatccacggaagttttcagagatgagaatgtgccttcgggaaccgtgagacaggtgctgcatggctgtcgtcagctcgtgttgtgaaatgttgggttaagtcccgcaacgagcgcaacccttatcctttgttgccagcggtccggccgggaactcaaaggagactgccagtgataaactggaggaaggtggggatgacgtcaagtcatcatggcccttacgaccagggctacacacgtgctacaatggcgcatacaaagagaagcgacctcgcgagagcaagcggacctcataaagtgcgtcgtagtccggattggagtctgcaactcgactccatgaagtcggaatcgctagtaatcgtggatcagaatgccacggtgaatacgttcccgggccttgtacacaccgcccgtcacaccatgggagtgggttgcaaaagaagtaggtagcttaaccttcgggagggcgcttaccactttgtgattcatgactggggtgaagtcgtaacaaggtaaccgtaggggaacctgcggttggatcacct

SEQ ID NO: 106 - DNA, 1339 bp, Unknown
  I01
  misc_feature (139)..(139): n is a, c, g, or t
  misc_feature (237)..(237): n is a, c, g, or t
  misc_feature (248)..(248): n is a, c, g, or t
  misc_feature (308)..(309): n is a, c, g, or t
  misc_feature (311)..(313): n is a, c, g, or t
  misc_feature (489)..(489): n is a, c, g, or t
  misc_feature (1158)..(1158): n is a, c, g, or t
  misc_feature (1284)..(1284): n is a, c, g, or t
  misc_feature (1286)..(1286): n is a, c, g, or t
ctgggtgagagtggcgaacgggtgagtaatgcgtgaccgacctgccccatacaccggaatagctcctggaaacgggtggtaatgccggatgctccagttggatgcatgtccttctgggaaagattcatcggtatggganggggtcgcgtcctatcagcttgatggcggggtaacggcccaccatggcttccacgggtagccggcctgagagggcgaccggccacattgggactgagntacggcccagnctcctacgggaggcagcagtggggaatattgcacaatgggcgcaagcctgatgcagcganncnnngtgcgggatgacggccttcgggttgtaaaccgcttttgactgggagcaagcccttcggggtgagtgtacctttcgaataagcaccggctaactacgtgccagcagccgcggtaatacgtaaggtgcaagcgttatccggaattattgggcgtaaagggctcgtaagcggttcgtcncgtccggtgtgaaagtccatcgcttaacggtggatccgcgccgggtacgggcgggcttgagtgcggtaggggagactggaattcccggtgtaacggtggaatgtgtagatatcgggaagaacaccaatggcgaaggcaggtctctgggccgtcactgacgctgaggagcgaaagcgtggggagcgaacaggattagataccctggtagtccacgccgtaaacggtggatgctggatgtggggaccattccacggtctccgtgtcggagccaacgcgttaagcatcccgcctggggagtacggccgcaaggctaaaactcaaagaaattgacgggggcccgcacaagcggcggagcatgcggattaattcgatgcaacgcgaagaaccttacctgggcttgacatgttcccgacagccgtagagatacggtttcccttcggggcgggttcacaggtggtgcatggtcgtcgtcagctcgtgtcgtgagatgttgggttaagtcccgcaacgagcgcaaccctcgccctgtgttgccagcacgtcgtggtgggaactcacgggggaccgccggggtcaactcggaggaaggtggggatgacgtcagatcatcatgccccttacgtccagggcttcacgcatgctacaatggccggtacaacgggatgcganaccgcgaggtggagcggatcccttaaaaccggtctcagttcggattggagtctgcaacccgactccatgaaggcggagtcgctagtaatcgcggatcagcaacgccgcggtgaatgcgttcccggncnttgtacacaccgcccgtcaagtcatgaaagtgggtagcacccgaagccggtgg

SEQ ID NO: 107 - DNA, 1346 bp, Unknown
  I02
  misc_feature (911)..(913): n is a, c, g, or t
  misc_feature (923)..(923): n is a, c, g, or t
ttgcttggtggtgagagtggcgaacgggtgagtaatgcgtgaccgacctgccccatacaccggaatagctcctggaaacgggtggtaatgccggatgctccgactcctcgcatggggtgtcgggaaagatttcatcggtatgggatggggtcgcgtcctatcaggtagtcggcggggtaacggcccaccgagcctacgacgggtagccggcctgagagggcgaccggccacattgggactgagatacggcccagactcctacgggaggcagcagtggggaatattgcacaatgggcgcaagcctgatgcagcgacgccgcgtgcgggatgacggccttcgggttgtaaaccgcttttgatcgggagcaagccttcgggtgagtgtacctttcgaataagcaccggctaactacgtgccagcagccgcggtaatacgtagggtgcaagcgttatccggaattattgggcgtaaagggctcgtaggcggttcgtcgcgtccggtgtgaaagtccatcgcttaacggtggatctgcgccgggtacgggcgggctggagtgcggtaggggagactggaattcccggtgtaacggtggaatgtgtagatatcgggaagaacaccaatggcgaaggcaggtctctgggccgttactgacgctgaggagcgaaagcgtggggagcgaacaggattagataccctggtagtccacgccgtaaacggtggatgctggatgtggggcccgttccacgggttccgtgtcggagctaacgcgttaagcatcccgcctggggagtacggccgcaaggctaaaactcaaagaaattgacgggggcccgcacaagcggcggagcatgcggattaattcgatgcaacgcgaagaaccttacctgggcttgacatgttcccgacagcnnnagagatatgncctcccttcggggcgggttcacaggtggtgcatggtcgtcgtcagctcgtgtcgtgagatgttgggttaagtcccgcaacgagcgcaaccctcgccctgtgttgccagcacgtcgtggtgggaactcacgggggaccgccggggtcaactcggaggaaggtggggatgacgtcagatcatcatgccccttacgtccagggcttcacgcatgctacaatggccggtacaacgggatgcgacacggcgacgtggagcggatccctgaaaaccggtctcagttcggattggagtctgcaacccgactccatgaaggcggagtcgctagtaatcgcggatcagcaacgccgcggtgaatgcgttcccgggccttgtacacaccgcccgtcaagtcatgaaagtgggtagcacccgaagccggtggcc

SEQ ID NO: 108 - DNA, 1353 bp, Unknown
  I03
aagcttgcttggtggtgagagtggcgaacgggtgagtaatgcgtgaccgacctgccccatgctccggaatagctcctggaaacgggtggtaatgccggatgttccacatgatcgcatgtgattgtgggaaagattctatcggcgtgggatggggtcgcgtcctatcagcttgttggtgaggtaacggctcaccaaggcttcgacgggtagccggcctgagagggcgaccggccacattgggactgagatacggcccagactcctacgggaggcagcagtggggaatattgcacaatgggcgcaagcctgatgcagcgacgccgcgtgagggatggaggccttcgggttgtaaacctcttttgtttgggagcaagccttcgggtgagtgtacctttcgaataagcgccggctaactacgtgccagcagccgcggtaatacgtagggcgcaagcgttatccggatttattgggcgtaaagggctcgtaggcggctcgtcgcgtccggtgtgaaagtccatcgcttaacggtggatctgcgccgggtacgggcgggctggagtgcggtaggggagactggaattcccggtgtaacggtggaatgtgtagatatcgggaagaacaccgatggcgaaggcaggtctctgggccgtcactgacgctgaggagcgaaagcgtggggagcgaacaggattagataccctggtagtccacgccgtaaacggtggacgctggatgtggggcacgttccacgtgttccgtgtcggagctaacgcgttaagcgtcccgcctggggagtacggccgcaaggctaaaactcaaagaaattgacgggggcccgcacaagcggcggagcatgcggattaattcgatgcaacgcgaagaaccttacctgggcttgacatgttcccgacgacgccagagatggcgtttcccttcggggcgggttcacaggtggtgcatggtcgtcgtcagctcgtgtcgtgagatgttgggttaagtcccgcaacgagcgcaaccctcgccccgtgttgccagcacgttatggtgggaactcacgggggaccgccggggttaactcggaggaaggtggggatgacgtcagatcatcatgccccttacgtccagggcttcacgcatgctacaatggccggtacagcgggatgcgacatggcgacatggagcggatccctgaaaaccggtctcagttcggatcggagcctgcaacccggctccgtgaaggcggagtcgctagtaatcgcggatcagcaacgccgcggtgaatgcgttcccgggccttgtacacaccgcccgtcaagtcatgaaagtgggcagcacccgaagccggtggcctaa

SEQ ID NO: 109 - DNA, 1338 bp, Unknown
  I04
ggtggtgagagtggcgaacgggtgagtaatgcgtgaccgacctgccccatacaccggaatagctcctggaaacgggtggtaatgccggatgctccagttgatcgcatggtcttctgggaaagctttcgcggtatgggatggggtcgcgtcctatcagcttgacggcggggtaacggcccaccgtggcttcgacgggtagccggcctgagagggcgaccggccacattgggactgagatacggcccagactcctacgggaggcagcagtggggaatattgcacaatgggcgcaagcctgatgcagcgacgccgcgtgagggatggaggccttcgggttgtaaacctcttttatcggggagcaagcgagagtgagtttacccgttgaataagcaccggctaactacgtgccagcagccgcggtaatacgtagggtgcaagcgttatccggaattattgggcgtaaagggctcgtaggcggttcgtcgcgtccggtgtgaaagtccatcgcttaacggtggatccgcgccgggtacgggcgggcttgagtgcggtaggggagactggaattcccggtgtaacggtggaatgtgtagatatcgggaagaacaccaatggcgaaggcaggtctctgggccgttactgacgctgaggagcgaaagcgtggggagcgaacaggattagataccctggtagtccacgccgtaaacggtggatgctggatgtggggcccgttccacgggttccgtgtcggagctaacgcgttaagcatcccgcctggggagtacggccgcaaggctaaaactcaaagaaattgacgggggcccgcacaagcggcggagcatgcggattaattcgatgcaacgcgaagaaccttacctgggcttgacatgttcccgacggtcgtagagatgcggcttcccttcggggcgggttcacaggtggtgcatggtcgtcgtcagctcgtgtcgtgagatgttgggttaagtcccgcaacgagcgcaaccctcgccccgtgttgccagcggattatgccgggaactcacgggggaccgccggggttaactcggaggaaggtggggatgacgtcagatcatcatgccccttacgtccagggcttcacgcatgctacaatggccggtacaacgggatgcgacgcggcgacgcggagcggatccctgaaaaccggtctcagttcggatcgcagtctgcaactcgactgcgtgaaggcggagtcgctagtaatcgcgaatcagcaacgtcgcggtgaatgcgttcccgggccttgtacacaccgcccgtcaagtcatgaaagtgggcagcacccgaagccggtggcct

SEQ ID NO: 110 - DNA, 1326 bp, Unknown
  I05
gatagaagcgagtggcgaacggctgagtaacacgtggagaacctgccccctcccccgggatagccgcccgaaaggacgggtaataccggataccccggggtgccgcatggcaccccggctaaagccccgacgggaggggatggctccgcggcccatcaggtagacggcggggtgacggcccaccgtgccgacaacgggtagccgggttgagagaccgaccggccagattgggactgagacacggcccagactcctacgggaggcagcagtggggaatcttgcgcaatggggggaaccctgacgcagcgacgccgcgtgcgggacggaggccttcgggtcgtaaaccgctttcagcagggaagagtcaagactgtacctgcagaagaagccccggctaactacgtgccagcagccgcggtaatacgtagggggcgagcgttatccggattcattgggcgtaaagcgcgcgtaggcggcccggcaggccgggggtcgaagcggggggctcaaccccccgaagcccccggaacctccgcggcttgggtccggtaggggagggtggaacacccggtgtagcggtggaatgcgcagatatcgggtggaacaccggtggcgaaggcggccctctgggccgagaccgacgctgaggcgcgaaagctgggggagcgaacaggattagataccctggtagtcccagccgtaaacgatggacgctaggtgtggggggacgatccccccgtgccgcagccaacgcattaagcgtcccgcctggggagtacggccgcaaggctaaaactcaaaggaattgacgggggcccgcacaagcagcggagcatgtggcttaattcgaagcaacgcgaagaaccttaccagggcttgacatatgggtgaagcgggggagaccccgtggccgagaggagcccatacaggtggtgcatggctgtcgtcagctcgtgtcgtgagatgttgggttaagtcccgcaacgagcgcaacccccgccgcgtgttgccatcgggtgatgccgggaacccacgcgggaccgccgccgtcaaggcggaggagggcggggacgacgtcaagtcatcatgccccttatgccctgggctgcacacgtgctacaatggccggtacagagggatgccaccccgcgagggggagcggatcccggaaagccggccccagttcggattgggggctgcaacccgcccccatgaagtcggagttgctagtaatcgcggatcagcatgccgcggtgaatgcgttcccgggccttgtacacaccgcccgtcacaccacccgagtcgtctgcacccgaagtcgccggc

SEQ ID NO: 111 - DNA, 729 bp, Unknown
  I06
  misc_feature (13)..(13): n is a, c, g, or t
acctgccttcggncagaagcgagtggcgaacggctgagtaacacgtggagaacctgccccctcccccgggatagccgcccgaaaggacgggtaataccggataccccggggtgccgcatggcaccccggctaaagccccgacgggaggggatggctccgcggcccatcaggtagacggcggggtgacggcccaccgtgccgacaacgggtagccgggttgagagaccgaccggccagattgggactgagacacggcccagactcctacgggaggcagcagtggggaatcttgcgcaatggggggaaccctgacgcagcgacgccgcgtgcgggacggaggccttcgggtcgtaaaccgctttcagcagggaagagtcaagactgtacctgcagaagaagccccggctaactacgtgccagcagccgcggtaatacgtagggggcgagcgttatccggattcattgggcgtaaagcgcgcgtaggcggcccggcaggccgggggtcgaagcggggggctcaacccctcgaagcccccggaacctccgcggcttgggtccggtaggggagggtggaacacccggtgtagcggtggaatgcgcagatatcgggtggaacaccggtggcgaaggcggccctctgggccgagaccgacgctgaggcgcgaaagctgggggagcgaacaggattagataccctggtagtcccagccgtaaacgatggacgctagg

SEQ ID NO: 112 - DNA, 1338 bp, Unknown
  I07
gtggtgagagtggcgaacgggtgagtaatgcgtgaccgacctgccccatacaccggaatagctcctggaaacgggtggtaatgccggatgctccagttgatcgcatggtcttctgggaaagctttcgcggtatgggatggggtcgcgtcctatcagcttgacggcggggtaacggcccaccgtggcttcgacgggtagccggcctgagagggcgaccggccacattgggactgagatacggcccagactcctacgggaggcagcagtggggaatattgcacaatgggcgcaagcctgatgcagcgacgccgcgtgagggatggaggccttcgggttgtaaacctcttttatcggggagcaagcgagagtgagtttacccgttgaataagcaccggctaactacgtgccagcagccgcggtaatacgtagggtgcaagcgttatccggaattattgggcgtaaagggctcgtaggcggttcgtcgcgtccggtgtgaaagtccatcgcttaacggtggatccgcgccgggtacgggcgggcttgagtgcggtaggggagactggaattcccggtgtaacggtggaatgtgtagatatcgggaagaacaccaatggcgaaggcaggtctctgggccgttactgacgctgaggagcgaaagcgtggggagcgaacaggattagataccctggtagtccacgccgtaaacggtggatgctggatgtggggcccgttccacgggttccgtgtcggagctaacgcgttaagcatcccgcctggggagtacggccgcaaggctaaaactcaaagaaattgacgggggcccgcacaagcggcggagcatgcggattaattcgatgcaacgcgaagaaccttacctgggcttgacatgttcccgacggtcgtagagatgcggcttcccttcggggcgggttcacaggtggtgcatggtcgtcgtcagctcgtgtcgtgagatgttgggttaagtcccgcaacgagcgcaaccctcgccccgtgttgccagcggattatgccgggaactcacgggggaccgccggggttaactcggaggaaggtggggatgacgtcagatcatcatgccccttacgtccagggcttcacgcatgctacaatggccggtacaacgggatgcgacgcggcgacgcggagcggatccctgaaaaccggtctcagttcggatcgcagtctgcaactcgactgcgtgaaggcggagtcgctagtaatcgcgaatcagcaacgtcgcggtgaatgcgttcccgggccttgtacacaccgcccgtcaagtcatgaaagtgggcagcacccgaagccggtggccta

SEQ ID NO: 113 - DNA, 1337 bp, Unknown
  I08
  misc_feature (105)..(105): n is a, c, g, or t
  misc_feature (117)..(119): n is a, c, g, or t
ttgatggatggcgaccggcgcacgggtgagtaacacgtatccaacctgccgacaacactgggatagcctttcgaaagaaagattaataccggatggcataattantccgcatgggannnttattaaagaatttcggttgtcgatggggatgcgttccattaggcagttggcggggtaacggcccaccaaaccaacgatggataggggttctgagaggaaggtcccccacattggaactgagacacggtccaaactcctacgggaggcagcagtgaggaatattggtcaatggacgagagtctgaaccagccaagtagcgtgaaggatgactgccctatgggttgtaaacttcttttatacgggaataaagttagccacgtgtggctttttgtatgtaccgtatgaataaggatcggctaactccgtgccagcagccgcggtaatacggaggatccgagcgttatccggatttattgggtttaaagggagcgtaggcgggttgttaagtcagttgtgaaagtttgcggctcaaccgtaaaattgcagttgatactggcgaccttgagtgcaacagaggtaggcggaattcgtggtgtagcggtgaaatgcttagatatcacgaagaactccgattgcgaaggcagcttactggattgtaactgacgctgatgctcgaaagtgtgggtatcaaacaggattagataccctggtagtccacacagtaaacgatgaatactcgctgttggcgatatactgtcagcggccaagcgaaagcattaagtattccacctggggagtacgccggcaacggtgaaactcaaaggaattgacgggggcccgcacaagcggaggaacatgtggtttaattcgatgatacgcgaggaaccttacccgggcttaaattgcaactgacggaatcggaaacggttctttcttcggacagttgtgaaggtgctgcatggttgtcgtcagctcgtgccgtgaggtgtcggcttaagtgccataacgagcgcaacccttacgggtagttaccatcaggttatgctggggactctacccggactgccgtcgtaagatgtgaggaaggtggggatgacgtcaaatcagcacggcccttacgtccggggctacacacgtgttacaatggggggtacagaaggcagctacacggcgacgtggtgctaatcccgaaagcctctctcagttcggattggagtctgcaacccgactccatgaagctggattcgctagtaatcgcgcatcagccacggcgcggtgaatacgttcccgggccttgtacacaccgcccgtcaagccatgaaagccgggggtacctg

SEQ ID NO: 114 - DNA, 1353 bp, Unknown
  I09
ttagcttgctaaggccgatggcgaccggcgcacgggtgagtaacgcgtatccaacctgccttacactcttggacagccttctgaaagggagattaatacaagatgttatcatgagtaagcattttcgcatgattaaaggtttaccggtgtaagatggggatgcgttccattagatagtaggcggggtaacggcccacctagtcttcgatggataggggttctgagaggaaggtcccccacattggaactgagacacggtccaaactcctacgggaggcagcagtgaggaatattggtcaatggacgagagtctgaaccagccaagtagcgtgaaggatgaaggttctatggattgtaaacttcttttatacgggaataaacgaatccacgcgtggatttttgcatgtaccgtatgaataaggatcggctaactccgtgccagcagccgcggtaatacggaggatccgagcgttatccggatttattgggtttaaagggagcgtagatgggttgttaagtcagttgtgaaagtttgcggctcaaccgtaaaattgcaattgatactggcagtcttgagtacagttgaggtaggcggaattcgtggtgtagcggtgaaatgcttagatatcacgaagaactccgattgcgaaggcagcttactaacctgtaactgacattgatgctcgaaagtgtgggtatcaaacaggattagataccctggtagtccacacggtaaacgatgaatactcgctgtaggcgatatacggtctgcggccaagcgaaagcattaagtattccacctggggagtacgccggcaacggtgaaactcaaaggaattgacgggggcccgcacaagcggaggaacatgtggtttaattcgatgatacgcgaggaaccttacccgggcttaaattgcaaccgaatatggcggaaacgccatagctagcaatagcggttgtgaaggtgctgcatggttgtcgtcagctcgtgccgtgaggtgtcggcttaagtgccataacgagcgcaacccttgccgatagttactaacaggttatgctgaggactctgtcgggactgccatcgtaagatgtgaggaaggtggggatgacgtcaaatcagcacggcccttacgtccggggctacacacgtgttacaatggggggtacagagggctgctaccacgcaagtggatgccaatcccaaaaacctctctcagttcggattgaagtctgcaacccgacttcatgaagctggattcgctagtaatcgcgcatcagccacggcgcggtgaatacgttcccgggccttgtacacaccgcccgtcaagccatgggagccgggggtacctgaag

SEQ ID NO: 115 - DNA, 1350 bp, Unknown
  I10
cttagcttgctaaggccgatggcgaccggcgcacgggtgagtaacacgtatccaacctgccgtctactcttggacagccttctgaaaggaagattaatacaagatggcatcatgagtccgcatgttcacatgattaaaggtattccggtagacgatggggatgcgttccattagatagtaggcggggtaacggcccacctagtcttcgatggataggggttctgagaggaaggtcccccacattggaactgagacacggtccaaactcctacgggaggcagcagtgaggaatattggtcaatgggcgagagcctgaaccagccaagtagcgtgaaggatgactgccctatgggttgtaaacttcttttataaaggaataaagtcgggtatggatacccgtttgcatgtactttatgaataaggatcggctaactccgtgccagcagccgcggtaatacggaggatccgagcgttatccggatttattgggtttaaagggagcgtagatggatgtttaagtcagttgtgaaagtttgcggctcaaccgtaaaattgcagttgatactggatatcttgagtgcagttgaggcaggcggaattcgtggtgtagcggtgaaatgcttagatatcacgaagaactccgattgcgaaggcagcctgctaagctgcaactgacattgaggctcgaaagtgtgggtatcaaacaggattagataccctggtagtccacacggtaaacgatgaatactcgctgtttgcgatatactgcaagcggccaagcgaaagcgttaagtattccacctggggagtacgccggcaacggtgaaactcaaaggaattgacgggggcccgcacaagcggaggaacatgtggtttaattcgatgatacgcgaggaaccttacccgggcttaaattgcagatgaattacggtgaaagccgtaagccgcaaggcatctgtgaaggtgctgcatggttgtcgtcagctcgtgccgtgaggtgtcggcttaagtgccataacgagcgcaacccttgttgtcagttactaacaggttccgctgaggactctgacaagactgccatcgtaagatgtgaggaaggtggggatgacgtcaaatcagcacggcccttacgtccggggctacacacgtgttacaatggggggtacagagggccgctaccacgcgagtggatgccaatccccaaaacctctctcagttcggactggagtctgcaacccgactccacgaagctggattcgctagtaatcgcgcatcagccacggcgcggtgaatacgttcccgggccttgtacacaccgcccgtcaagccatgggagccgggggtacctga

SEQ ID NO: 116 - DNA, 1356 bp, Unknown
  I11
tcttagcttgctaaggctgatggcgaccggcgcacgggtgagtaacacgtatccaacctgccgtctactcttggccagccttctgaaaggaagattaatccaggatgggatcatgagttcacatgtccgcatgattaaaggtattttccggtagacgatggggatgcgttccattagatagtaggcggggtaacggcccacctagtcaacgatggataggggttctgagaggaaggtcccccacattggaactgagacacggtccaaactcctacgggaggcagcagtgaggaatattggtcaatgggcgatggcctgaaccagccaagtagcgtgaaggatgactgccctatgggttgtaaacttcttttataaaggaataaagtcgggtatgcatacccgtttgcatgtactttatgaataaggatcggctaactccgtgccagcagccgcggtaatacggaggatccgagcgttatccggatttattgggtttaaagggagcgtagatggatgtttaagtcagttgtgaaagtttgcggctcaaccgtaaaattgcagttgatactggatgtcttgagtgcagttgaggcaggcggaattcgtggtgtagcggtgaaatgcttagatatcacgaagaactccgattgcgaaggcagcctgctaagctgcaactgacattgaggctcgaaagtgtgggtatcaaacaggattagataccctggtagtccacacggtaaacgatgaatactcgctgtttgcgatatacggcaagcggccaagcgaaagcgttaagtattccacctggggagtacgccggcaacggtgaaactcaaaggaattgacgggggcccgcacaagcggaggaacatgtggtttaattcgatgatacgcgaggaaccttacccgggcttaaattgcactcgaatgatccggaaacggttcagctagcaatagcgagtgtgaaggtgctgcatggttgtcgtcagctcgtgccgtgaggtgtcggcttaagtgccataacgagcgcaacccttgttgtcagttactaacaggtgatgctgaggactctgacaagactgccatcgtaagatgtgaggaaggtggggatgacgtcaaatcagcacggcccttacgtccggggctacacacgtgttacaatggggggtacagagggccgctaccacgcgagtggatgccaatccctaaaacccctctcagttcggactggagtctgcaacccgactccacgaagctggattcgctagtaatcgcgcatcagccacggcgcggtgaatacgttcccgggccttgtacacaccgcccgtcaagccatgggagccgggggtacctgaa

SEQ ID NO: 117 - DNA, 1353 bp, Unknown
  I12
  misc_feature (6)..(6): n is a, c, g, or t
  misc_feature (8)..(8): n is a, c, g, or t
tgtagnantacagattgatggcgaccggcgcacgggtgagtaacgcgtatgcaacttacctatcagagggggatagcccggcgaaagtcggattaataccccataaaacaggggtcccgcatgggaatatttgttaaagattcatcgctgatagataggcatgcgttccattaggcagttggcggggtaacggcccaccaaaccgacgatggataggggttctgagaggaaggtcccccacattggtactgagacacggaccaaactcctacgggaggcagcagtgaggaatattggtcaatggccgagaggctgaaccagccaagtcgcgtgaaggaagaaggatctatggtttgtaaacttcttttataggggaataaagtggaggacgtgtccttttttgtatgtaccctatgaataagcatcggctaactccgtgccagcagccgcggtaatacggaggatgcgagcgttatccggatttattgggtttaaagggtgcgtaggtggtgatttaagtcagcggtgaaagtttgtggctcaaccataaaattgccgttgaaactgggttacttgagtgtgtttgaggtaggcggaatgcgtggtgtagcggtgaaatgcatagatatcacgcagaactccgattgcgaaggcagcttactaaaccataactgacactgaagcacgaaagcgtggggatcaaacaggattagataccctggtagtccacgcagtaaacgatgattactaggagtttgcgatacaatgtaagctctacagcgaaagcgttaagtaatccacctggggagtacgccggcaacggtgaaactcaaaggaattgacgggggcccgcacaagcggaggaacatgtggtttaattcgatgatacgcgaggaaccttacccgggtttgaacgtagtctgaccggagtggaaacactccttctagcaatagcagattacgaggtgctgcatggttgtcgtcagctcgtgccgtgaggtgtcggcttaagtgccataacgagcgcaacccttatcactagttactaacaggtgaagctgaggactctggtgagactgccagcgtaagctgtgaggaaggtggggatgacgtcaaatcagcacggcccttacatccggggcgacacacgtgttacaatggcatggacaaagggcagctacctggcgacaggatgctaatctccaaaccatgtctcagttcggatcggagtctgcaactcgactccgtgaagctggattcgctagtaatcgcgcatcagccatggcgcggtgaatacgttcccgggccttgtacacaccgcccgtcaagccatgggagccgggggtacctgaa

SEQ ID NO: 118 - DNA, 824 bp, Unknown
  I13
ggcgaccggcgcacgggtgagtaacgcgtatgcaacttacctatcagagggggataacccggcgaaagtcggactaataccgcatgaagcaggggccccgcatggggatatttgctaaagattcatcgctgatagataggcatgcgttccattaggcagttggcggggtaacggcccaccaaaccgacgatggataggggttctgagaggaaggtcccccacattggtactgagacacggaccaaactcctacgggaggcagcagtgaggaatattggtcaatgggcgtaagcctgaaccagccaagtcgcgtgagggatgaaggttctatggatcgtaaacctcttttataagggaataaagtgcgggacgtgtcctgttttgtatgtaccttatgaataaggatcggctaactccgtgccagcagccgcggtaatacggaggatccgagcgttatccggatttattgggtttaaagggtgcgtaggcggccttttaagtcagcggtgaaagtctgtggctcaaccatagaattgccgttgaaactggggggcttgagtatgtttgaggcaggcggaatgcgtggtgtagcggtgaaatgcttagatatcacgcagaaccccgattgcgaaggcagcctgccaagccatgactgacgctgatgcacgaaagcgtggggatcaaacaggattagataccctggtagtccacgcagtaaacgatgatcactagctgtttgcgatacagtgtaagcggcacagcgaaagcgttaagtgatccacctggggagtacgccggcaacggtgaaactcaaaggaattgac

SEQ ID NO: 119 - DNA, 1348 bp, Unknown
  I14
gatagcaatatctatggtggcgaccggcgcacgggtgcgtaacgcgtatgcaacctacctttaacagggggataacactgagaaattggtactaataccccataatatcatagaaggcatcttttatggttgaaaattccgatggttagagatgggcatgcgttgtattagctagttggtggggtaacggctcaccaaggcgacgatacatagggggactgagaggttaaccccccacactggtactgagacacggaccagactcctacgggaggcagcagtgaggaatattggtcaatggacgcaagtctgaaccagccatgccgcgtgcaggatgacggctctatgagttgtaaactgcttttgtacgagggtaaacgcagatacgtgtatctgtctgaaagtatcgtacgaataaggatcggctaactccgtgccagcagccgcggtaatacggaggattcaagcgttatccggatttattgggtttaaagggtgcgtaggcggtttgataagttagaggtgaaatttcggggctcaaccctgaacgtgcctctaatactgttgagctagagagtagttgcggtaggcggaatgtatggtgtagcggtgaaatgcttagagatcatacagaacaccgattgcgaaggcagcttaccaaactatatctgacgttgaggcacgaaagcgtggggagcaaacaggattagataccctggtagtccacgcagtaaacgatgataactcgttgtcggcgatacacagtcggtgactaagcgaaagcgataagttatccacctggggagtacgttcgcaagaatgaaactcaaaggaattgacgggggcccgcacaagcggaggaacatgtggtttaattcgatgatacgcgaggaaccttacccgggcttgaaagttagcgacgattcttgaaagaggatttcccttcggggcgcgaaactaggtgctgcatggttgtcgtcagctcgtgccgtgaggtgtcgggttaagtcccataacgagcgcaacccctaccgttagttgccatcaggtgaagctgggcactctggcgggactgccggtgtaagccgagaggaaggtggggatgacgtcaaatcagcacggcccttacgtccggggctacacacgtgttacaatggtaggtacagagggcagctacccagcgatgggatgcgaatctcgaaagcctatctcagttcggattggaggctgaaacccgcctccatgaagttggattcgctagtaatcgcgcatcagccatggcgcggtgaatacgttcccgggccttgtacacaccgcccgtcaagccatgggagccgggggtgcctga

SEQ ID NO: 120 - DNA, 1337 bp, Unknown
  I15
  misc_feature (838)..(839): n is a, c, g, or t
ttctttgctggcgaccggcgcacgggtgagtaacacgtatccaacctgccgatgactcggggatagcctttcgaaagaaagattaatacccgatggtatatctgaaaggcatctttcagctattaaagaatttcggtcattgatggggatgcgttccattaggttgttggcggggtaacggcccaccaagccatcgatggataggggttctgagaggaaggtcccccacattggaactgagacacggtccaaactcctacgggaggcagcagtgaggaatattggtcaatggacgagagtctgaaccagccaagtagcgtgaaggatgactgccctatgggttgtaaacttcttttatacgggaataaagttgggcacgtgtgcctttttgtatgtaccgtatgaataaggatcggctaactccgtgccagcagccgcggtaatacggaggatccgagcgttatccggatttattgggtttaaagggagcgtaggcggatgcttaagtcagttgtgaaagtttgcggctcaaccgtaaaattgcagttgatactgggtgtcttgagtacagtagaggcaggcggaattcgtggtgtagcggtgaaatgcttagatatcacgaagaactccgattgcgaaggcagcttgctggactgtaactgacgctgatgctcgaaagtgtgggtatcaaacaggattagataccctggtagtccacacagtaaacgatgaatactcgctgtttgcgatatacagtaagcggccaagcgaaagcgttaagtattccacctggggagtacgccggcaacggtgaaactcaaaggaattgacgggggcnngcacaagcggaggaacatgtggtttaattcgatgatacgcgaggaaccttacccgggcttaaattgcaaatgaatgttctggaaacagatcagccgcaaggcatttgtgaaggtgctgcatggttgtcgtcagctcgtgccgtgaggtgtcggcttaagtgccataacgagcgcaacccttatcgatagttaccatcaggttatgctggggactctgtcgagactgccgtcgtaagatgtgaggaaggtggggatgacgtcaaatcagcacggcccttacgtccggggctacacacgtgttacaatggggggtacagaaggcagctacacggcgacgtgatgctaatccctaaaacctctctcagttcggattggagtctgcaacccgactccatgaagctggattcgctagtaatcgcgcatcagccacggcgcggtgaatacgttcccgggccttgtacacaccgcccgtcaagccatgaaagccgggggtacctg

SEQ ID NO: 121 - DNA, 1343 bp, Unknown
  I16
  misc_feature (5)..(5): n is a, c, g, or t
  misc_feature (7)..(7): n is a, c, g, or t
  misc_feature (110)..(113): n is a, c, g, or t
  misc_feature (337)..(338): n is a, c, g, or t
  misc_feature (1170)..(1170): n is a, c, g, or t
cttgnanactgaagatggcgaccggcgcacgggtgagtaacacgtatccaacctgccgataactccggaatagcctttcgaaagaaagattaataccggatagcatacgnnnntcgcatgatatttttattaaagaatttcggttatcgatggggatgcgttccattagtttgttggcggggtaacggcccaccaagactacgatggataggggttctgagaggaaggtcccccacattggaactgagacacggtccaaactcctacgggaggcagcagtgaggaatattggtcaatgggcgagagcctgaaccagccaagtagcgtgaaggatganngctctatgggtcgtaaacttcttttatatgggaataaagttttccacgtgtggaattttgtatgtaccatatgaataaggatcggctaactccgtgccagcagccgcggtaatacggaggatccgagcgttatccggatttattgggtttaaagggagcgtaggtggattgttaagtcagttgtgaaagtttgcggctcaaccgtaaaattgcagttgaaactggcagtcttgagtacagtagaggtgggcggaattcgtggtgtagcggtgaaatgcttagatatcacgaagaactccgattgcgaaggcagctcactagactgtcactgacactgatgctcgaaagtgtgggtatcaaacaggattagataccctggtagtccacacagtaaacgatgaatactcgctgtttgcgatatacagtaagcggccaagcgaaagcattaagtattccacctggggagtacgccggcaacggtgaaactcaaaggaattgacgggggcccgcacaagcggaggaacatgtggtttaattcgatgatacgcgaggaaccttacccgggcttaaattgcaacagaatatattggaaacagtatagccgtaaggctgttgtgaaggtgctgcatggttgtcgtcagctcgtgccgtgaggtgtcggcttaagtgccataacgagcgcaacccttatctttagttactaacaggtcatgctgaggactctagagagactgccgtcgtaagatgtgaggaaggtggggatgacgtcaaatcagcacggcccttacgtccggggctacacacgtgttacaatggggggtacagaaggcanctacctggtgacaggatgctaatcccaaaaacctctctcagttcggatcgaagtctgcaacccgacttcgtgaagctggattcgctagtaatcgcgcatcagccatggcgcggtgaatacgttcccgggccttgtacacaccgcccgtcaagccatgaaagccgggggtacct

SEQ ID NO: 122 - DNA, 1335 bp, Unknown
  I17
gggtggcgaccggcgcacgggtgcgtaacgcgtatgcaacctacccataacagggggataacactgagaaattggtactaataccccataacatcagaaccggcatcggttttggttgaaaactccggtggttatggatgggcatgcgttgtattagctggttggtgaggtaacggctcaccaaggcaacgatacatagggggactgagaggttaaccccccacattggtactgagacacggaccaaactcctacgggaggcagcagtgaggaatattggtcaatggacgcaagtctgaaccagccatgccgcgtgcaggaagacggctctatgagttgtaaactgcttttgtacgagggtaaacgcttctacgtgtaggagcctgaaagtatcgtacgaataaggatcggctaactccgtgccagcagccgcggtaatacggaggatccaagcgttatccggatttattgggtttaaagggtgcgtaggcggtttgataagttagaggtgaaataccggtgcttaacaccggaactgcctctaatactgttgaactagagagtagttgcggtaggcggaatgtatggtgtagcggtgaaatgcttagagatcatacagaacaccgattgcgaaggcagcttaccaaactatatctgacgttgaggcacgaaagcgtggggagcaaacaggattagataccctggtagtccacgcagtaaacgatgataactcgctgtcggcgatacacagtcggcggctaagcgaaagcgataagttatccacctggggagtacgttcgcaagaatgaaactcaaaggaattgacgggggcccgcacaagcggaggaacatgtggtttaattcgatgatacgcgaggaaccttacccgggcttgaaagttactgacgattctggaaacaggatttcccttcggggcaggaaactaggtgctgcatggttgtcgtcagctcgtgccgtgaggtgtcgggttaagtcccataacgagcgcaacccctaccgttagttgccatcaggtcaagctgggcactctggcgggactgccggtgtaagccgagaggaaggtggggatgacgtcaaatcagcacggcccttacgtccggggctacacacgtgttacaatggtaggtacagagggcagctacccagtgatgggatgcgaatctcgaaagcctatctcagttcggatcggaggctgaaacccgcctccgtgaagttggattcgctagtaatcgcgcatcagccatggcgcggtgaatacgttcccgggccttgtacacaccgcccgtcaagccatggaagctgggggtgcctgaa

SEQ ID NO: 123 - DNA, 1309 bp, Unknown
  I18
cgtatgcaacctgcccgataccggggtatagcccatggaaacgtggattaacaccccatagtacttttatcctgcatgggatgtgagttaaatgttcaaggtatcggatgggcatgcgtcctattagttagttggcggggtaacagcccaccaagacgatgataggtaggggttctgagaggaaggtcccccacattggaactgagacacggtccaaactcctacgggaggcagcagtgaggaatattggtcaatggacgtaagtctgaaccagccaagtcgcgtgagggaagactgccctatgggttgtaaacctcttttataagggaagaataagttctacgtgtagaatgatgcctgtaccttatgaataagcatcggctaactccgtgccagcagccgcggtaatacggaggatgcgagcgttatccggatttattgggtttaaagggtgcgtaggcggtttattaagttagtggttaaatatttgagctaaactcaattgtgccattaatactggtaaactggagtacagacgaggtaggcggaataagttaagtagcggtgaaatgcatagatataacttagaactccgatagcgaaggcagcttaccagactgtaactgacgctgatgcacgagagcgtgggtagcgaacaggattagataccctggtagtccacgccgtaaacgatgctcactggttctgtgcgatatattgtacgggattaagcgaaagtattaagtgagccacctggggagtacgtcggcaacgatgaaactcaaaggaattgacgggggcccgcacaagcggaggaacatgtggtttaattcgatgatacgcgaggaaccttacctgggtttaaatgggaaatgtcgtatttggaaacagatattctcttcggagcgtttttcaaggtgctgcatggttgtcgtcagctcgtgccgtgaggtgtcgggttaagtcccataacgagcgcaacccttaccgttagttgctagcatgtaatgatgagcactctaacgggactgccaccgtaaggtgagaggaaggcggggatgacgtcaaatcagcacggcccttacacccagggctacacacgtgttacaatggccggtacagagggccgctaccaggtgactggatgccaatctcaaaagccggtcgtagttcggattggagtctgtaacccgactccatgaagttggattcgctagtaatcgcgcatcagccatggcgcggtgaatacgttcccgggccttgtacacaccgcccgtcaagccatggaagccgggggtgcctgaagtcc

SEQ ID NO: 124 - DNA, 1339 bp, Unknown
  I19
  misc_feature (10)..(10): n is a, c, g, or t
  misc_feature (124)..(125): n is a, c, g, or t
  misc_feature (183)..(183): n is a, c, g, or t
  misc_feature (190)..(191): n is a, c, g, or t
  misc_feature (911)..(911): n is a, c, g, or t
agagagcttnctttctcgagcgagtggcgaacgggtgagtaacgcgtgaggaacctgcctcaaagagggggacaacagttggaaacgactgctaataccgcataagcccacgggtcggcatcgnncagagggaaaaggagcaatccgctttgagatggcctcgcgtccgattagctagttggngaggtannggcccaccaaggcgacgatcggtagccggactgagaggttgaacggccacattgggactgagacacggcccagactcctacgggaggcagcagtggggaatattgcacaatgggggaaaccctgatgcagcgacgccgcgtggaggaagaaggtcttcggattgtaaactcctgttgttggggaagataatgacggtacccaacaaggaagtgacggctaactacgtgccagcagccgcggtaaaacgtaggtcacaagcgttgtccggaattactgggtgtaaagggagcgcaggcgggaagacaagttggaagtgaaatctatgggctcaacccataaactgctttcaaaactgtttttcttgagtagtgcagaggtaggcggaattcccggtgtagcggtggaatgcgtagatatcgggaggaacaccagtggcgaaggcggcctactgggcaccaactgacgctgaggctcgaaagtgtgggtagcaaacaggattagataccctggtagtccacaccgtaaacgatgattactaggtgttggaggattgaccccttcagtgccgcagttaacacaataagtaatccacctggggagtacgaccgcaaggttgaaactcaaaggaattgacgggggcccgcacaagcagtggagtatgtggtttaattcgacgcaacgcgaagaaccttaccaagtcttgacatcccttgacaganatagaaatatgttttctcttcggagcaaggagacaggtggtgcatggttgtcgtcagctcgtgtcgtgagatgttgggttaagtcccgcaacgagcgcaacccttatggtcagttactacgcaagaggactctggccagactgccgttgacaaaacggaggaaggtggggatgacgtcaaatcatcatgccctttatgacttgggctacacacgtactacaatggcgttaaacaaagagaagcaagaccgcgaggtggagcaaaactcagaaacaacgtcccagttcggactgcaggctgcaactcgcctgcacgaagtcggaattgctagtaatcgtggatcagcatgccacggtgaatacgttcccgggccttgtacacaccgcccgtcacaccatgagagccggggggacccgaagtcggtagtc

SEQ ID NO: 125 - DNA, 1339 bp, Unknown
  I20
  misc_feature (192)..(192): n is a, c, g, or t
  misc_feature (205)..(206): n is a, c, g, or t
  misc_feature (1337)..(1337): n is a, c, g, or t
gagagagcttgctttctcgagcgagtggcgaacgggtgagtaacgcgtgaggaacctgcctcaaagagggggacaacagttggaaacgactgctaataccgcataagcccacgggtcggcatcgaccagagggaaaaggagtaatccgctttgagatggcctcgcgtccgattagctagttggtgaggtaanggcccaccaaggnnacgatcggtagccggactgagaggttgaacggccacattgggactgagacacggcccagactcctacgggaggcagcagtggggaatattgcacaatgggggaaaccctgatgcagcgacgccgcgtggaggaagaaggtcttcggattgtaaactcctgttgttggggaagataatgacggtacccaacaaggaagtgacggctaactacgtgccagcagccgcggtaaaacgtaggtcacaagcgttgtccggaattactgggtgtaaagggagcgcaggcgggaagacaagttggaagtgaaatctatgggctcaacccataaactgctttcaaaactgtttttcttgagtagtgcagaggtaggcggaattcccggtgtagcggtggaatgcgtagatatcgggaggaacaccagtggcgaaggcggcctactgggcaccaactgacgctgaggctcgaaagtgtgggtagcaaacaggattagataccctggtagtccacaccgtaaacgatgattactaggtgttggaggattgaccccttcagtgccgcagttaacacaataagtaatccacctggggagtacgaccgcaaggttgaaactcaaaggaattgacgggggcccgcacaagcagtggagtatgtggtttaattcgacgcaacgcgaagaaccttaccaagtcttgacatcccttgacagacatagaaatatgttttctcttcggagcaaggagacaggtggtgcatggttgtcgtcagctcgtgtcgtgagatgttgggttaagtcccgcaacgagcgcaacccttatggtcagttactacgcaagaggactctggccagactgccgttgacaaaacggaggaaggtggggatgacgtcaaatcatcatgccctttatgacttgggctacacacgtactacaatggcgttaaacaaagagaagcaagaccgcgaggtggagcaaaactcagaaacaacgtcccagttcggactgcaggctgcaactcgcctgcacgaagtcggaattgctagtaatcgtggatcagcatgccacggtgaatacgttcccgggccttgtacacaccgcccgtcacaccatgagagccggggggacccgaagtcggtngt

SEQ ID NO: 126 - DNA, 1354 bp, Unknown
  I21
  misc_feature (184)..(187): n is a, c, g, or t
  misc_feature (573)..(574): n is a, c, g, or t
  misc_feature (752)..(755): n is a, c, g, or t
  misc_feature (1175)..(1176): n is a, c, g, or t
cattgagacttcggtggatttgatctatttctagtggcggacgggtgagtaacgcgtgggtaacctgccttatacagggggataacagtcagaaatggctgctaataccgcataagcgcacagagctgcatggctcagtgtgaaaaactccggtggtataagatggacccgcgttggattagcnnnntggtggggtaacggcccaccaaggcgacgatccatagccggcctgagagggtgaacggccacattgggactgagacacggcccagactcctacgggaggcagcagtggggaatattgcacaatgggggaaaccctgatgcagcgacgccgcgtgaaggaagaagtatctcggtatgtaaacttctatcagcagggaagatagtgacggtacctgactaagaagccccggctaactacgtgccagcagccgcggtaatacgtagggggcaagcgttatccggatttactgggtgtaaagggagcgtagacggtgtggcaagtctgatgtgaaaggcatgggctcaacctgtggactgcattggaaactgtcatacttgagtgccggnngggtaagcggaattcctagtgtagcggtgaaatgcgtagatattaggaggaacaccagtggcgaaggcggcttactggacggtaactgacgttgaggctcgaaagcgtggggagcaaacaggattagataccctggtagtccacgccgtaaacgatgaatactaggtgtcggggagcnnnnctcttcggtgccgtcgcaaacgcagtaagtattccacctggggagtacgttcgcaagaatgaaactcaaaggaattgacggggacccgcacaagcggtggagcatgtggtttaattcgaagcaacgcgaagaaccttaccaagtcttgacatccgcctgaccgatccttaaccggatctttccttcgggacaggcgagacaggtggtgcatggttgtcgtcagctcgtgtcgtgagatgttgggttaagtcccgcaacgagcgcaacccctatcctcagtagccagcatttaaggtgggcactctggggagactgccagggataacctggaggaaggcggggatgacgtcaaatcatcatgccccttatgatttgggctacacacgtgctacaatggcgtaaacaaagggaagcgagatnntgagatggagcaaatcccaaaaataacgtcccagttcggactgtagtctgcaacccgactacacgaagctggaatcgctagtaatcgcggatcagaatgccgcggtgaatacgttcccgggtcttgtacacaccgcccgtcacaccatgggagtcagtaacgcccgaagtcagtgacc

SEQ ID NO: 127 - DNA, 1264 bp, Unknown
  I22
  misc_feature (144)..(145): n is a, c, g, or t
ttacttggatttcttcggaatgacgagtattgtgactgagcggcggacgggtgagtaacgcgtgggtaacctgcctcatacagggggataacagttagaaatgactgctaataccgcataagaccacagcaccgcatggtgcannggtaaaaactccggtggtatgagatggacccgcgtctgattagctggttggtggggtaacggcctaccaaggcgacgatcagtagccggcctgagagggcgaccggccacattgggactgagacacggcccaaactcctacgggaggcagcagtggggaatattgcacaatgggggaaaccctgatgcagcgacgccgcgtgaaggaagaagtatttcggtatgtaaacttctatcagcagggaagaaaatgacggtacctgactaagaagccccggctaactacgtgccagcagccgcggtaatacgtagggggcccgtttttctagagtgtcggagaggtaagcggaattcctagtgtagcggtgaaatgcgtagatattaggaggaacaccagtggcgaaggcggcttactggacgatgactgacgttgaggctcgaaagcgtggggagcaaacaggattagataccctggtagtccacgccgtaaacgatgactactaggtgtcgggtggcaaagccattcggtgccgcagcaaacgcaataagtagtccacctggggagtacgttcgcaagaatgaaactcaaaggaattgacggggacccgcacaagcggtggagcatgtggtttaattcgaagcaacgcgaagaaccttacctgctcttgacatcccggtgaccgctccgtaatgggagcttttcttcggaacaccggagacaggtggtgcatggttgtcgtcagctcgtgtcgtgagatgttgggttaagtcccgcaacgagcgcaacccctatcttcagtagccagcggtttggccgggcactctggagagactgccagggataacctggaggaaggtggggatgacgtcaaatcatcatgccccttatgagcagggctacacacgtgctacaatggcgtaaacaaagggaggcgaactcgcgagggtaagcaaatcccaaaaataacgtctcagttcggattgtagtctgcaactcgactacatgaagctggaatcgctagtaatcgcgaatcagaatgtcgcggtgaatacgttcccgggtcttgtacacaccgcccgtcacaccatgggagtcagtaacgcccgaagtcagtgaccc

SEQ ID NO: 128 - DNA, 1340 bp, Unknown
  I23
gagaagcttgcttttctgatctagtggcggacgggtgagtaacacgtgagcaatctgcctttcagagggggataccgattggaaacgatcgttaataccgcataatataattgaaccgcatgatttgattatcaaagatttatcgctgaaagatgagctcgcgtctgattagctagttggtaaggtaacggcttaccaaggcgacgatcagtagccggactgagaggttgatcggccacattgggactgagacacggcccagactcctacgggaggcagcagtggggaatattgcacaatggaggaaactctgatgcagcgatgccgcgtgagggaagaaggttttaggattgtaaacctctgtcttcagggacgaaaaatgacggtacctgaggaggaagctccggctaactacgtgccagcagccgcggtaatacgtagggagcgagcgttgtccggaattactgggtgtaaagggagcgtaggcgggatcgcaagtcagatgtgaaaactatgggcttaacccataaactgcatttgaaactgtggttcttgagtgaagtagaggtaagcggaattcctagtgtagcggtgaaatgcgtagatattaggaggaacatcagtggcgaaggcggcttactgggctttaactgacgctgaggctcgaaagcgtggggagcaaacaggattagataccctggtagtccacgccgtaaacgatgattactaggtgtggggggactgaccccttccgtgccgcagcaaacgcaataagtaatccacctggggagtacgaccgcaaggttgaaactcaaaggaattgacgggggcccgcacaagcagtggagtatgtggattaattcgaagcaacgcgaagaaccttaccaggtcttgacatcgtatgcatagctcagagatgagtgaaatctcttcggagacatatagacaggtggtgcatggttgtcgtcagctcgtgtcgtgagatgttgggttaagtcccgcaacgagcgcaacccttactgttagttgctacgcaagagcactctagcaggactgccgttgacaaaacggaggaaggtggggatgacgtcaaatcatcatgccccttatgacctgggcctcacacgtactacaatggctgtcaacagagggatgcaaagccgcgaggtggagcgaacccctaaaagcagtcttagttcggattgtaggctgcaacccgcctacatgaagtcggaattgctagtaatcgcagatcagcatgctgcggtgaatacgttcccgggccttgtacacaccgcccgtcacgccatgggagtcggtaacacccgaagcctgtagtc

SEQ ID NO: 129 - DNA, 1337 bp, Unknown
  I24
  misc_feature (53)..(54): n is a, c, g, or t
  misc_feature (113)..(115): n is a, c, g, or t
  misc_feature (123)..(125): n is a, c, g, or t
  misc_feature (1155)..(1156): n is a, c, g, or t
  misc_feature (1336)..(1336): n is a, c, g, or t
agagagcttgctttctcgagcgagtggcgaacgggtgagtaacgcgtgaggannctgcctcaaagagggggacaacagttggaaacgactgctaataccgcataagcccacgnnnccgcatgnnncagagggaaaaggagtaatccgctttgagatggcctcgcgtccgattagctagttggtgaggtaacggcccaccaaggcgacgatcggtagccggactgagaggttgaacggccacattgggactgagacacggcccagactcctacgggaggcagcagtggggaatattgcacaatgggggaaaccctgatgcagcgacgccgcgtggaggaagaaggtcttcggattgtaaactcctgttgttggggaagataatgacggtacccaacaaggaagtgacggctaactacgtgccagcagccgcggtaaaacgtaggtcacaagcgttgtccggaattactgggtgtaaagggagcgcaggcgggaagacaagttggaagtgaaatctatgggctcaacccataaactgctttcaaaactgtttttcttgagtagtgcagaggtaggcggaattcccggtgtagcggtggaatgcgtagatatcgggaggaacaccagtggcgaaggcggcctactgggcaccaactgacgctgaggctcgaaagtgtgggtagcaaacaggattagataccctggtagtccacaccgtaaacgatgattactaggtgttggaggattgaccccttcagtgccgcagttaacacaataagtaatccacctggggagtacgaccgcaaggttgaaactcaaaggaattgacgggggcccgcacaagcagtggagtatgtggtttaattcgacgcaacgcgaagaaccttaccaagtcttgacatcccttgacagacatagaaatatgtaatctcttcggagcaaggagacaggtggtgcatggttgtcgtcagctcgtgtcgtgagatgttgggttaagtcccgcaacgagcgcaacccttatggtcagttactacgcaagaggactctggccagactgccgttgacaaaacggaggaaggtggggatgacgtcaaatcatcatgccctttatgacttgggctacacacgtactacaatggcgttaaacaaagagaagcnngaccgcgaggtggagcaaaactcagaaacaacgtcccagttcggactgcaggctgcaactcgcctgcacgaagtcggaattgctagtaatcgtggatcagcatgccacggtgaatacgttcccgggccttgtacacaccgcccgtcacaccatgagagccggggggacccgaagtcggtng

SEQ ID NO: 130 - DNA, 1353 bp, Unknown
  I25
  misc_feature (570)..(572): n is a, c, g, or t
gattcttcggatgaagacttttgtgactgagcggcggacgggtgagtaacgcgtgggtaacctgcctcatacagggggataacagttagaaatgactgctaataccgcataagaccacggtaccgcatggtacagtggtaaaaactccggtggtatgagatggacccgcgtctgattaggtagttggtggggtaacggcctaccaagccgacgatcagtagccgacctgagagggtgaccggccacattgggactgagacacggcccagactcctacgggaggcagcagtggggaatattgcacaatggaggaaactctgatgcagcgacgccgcgtgaaggatgaagtatttcggtatgtaaacttctatcagcagggaagaaaatgacggtacctgactaagaagccccggctaactacgtgccagcagccgcggtaatacgtagggggcaagcgttatccggatttactgggtgtaaagggagcgtagacggcacggcaagccagatgtgaaagcccggggctcaaccccgggactgcatttggaactgctgagctagagtgtcggnnnggcaagtggaattcctagtgtagcggtgaaatgcgtagatattaggaggaacaccagtggcgaaggcggcttgctggacgatgactgacgttgaggctcgaaagcgtggggagcaaacaggattagataccctggtagtccacgccgtaaacgatgactgctaggtgtcgggtggcaaagccattcggtgccgcagctaacgcaataagcagtccacctggggagtacgttcgcaagaatgaaactcaaaggaattgacggggacccgcacaagcggtggagcatgtggtttaattcgaagcaacgcgaagaaccttacctgatcttgacatcccgatgaccgcttcgtaatggaagcttttcttcggaacatcggtgacaggtggtgcatggttgtcgtcagctcgtgtcgtgagatgttgggttaagtcccgcaacgagcgcaacccctatcttcagtagccagcaggttaagctgggcactctggagagactgccagggataacctggaggaaggtggggatgacgtcaaatcatcatgccccttatgaccagggctacacacgtgctacaatggcgtaaacaaagagaagcgaactcgcgagggtaagcaaatctcaaaaataacgtctcagttcggattgtagtctgcaactcgactacatgaagctggaatcgctagtaatcgcagatcagaatgctgcggtgaatacgttcccgggtcttgtacacaccgcccgtcacaccatgggagtcagtaacgcccgaagtcagtgaccc

SEQ ID NO: 131 - DNA, 1361 bp, Unknown
  I26
  misc_feature (9)..(9): n is a, c, g, or t
  misc_feature (939)..(940): n is a, c, g, or t
  misc_feature (1052)..(1053): n is a, c, g, or t
  misc_feature (1357)..(1357): n is a, c, g, or t
cttaagttngattcttcggatgaagacttttgtgactgagcggcggacgggtgagtaacgcgtgggtaacctgcctcatacagggggataacagttagaaatggctgctaataccgcataagaccacagtactgcatggtacagtggtaaaaactccggtggtatgagatggacccgcgtctgattaggtagttggtgaggtaacggcccaccaagccgacgatcagtagccgacctgagagggtgaccggccacattgggactgagacacggcccagactcctacgggaggcagcagtggggaatattgcacaatgggcgaaagcctgatgcagcgacgccgcgtgaaggatgaagtatttcggtatgtaaacttctatcagcagggaagaaaatgacggtacctgactaagaagccccggctaactacgtgccagcagccgcggtaatacgtagggggcaagcgttatccggatttactgggtgtaaagggagcgtagacggctgtgcaagtctgaagtgaaaggcatgggctcaacctgtggactgctttggaaactgtgcagctagagtgtcggagaggtaagtggaattcctagtgtagcggtgaaatgcgtagatattaggaggaacaccagtggcgaaggcggcttactggacgatgactgacgttgaggctcgaaagcgtggggagcaaacaggattagataccctggtagtccacgccgtaaacgatgactgctaggtgtcgggtagcaaagctattcggtgccgcagctaacgcaataagcagtccacctggggagtacgttcgcaagaatgaaactcaaaggaattgacggggacccgcacaagcggtggagcatgtggtttaattcgaagcaacgcgaagaaccttacctgatcttgacatcccgatgaccgcttcgtaatggaagnntttcttcggaacatcggtgacaggtggtgcatggttgtcgtcagctcgtgtcgtgagatgttgggttaagtcccgcaacgagcgcaacccttatcttcagtagccagcattnnggatgggcactctggagagactgccagggataacctggaggaaggtggggatgacgtcaaatcatcatgccccttatgaccagggctacacacgtgctacaatggcgtaaacaaagggaagcagagccgcgaggccgagcaaatctcaaaaataacgtctcagttcggattgtagtctgcaactcgactacatgaagctggaatcgctagtaatcgcagatcagaatgctgcggtgaatacgttcccgggtcttgtacacaccgcccgtcacaccatgggagtcagtaacgcccgaagtcagtnaccc

SEQ ID NO: 132 - DNA, 1345 bp, Unknown
  I27
tttcttcggaactgaagatttggtgattgagtggcggacgggtgagtaacgcgtgggtaacctgccctgtacagggggataacagtcagaaatgactgctaataccgcataagaccacagcaccgcatggtgcaggggtaaaaactccggtggtacaggatggacccgcgtctgattagctggttggtgaggtaacggctcaccaaggcgacgatcagtagccggcttgagagagtgaacggccacattgggactgagacacggcccaaactcctacgggaggcagcagtggggaatattgcacaatgggggaaaccctgatgcagcgacgccgcgtgagtgaagaagtatctcggtatgtaaagctctatcagcagggaagaaaatgacggtacctgactaagaagccccggctaactacgtgccagcagccgcggtaatacgtagggggcaagcgttatccggaattactgggtgtaaagggtgcgtaggtggtatggcaagtcagaagtgaaaacccagggcttaactctgggactgcttttgaaactgtcagactggagtgcaggagaggtaagcggaattcctagtgtagcggtgaaatgcgtagatattaggaggaacatcagtggcgaaggcggcttactggactgaaactgacactgaggcacgaaagcgtggggagcaaacaggattagataccctggtagtccacgccgtaaacgatgaatactaggtgtcggggccgtagaggcttcggtgccgcagccaacgcagtaagtattccacctggggagtacgttcgcaagaatgaaactcaaaggaattgacggggacccgcacaagcggtggagcatgtggtttaattcgaagcaacgcgaagaaccttacctggtcttgacatccttctgaccggtccttaaccggacctttccttcgggacaggagagacaggtggtgcatggttgtcgtcagctcgtgtcgtgagatgttgggttaagtcccgcaacgagcgcaacccctatctttagtagccagcatatcaggtgggcactctagagagactgccagggataacctggaggaaggtggggacgacgtcaaatcatcatgccccttatgaccagggctacacacgtgctacaatggcgtaaacagagggaagcagcctcgtgagagtgagcaaatcccaaaaataacgtctcagttcggattgtagtctgcaactcgactacatgaagctggaatcgctagtaatcgcgaatcagaatgtcgcggtgaatacgttcccgggtcttgtacacaccgcccgtcacaccatgggagtcagtaacgcccgaagtca

SEQ ID NO: 133 - DNA, 400 bp, Unknown
  I28
  misc_feature (63)..(68): n is a, c, g, or t
  misc_feature (120)..(121): n is a, c, g, or t
gcggcggacgggtgagtaacgcgtgggtaacctgccctgtacacacggataacataccgaaannnnnnctaatacgggataacataagaaattcgcatgtttttcttatcaaagctccgnnggtacaggatggacccgcgtctgattagctagttggtgaggtaacggctcaccaaggcgacgatcagtagccgacctgagagggtgatcggccacattggaactgagacacggtccaaactcctacgggaggcagcagtggggaatattgcacaatgggcgaaagcctgatgcagcaacgccgcgtgagcaatgaaggccttcgggtcgtaaagctctgtcctcaaggaagataatgacggtacttgaggaggaagccccggctaactacgtgccagca

SEQ ID NO: 134 - DNA, 1366 bp, Unknown
  I29
gggtgctcatgacggaggattcgtccaacggattgagttacctagtggcggacgggtgagtaacgcgtgaggaacctgccttggagaggggaataacactccgaaaggagtgctaataccgcatgatgcagttgggtcgcatggctctgactgccaaagatttatcgctctgagatggcctcgcgtctgattagctagtaggcggggtaacggcccacctaggcgacgatcagtagccggactgagaggttgaccggccacattgggactgagacacggcccagactcctacgggaggcagcagtggggaatattgggcaatgggcgcaagcctgacccagcaacgccgcgtgaaggaagaaggctttcgggttgtaaacttcttttgtcggggacgaaacaaatgacggtacctgacgaataagccacggctaactacgtgccagcagccgcggtaatacgtaggtggcaagcgttatccggatttactgggtgtaaagggcgtgtaggcgggattgcaagtcagatgtgaaaactgggggctcaacctccagcctgcatttgaaactgtagttcttgagtgctggagaggcaatcggaattccgtgtgtagcggtgaaatgcgtagatatacggaggaacaccagtggcgaaggcggattgctggacagtaactgacgctgaggcgcgaaagcgtggggagcaaacaggattagataccctggtagtccacgccgtaaacgatggatactaggtgtggggggtctgaccccctccgtgccgcagttaacacaataagtatcccacctggggagtacgatcgcaaggttgaaactcaaaggaattgacgggggcccgcacaagcggtggagtatgtggtttaattcgaagcaacgcgaagaaccttaccagggcttgacatcccactaacgaggcagagatgcgttaggtgcccttcggggaaagtggagacaggtggtgcatggttgtcgtcagctcgtgtcgtgagatgttgggttaagtcccgcaacgagcgcaacccttattgttagttgctacgcaagagcactctagcgagactgccgttgacaaaacggaggaaggtggggacgacgtcaaatcatcatgccccttatgtcctgggccacacacgtactacaatggtggtaaacagagggaggcaataccgcgaggtggagcaaatccctaaaagccatcccagttcggattgcaggctgaaacccgcctgtatgaagttggaatcgctagtaatcgcggatcagcatgccgcggtgaatacgttcccgggccttgtacacaccgcccgtcacaccatgagagtcgggaacacccgaagtccgtagcc

SEQ ID NO: 135 - DNA, 1358 bp, Unknown
  I30
ttagaaagaggattcgtccaattgataaggttacttagtggcggacgggtgagtaacgcgtgaggaacctgcctcggagtggggaataacagaccgaaaggcctgctaataccgcatgatgcagttggaccgcatggtcctgactgccaaagatttatcgctctgagatggcctcgcgtctgattagcttgttggcggggtaatggcccaccaaggcgacgatcagtagccggactgagaggttggccggccacattgggactgagacacggcccagactcctacgggaggcagcagtggggaatattgggcaatgggcgcaagcctgacccagcaacgccgcgtgaaggaagaaggctttcgggttgtaaacttcttttctcagggacgaacaaatgacggtacctgaggaataagccacggctaactacgtgccagcagccgcggtaatacgtaggtggcaagcgttatccggatttactgggtgtaaagggcgtgtaggcgggaaggcaagtcagatgtgaaaactatgggctcaacccatagcctgcatttgaaactgtttttcttgagtgctggagaggcaatcggaattccgtgtgtagcggtgaaatgcgtagatatacggaggaacaccagtggcgaaggcggattgctggacagtaactgacgctgaggcgcgaaagcgtggggagcaaacaggattagataccctggtagtccacgctgtaaacgatggatactaggtgtggggggtctgaccccctccgtgccgcagttaacacaataagtatcccacctggggagtacgatcgcaaggttgaaactcaaaggaattgacgggggcccgcacaagcggtggagtatgtggtttaattcgaagcaacgcgaagaaccttaccagggcttgacatcctactaacgaagcagagatgcattaggtgcccttcggggaaagtagagacaggtggtgcatggttgtcgtcagctcgtgtcgtgagatgttgggttaagtcccgcaacgagcgcaacccttattgttagttgctacgcaagagcactctagcgagactgccgttgacaaaacggaggaaggcggggacgacgtcaaatcatcatgccccttatgtcctgggctacacacgtactacaatggtggtaaacagagggaagcaagaccgcgaggtggagcaaatccctaaaagccatcccagttcggattgcaggctgaaacccgcctgtatgaagttggaatcgctagtaatcgcggatcagcatgccgcggtgaatacgttcccgggccttgtacacaccgcccgtcacaccatgagagtcgggaacacccgaagtccgtagtc

SEQ ID NO: 136 - DNA, 1342 bp, Unknown
  I31
ggcgaacgggtgagtaatacataagtaacctggcatctacagggggataactgatggaaacgtcagctaagaccgcataggtgtagagatcgcatgaactctatatgaaaagtgctacgggactggtagatgatggacttatggcgcattagctggttggtagggtaacggcctaccaaggcgacgatgcgtagccgacctgagagggtgaccggccacactgggactgagacacggcccagactcctacgggaggcagcagtagggaattttcggcaatgggggaaaccctgaccgagcaacgccgcgtgaaggaagaagtaattcgttatgtaaacttctgtcatagaggaagaacggtggatatagggaatgatatccaagtgacggtactctataagaaagccacggctaactacgtgccagcagccgcggtaatacgtaggtggcgagcgttatccggaattattgggcgtaaagagggagcaggcggcactaagggtctgtggtgaaagatcgaagcttaacttcggtaagccatggaaaccgtagagctagagtgtgtgagaggatcgtggaattccatgtgtagcggtgaaatgcgtagatatatggaggaacaccagtggcgaaggcgacgatctggcgcataactgacgctcagtcccgaaagcgtggggagcaaataggattagataccctagtagtccacgccgtaaacgatgagtactaagtgttgggagtcaaatctcagtgctgcagttaacgcaataagtactccgcctgagtagtacgttcgcaagaatgaaactcaaaggaattgacgggggcccgcacaagcggtggagcatgtggtttaattcgaagcaacgcgaagaaccttaccaggtcttgacatcgatctaaaggctccagagatggagagatagctatagagaagacaggtggtgcatggttgtcgtcagctcgtgtcgtgagatgttgggttaagtcccgcaacgagcgcaacccctgttgccagttgccagcattaagttggggactctggcgagactgccggtgacaagccggaggaaggcggggatgacgtcaaatcatcatgccccttatgacctgggctacacacgtgctacaatggacagagcagagggaagcgaagccgcgaggtggagcgaaacccataaaactgttctcagttcggactgcagtctgcaactcgactgcacgaagatggaatcgctagtaatcgcgaatcagcatgtcgcggtgaatacgttctcgggccttgtacacaccgcccgtcacaccatgagagtcggtaacacccgaagccggtggccta

SEQ ID NO: 137 - DNA, 1390 bp, Unknown
  I32
  misc_feature (921)..(923): n is a, c, g, or t
  misc_feature (972)..(972): n is a, c, g, or t
  misc_feature (983)..(983): n is a, c, g, or t
  misc_feature (990)..(991): n is a, c, g, or t
atgagaagcttgcttcttattgattcgagtggcaaacgggtgagtaacgcgtaagcaacctgcccttcagatggggacaacagctggaaacggctgctaataccgaatacgttctttttgtcgcatggcagagggaagaaagggaggctcttcggagctttcgctgaaggaggggcttgcgtctgattagctagttggaggggtaacggcccaccaaggcgacgatcagtagccggtctgagaggatgaacggccacattgggactgagacacggcccagactcctacgggaggcagcagtggggaatcttccgcaatggacgaaagtctgacggagcaacgccgcgtgaacgatgacggccttcgggttgtaaagttctgttatacgggacgaatggcgtagcggtcaatacccgttacgagtgacggtaccgtaagagaaagccacggctaactacgtgccagcagccgcggtaatacgtaggtggcaagcgttgtccggaattattgggcgtaaagggcgcgcaggcggcgtcgtaagtcggtcttaaaagtgcggggcttaaccccgtgaggggaccgaaactgcgatgctagagtatcggagaggaaagcggaattcctagtgtagcggtgaaatgcgtagatattaggaggaacaccagtggcgaaagcggctttctggacgacaactgacgctgaggcgcgaaagccaggggagcaaacgggattagataccccggtagtcctggccgtaaacgatggatactaggtgtaggaggtatcgaccccttctgtgccggagttaacgcaataagtatcccgcctggggagtacggccgcaaggctgaaactcaaaggaattgacgggggcccgcacaagcggtggagtatgtggtttaattcgacgcaacgcgaagnnncttaccaagccttgacattgattgctatggatagagatatccagttccncttcggagganaagaaannaggtggtgcacggctgtcgtcagctcgtgtcgtgagatgttgggttaagtcccgcaacgagcgcaacccctatcttctgttaccagcggttcggccggggactcaggagagactgccgcagacaatgcggaggaaggcggggatgacgtcaagtcatcatgccccttatggcttgggctacacacgtactacaatggctcttaatagagggaagcgaaggagcgatccggagcaaaccccaaaaacagagtcccagttcggattgcaggctgcaactcgcctgcatgaagcaggaatcgctagtaatcgcaggtcagcatactgcggtgaatacgttcccgggccttgtacacaccgcccgtcacaccacgaaagtcattcacacccgaagccggtgag

SEQ ID NO: 138 - DNA, 1373 bp, Unknown
  I33
atctagtggcaaacgggtgagtaacacgtaaacaacctgccttcaggatggggacaacagacggaaacgactgctaataccgaatacgttccttaggtcgcatgactttaggaagaaagggtggcctctacttgtaagctatcgcctgaagaggggtttgcgtctgattaggtagttggtgaggtaacggcccaccaagccgacgatcagtagccggtctgagaggatgaacggccacactggaactgagacacggtccagactcctacgggaggcagcagtggggaatcttccgcaatgggcgaaagcctgacggagcaacgccgcgtgagtgatgacggccttcgggttgtaaagctctgtgatcggggacgaacggtcagcagacgaatactctgctgaagtgacggtacccgaatagcaagccacggctaactacgtgccagcagccgcggtaatacgtaggtggcaagcgttgtccggaattattgggcgtaaagcgcgcgcaggcggcttcttaagtccatcttaaaagtgcggggcttaaccccgtgatgggatggaaactgagaggctggagtatcggagaggaaagtggaattcctagtgtagcggtgaaatgcgtagagattaggaagaacaccggtggcgaaggcgactttctggacgacaactgacgctgaggcgcgaaagcgtggggagcaaacaggattagataccctggtagtccacgccgtaaacgatgaatactaggtgtaggaggtatcgaccccttctgtgccggagctaacacaataagtattccgcctgggaagtacgatcgcaagattaaaactcaaaggaattgacgggggcccgcacaagcggtggagtatgtggtttaattcgacgcaacgcgaagaaccttaccaggtcttgacattgatcgctattccaagaaattggaagttctccttcgggagacgagaaaacaggtggtgcacggctgtcgtcagctcgtgtcgtgagatgttgggttaagtcccgcaacgagcgcaacccctatcttatgttaccagcacgttatggtggggactcatgagagaccgccgcggacaacgcggaggaaggtggggatgacgtcaagtcatcatgccccttatgacctgggctacacacgtactacaatgggtgtcaacaaagagaagcgaagccgcgaggcagagcaaacctcaaaaacacacccccagttcagattgcaggctgcaacccgcctgcatgaagtaggaatcgctagtaatcgcgggtcagcataccgcggtgaatacgttcccgggccttgtacacaccgcccgtcacactatgagagtcagaaacacccgaagccggtgagg

SEQ ID NO: 139 - DNA, 1366 bp, Unknown
  I34
ttcttagtggcgaacgggtgagtaacgcgtgggcaacctgccctccagttggggacaacattccgaaagggatgctaataccgaatgtgctccctcctccgcatggaggagggaggaaagatggcctctgcttgcaagctatcgctggaagatgggcccgcgtctgattagctagttggtggggtaacggctcaccaaggcgatgatcagtagccggtctgagaggatgaacggccacattgggactgagacacggcccaaactcctacgggaggcagcagtggggaatcttccgcaatggacgaaagtctgacggagcaacgccgcgtgagtgatgaaggtcttcggattgtaaaactctgttgttagggacgaaagcaccgtgttcgaacaggtcatggtgttgacggtacctaacgaggaagccacggctaactacgtgccagcagccgcggtaatacgtaggtggcaagcgttgtccggaattattgggcgtaaagagcatgtaggcgggcttttaagtctgacgtgaaaatgcggggcttaaccccgtatggcgttggatactggaagtcttgagtgcaggagaggaaaggggaattcccagtgtagcggtgaaatgcgtagatattgggaggaacaccagtggcgaaggcgcctttctggactgtgtctgacgctgagatgcgaaagccagggtagcaaacgggattagataccccggtagtcctggccgtaaacgatggatactaggtgtaggaggtatcgaccccttctgtgccggagttaacgcaataagtatcccgcctggggactacgatcgcaagattgaaactcaaaggaattgacgggggcccgcacaagcggtggagtatgtggtttaattcgacgcaacgcgaagaaccttaccaaggcttgacattgagtgaaagacctagagataggtccctcccttcggggacacgaaaacaggtggtgcatggctgtcgtcagctcgtgtcgtgagatgttgggttaagtcccgcaacgagcgcaacccctatcctatgttaccagcgcgtaatggcggggactcataggagactgccagggataacttggaggaaggcggggatgacgtcaagtcatcatgccccttatgtcttgggctacacacgtactacaatggtcggcaacaaagggcagcgaaaccgcgaggtggagcaaatcccagaaacccgaccccagttcggatcgtaggctgcaacccgcctacgtgaagttggaatcgctagtaatcgcaggtcagcatactgcggtgaatacgttcccgggccttgtacacaccgcccgtcacaccacgaaagttggtaacacccgaagccgg

SEQ ID NO: 140 - DNA, 1387 bp, Unknown
  I35
  misc_feature (11)..(11): n is a, c, g, or t
  misc_feature (190)..(190): n is a, c, g, or t
  misc_feature (399)..(399): n is a, c, g, or t
cttgctctttnttggattctagtggcaaacgggtgagtaacacgtaaacaacctgccttcaggatggggacaacagacggaaacgactgctaataccgaataccttccaatttccgcatggagataggaagaaagggtggcctctacttgtaagctatcgcctgaagaggggtttgcgtctgattagctngttggtgaggtaacggcccaccaaggcgacgatcagtagccggtctgagaggatgaacggccacactggaactgagacacggtccagactcctacgggaggcagcagtggggaatcttccgcaatggacgaaagtctgacggagcaacgccgcgtgaacgatgaaggtcttcggattgtaaagttctgtgatccgggacgaaggcattnattgagaacattgattgatgttgacggtaccggaaaagcaagccacggctaactacgtgccagcagccgcggtaatacgtaggtggcaagcgttgtccggaattattgggcgtaaagcgcgcgcaggcggccgtgcaagtccatcttaaaagcgtggggcttaaccccatgaggggatggaaactgcatggctggagtgtcggaggggaaagtggaattcctagtgtagcggtgaaatgcgtagagattaggaagaacaccggtggcgaaggcgactttctagacgacaactgacgctgaggcgcgaaagcgtggggagcaaacaggattagataccctggtagtccacgccgtaaacgatggatactaggtgtaggaggtatcgaccccttctgtgccggagttaacgcaataagtatcccgcctgggaagtacgatcgcaagattaaaactcaaaggaattgacgggggcccgcacaagcggtggagtatgtggtttaattcgacgcaacgcgaagaaccttaccaagccttgacattgatcgcaatctgcagaaatgcggagttcctcttcggaggacgagaaaacaggtggtgcacggctgtcgtcagctcgtgtcgtgagatgttgggttaagtcccgcaacgagcgcaacccctatcttctgttgccagcacgtaaaggtgggaactcaggagagaccgccgcggacaacgcggaggaaggcggggatgacgtcaagtcatcatgccccttatggcttgggctacacacgtactacaatgggtgcaaacaaagagaagcgaagtcgcgagacggagcggacctcataaacgcactcccagttcagattgcaggctgcaacccgcctgcatgaagtaggaatcgctagtaatcgcgggtcagcataccgcggtgaatacgttcccgggccttgtacacaccgcccgtcacactatgagagtcagagacacccaaagccggtgg

SEQ ID NO: 141 - DNA, 1386 bp, Unknown
  I36
  misc_feature (20)..(20): n is a, c, g, or t
  misc_feature (112)..(113): n is a, c, g, or t
  misc_feature (115)..(117): n is a, c, g, or t
  misc_feature (130)..(130): n is a, c, g, or t
  misc_feature (189)..(189): n is a, c, g, or t
  misc_feature (1200)..(1201): n is a, c, g, or t
gagaagcttgcttcttatcnattctagtggcaaacgggtgagtaacgcgtaagcaacctgcccttcagatggggacaacagctggaaacggctgctaataccgaatacgttnntnnngccgcatgacganatgaagaaagggaggccttcgggctttcgctggaggaggggcttgcgtctgattagctngttggaggggtaacggcccaccaaggcgacgatcagtagccggtctgagaggatgaacggccacattgggactgagacacggcccagactcctacgggaggcagcagtggggaatcttccgcaatggacgaaagtctgacggagcaacgccgcgtgaacgatgacggccttcgggttgtaaagttctgttatatgggacgaacaggacatcggttaatacccggtgtctttgacggtaccgtaagagaaagccacggctaactacgtgccagcagccgcggtaatacgtaggtggcaagcgttgtccggaattattgggcgtaaagggcgcgcaggcggcatcgcaagtcggtcttaaaagtgcggggcttaaccccgtgaggggaccgaaactgtgaagctcgagtgtcggagaggaaagcggaattcctagtgtagcggtgaaatgcgtagatattaggaggaacaccagtggcgaaagcggctttctggacgacaactgacgctgaggcgcgaaagccaggggagcaaacgggattagataccccggtagtcctggccgtaaacgatggatactaggtgtaggaggtatcgactccttctgtgccggagttaacgcaataagtatcccgcctggggagtacggccgcaaggctgaaactcaaaggaattgacgggggcccgcacaagcggtggagtatgtggtttaattcgacgcaacgcgaagaaccttaccaagccttgacattgattgctacggaaagagatttccggttcttcttcggaagacaagaaaacaggtggtgcacggctgtcgtcagctcgtgtcgtgagatgttgggttaagtcccgcaacgagcgcaacccctatcttctgttgccagcacctcgggtggggactcagaagagactgccgcagacaatgcggaggaaggcggggatgacgtcaagtcatcatgccccttatggcttgggctacacacgtactacaatggctcttaatagaggganncgaaggagcgatccggagcaaaccccaaaaacagagtcccagttcggattgcaggctgcaactcgcctgcatgaagcaggaatcgctagtaatcgcaggtcagcatactgcggtgaatacgttcccgggccttgtacacaccgcccgtcacaccacgaaagtcattcacacccgaagccggtgag

SEQ ID NO: 142 - DNA, 1364 bp, Unknown
  I37
  misc_feature (939)..(940): n is a, c, g, or t
cggcagcgcggggagcttgctccctggcggcgagtggcgcacgggtgagtaatacatcggaacgtgtcttctagtgggggataactgcccgaaagggcagctaataccgcatgagacctgagggtgaaagcgggggatcgcaagacctcgcgctggaagagcggccgatgtccgattagctagttggtgaggtaaaggctcaccaaggcgacgatcggtagctggtctgagaggacgaccagccacactgggactgagacacggcccagactcctacgggaggcagcagtggggaattttggacaatgggggcaaccctgatccagccatgccgcgtgcaggatgaaggtcttcggattgtaaactgcttttgtcagggacgaaaagggatgcgataacaccgtattccgctgacggtacctgaagaataagcaccggctaactacgtgccagcagccgcggtaatacgtagggtgcaagcgttaatcggaattactgggcgtaaagcgtgcgcaggcggttctgtaagatagatgtgaaatccccgggctcaacctgggaattgcatatatgactgcaggacttgagtttgtcagaggagggtggaattccacgtgtagcagtgaaatgcgtagatatgtggaagaacaccgatggcgaaggcagccctctgggacatgactgacgctcatgcacgaaagcgtggggagcaaacaggattagataccctggtagtccacgccctaaacgatgtctactagttgttggggacgatagtccttggtaacgcagctaacgcgtgaagtagaccgcctggggagtacggtcgcaagattaaaactcaaaggaattgacggggacccgcacaagcggtggatgatgtggattaattcgatgcaacgcgaaaaaccttacctagccttgacatgccaggaaggnntgagagatcaggccgtgcccgcaagggaatctggacacaggtgctgcatggctgtcgtcagctcgtgtcgtgagatgttgggttaagtcccgcaacgagcgcaacccttgtcattagttgctacgaaagggcactctaatgagactgccggtgacaaaccggaggaaggtggggatgacgtcaagtcctcatggcccttatggctagggcctcacacgtcatacaatggtcggaacagagggaagcgaagccgcgaggtgaagccaatcccagaaaaccgatcgtagtccggattgcagtctgcaactcgactgcatgaagtcggaatcgctagtaatcgcggatcagcatgccgcggtgaatacgttcccgggtcttgtacacaccgcccgtcacaccatgggagtggggttcaccagaagac

SEQ ID NO: 143 - DNA, 1343 bp, Unknown
  I38
ggaaacggattagcggcggacgggtgagtaacacgtgggtaacctgcctcatagaggggaatagcctcccgaaagggagattaataccgcataacattgcagtttcgcatgaaacagcaattaaaggagcaatccgctatgagatggacccgcggcgcattagctagttggtaaggtaatggcttaccaaggcgacgatgcgtagccgacctgagagggtgatcggccacattgggactgagacacggcccagactcctacgggaggcagcagtggggaatattgcacaatgggggaaaccctgatgcagcaacgccgcgtgagtgatgacggtcttcggattgtaaagctctgtctttggggacgataatgacggtacccaaggaggaagccacggctaactacgtgccagcagccgcggtaatacgtaggtggcgagcgttgtccggatttactgggcgtaaagggagcgtaggcggatttttaagtgggatgtgaaatacccgggctcaacctgggtgctgcattccaaactgggaatctagagtgcaggaggggagagtggaattcctagtgtagcggtgaaatgcgtagagattaggaagaacaccagtggcgaaggcgactctctggactgtaactgacgctgaggctcgaaagcgtggggagcgaacaggattagataccctggtagtccacgccgtaaacgatgaatactaggtgtaggggtttcaacacctctgtgccgccgctaacgcattaagtattccgcctggggagtacggtcgcaagattaaaactcaaaggaattgacgggggcccgcacaagtagcggagcatgtggtttaattcgaagcaacgcgaagaaccttacctagacttgacatcctctgcattacccttaatcggggaagttccttcgggaacagagtgacaggtggtgcatggttgtcgtcagctcgtgtcgtgagatgttgggttaagtcccgcaacgagcgcaacccctattgttagttgctaccattaagttgagcactctagcgagactgcctgggttaaccaggaggaaggtggggatgacgtcaaatcatcatgccccttatgtctagggctacacacgtgctacaatggcaagtacagagagatgcaataccgcgaggtggagctaaacttcaaaacttgtctcagttcggattgtaggctgaaactcgcctacatgaagctggagttactagtaatcgcgaatcagcatgtcgcggtgaatacgttcccgggccttgtacacaccgcccgtcacaccatgagagttggcaatacccaaagttcgtgagctaacgcgtaag

SEQ ID NO: 144 - DNA, 1318 bp, Unknown
  I39
cttagtggcggacgggtgagtaacgcgtgagtaacctgcctttcagaggggaataacattctgaaaagaatgctaataccgcatgagatcgtagtatcgcatggtacagcgaccaaaggagcaatccgctgaaagatggactcgcgtccgattagctagttggtgagataaaggcccaccaaggcgacgatcggtagccggactgagaggttgaacggccacattgggactgagacacggcccagactcctacgggaggcagcagtgggggatattgcacaatgggggaaaccctgatgcagcaacgccgcgtgaaggaagaaggtcttcggattgtaaacttctgtcctcagggaagataatgacggtacctgaggaggaagctccggctaactacgtgccagcagccgcggtaatacgtagggagcaagcgttgtccggatttactgggtgtaaagggtgcgtaggcggatctgcaagtcagtagtgaaatcccagggcttaaccctggaactgctattgaaactgtgggtcttgagtgaggtagaggcaggcggaattcccggtgtagcggtgaaatgcgtagagatcgggaggaacaccagtggcgaaggcggcctgctgggccttaactgacgctgaggcacgaaagcatgggtagcaaacaggattagataccctggtagtccatgccgtaaacgatgattactaggtgtgggtggtctgaccccatccgtgccggagttaacacaataagtaatccacctggggagtacggccgcaaggttgaaactcaaaggaattgacgggggcccgcacaagcagtggagtatgtggtttaattcgaagcaacgcgaagaaccttaccaggtcttgacatcctgctaacgaggtagagatacgttaggtgcccttcggggaaagcagagacaggtggtgcatggttgtcgtcagctcgtgtcgtgagatgttgggttaagtcccgcaacgagcgcaacccctgctattagttgctacgcaagagcactctaataggactgccgttgacaaaacggaggaaggtggggacgacgtcaaatcatcatgccccttatgacctgggctacacacgtactacaatggccgtcaacagagagaagcaaagccgcgaggtggagcaaaactctaaaaacggtcccagttcggatcgtaggctgcaacccgcctacgtgaagttggaattgctagtaatcgcggatcatcatgccgcggtgaatacgttcccgggccttgtacacaccgcccgtcacaccatgggagccggtaatacccgaagtca

SEQ ID NO: 145 - DNA, 1360 bp, Unknown
  I40
tcatgacagaggattcgtccaatggagtgagttacttagtggcggacgggtgagtaacgcgtgagtaacctgccttggagtggggaataacaggtggaaacatctgctaataccgcatgatgcagttgggtcgcatggctctgactgccaaagatttatcgctctgagatggactcgcgtctgattagctggttggcggggtaacggcccaccaaggcgacgatcagtagccggactgagaggttggccggccacattgggactgagacacggcccagactcctacgggaggcagcagtggggaatattgggcaatgggcgcaagcctgacccagcaacgccgcgtgaaggaagaaggctttcgggttgtaaacttcttttctcagggacgaagcaagtgacggtacctgaggaataagccacggctaactacgtgccagcagccgcggtaatacgtaggtggcgagcgttatccggatttactgggtgtaaagggcgtgtaggcgggactgcaagtcagatgtgaaaaccatgggctcaacctgtggcctgcatttgaaactgtagttcttgagtactggagaggcagacggaattcctagtgtagcggtgaaatgcgtagatattaggaggaacaccagtggcgaaggcggtctgctggacagcaactgacgctgaggcgcgaaagcgtggggagcaaacaggattagataccctggtagtccacgctgtaaacgatggatactaggtgtggggggtctgaccccctccgtgccgcagttaacacaataagtatcccacctggggagtacgatcgcaaggttgaaactcaaaggaattgacgggggcccgcacaagcggtggagtatgtggtttaattcgaagcaacgcgaagaaccttaccagggcttgacatcccggtgaccggtgtagagatacaccttcttcttcggaagcgccggtgacaggtggtgcatggttgtcgtcagctcgtgtcgtgagatgttgggttaagtcccgcaacgagcgcaacccttattgttagttgctacgcaagagcactctagcgagactgccgttgacaaaacggaggaaggtggggacgacgtcaaatcatcatgccccttatgtcctgggccacacacgtactacaatggtggtcaacagagggaagcaagaccgcgaggtggagcaaacccctaaaagccatcccagttcggattgcaggctgcaactcgcctgtatgaagttggaatcgctagtaatcgcggatcagcatgccgcggtgaatacgttcccgggccttgtacacaccgcccgtcacaccatgagagtcgggaacacccgaagtccgtagcct

SEQ ID NO: 146 - DNA, 1370 bp, Unknown
  I41
gtgctcatgacggagttttcggacaacggattgggttacttagtggcggacgggtgagtaacgcgtgaggaacctgcctcggagtggggaataacacaccgaaaggtgtgctaataccgcataatgcagttgggtcgcatgactctgactgccaaagatttatcgctctgagatggcctcgcgtctgattagctagttggcggggtaacggcccaccaaggcgacgatcagtagccggactgagaggttgaccggccacattgggactgagacacggcccagactcctacgggaggcagcagtggggaatattgggcaatgggcgcaagcctgacccagcaacgccgcgtgaaggaagaaggctttcgggttgtaaacttcttttgtcagggacgaaacaaatgacggtacctgacgaataagccacggctaactacgtgccagcagccgcggtaatacgtaggtggcaagcgttatccggatttactgggtgtaaagggcgtgtaggcgggactgcaagtcaggtgtgaaaaccaggggctcaacctctggcctgcatttgaaactgtagttcttgagtgctggagaggcaatcggaattccgtgtgtagcggtgaaatgcgtagatatacggaggaacaccagtggcgaaggcggattgctggacagtaactgacgctgaggcgcgaaagcgtggggagcaaacaggattagataccctggtagtccacgccgtaaacgatggatactaggtgtggggggactgaccccctccgtgccgcagttaacacaataagtatcccacctggggagtacgatcgcaaggttgaaactcaaaggaattgacgggggcccgcacaagcggtggagtatgtggtttaattcgaagcaacgcgaagaaccttaccagggcttgacatcctactaacgaagcagagatgcattaggtgcccttcggggaaagtagagacaggtggtgcatggttgtcgtcagctcgtgtcgtgagatgttgggttaagtcccgcaacgagcgcaacccctattgttagttgctacgcaagagcactctagcgagactgccgttgacaaaacggaggaaggtggggacgacgtcaaatcatcatgccccttatgtcctgggccacacacgtactacaatggtggttaacagaggggagcaataccgcgaggtggagcaaatccctaaaagccatcccagttcggattgcaggctgaaacccgcctgtatgaagttggaatcgctagtaatcgcggatcagcatgccgcggtgaatacgttcccgggccttgtacacaccgcccgtcacaccatgagagtcgggaacacccgaagtccgtagcctaaccg

SEQ ID NO: 147 - DNA, 1341 bp, Unknown
  I42
  misc_feature (120)..(121): n is a, c, g, or t
ttgcaccttcaagttagtggcggacgggtgagtaacgcgtgagcaacctgcctcaaagagggggataacgtctggaaacggacgctaataccgcatgacgtattcgataggcatctattnnataccaaaggagcaatccgctttgagatgggctcgcgtctgattagctggttggtggggtaaaggcctaccaaggcgacgatcagtagccggactgagaggttgaacggccacattgggactgagacacggcccagactcctacgggaggcagcagtgggggatattgcacaatgggggaaaccctgatgcagcaacgccgcgtgaaggaagacggttttcggattgtaaacttctgttcttagtgacgataatgacggtagctaaggagaaagctccggctaactacgtgccagcagccgcggtaatacgtagggagcgagcgttgtccggaattactgggtgtaaagggagcgtaggcgggagatcaagtcagatgtgaaaactatgggctcaacccataacctgcatttgaaactggttttcttgagtgaagtagaggcaggcggaattccgagtgtagcggtgaaatgcgtagatattcggaggaacaccagtggcgaaggcggcctgctgggcttttactgacgctgaggctcgaaagcatggggagcaaacaggattagataccctggtagtccatgccgtaaacgatgattactaggtgtggggtggctgacccattccgtgccggagttaacacaataagtaatccacctggggagtacggccgcaaggttgaaactcaaaggaattgacgggggcccgcacaagcagtggagtatgtggtttaattcgaagcaacgcgaagaaccttaccaggtcttgacatccgactaacgaagtagagatacattaggtgcccttcggggaaagtcgagacaggtggtgcatggttgtcgtcagctcgtgtcgtgagatgttgggttaagtcccgcaacgagcgcaacccttgtcattagttgctacgcaagagcactctaatgagactgccgttgacaaaacggaggaaggtggggacgacgtcaaatcatcatgccccttatgacctgggctacacacgtactacaatggccgttaacagagggaagcaatactgtgaagtggagcaaacccctaaaaacggtcccagttcagattgcaggctgcaacccgcctgcatgaagtcggaattgctagtaatcgcggatcagcatgccgcggtgaatacgttcccgggccttgtacacaccgcccgtcacaccatgggagccggtaatacccgaagtcggtagtctaacc

SEQ ID NO: 148 - DNA, 20 bp, Artificial Sequence
  27Forward-mod
agrgtttgatymtggctcag

SEQ ID NO: 149 - DNA, 19 bp, Artificial Sequence
  1492Reverse
ggytaccttgttacgactt

SEQ ID NO: 150 - DNA, 20 bp, Artificial Sequence
  f01_42H6_Fw1
agctttcgcggtatgggatg

SEQ ID NO: 151 - DNA, 20 bp, Artificial Sequence
  f01_42H6_Rv1
gccgtatctcagtcccaatg

SEQ ID NO: 152 - DNA, 20 bp, Artificial Sequence
  f02_42I8_Fw1
caaactaaagatggcgaccg

SEQ ID NO: 153 - DNA, 21 bp, Artificial Sequence
  f02_42I8_Rv3
gcggttttaatatactatcgg

SEQ ID NO: 154 - DNA, 20 bp, Artificial Sequence
  f05_43D4_Fw4
cccgatggtataatcagacc

SEQ ID NO: 155 - DNA, 20 bp, Artificial Sequence
  f05_43D4_Rv2
acctcaccaactgcctaatg

SEQ ID NO: 156 - DNA, 20 bp, Artificial Sequence
  f06_42F4_Fw1
taggcggacgcttaagtcag

SEQ ID NO: 157 - DNA, 20 bp, Artificial Sequence
  f06_42F4_Rv1
ctgcctctactgtactcaag

SEQ ID NO: 158 - DNA, 20 bp, Artificial Sequence
  f07_42J6_Fw1
ttgcaaactggagatggcga

SEQ ID NO: 159 - DNA, 21 bp, Artificial Sequence
  f07_42J6_Rv1
ctcatgcgggagaaatatacc

SEQ ID NO: 160 - DNA, 20 bp, Artificial Sequence
  f08_42B5_Fw1
atccaacctgccctttactc

SEQ ID NO: 161 - DNA, 20 bp, Artificial Sequence
  f08_42B5_Rv1
cccatcctttaccggaatcc

SEQ ID NO: 162 - DNA, 20 bp, Artificial Sequence
  f09_43F1_Fw1
gaaagtcggactaataccgc

SEQ ID NO: 163 - DNA, 20 bp, Artificial Sequence
  f09_43F1_Rv1
cctcaccaactatctaatgg

SEQ ID NO: 164 - DNA, 20 bp, Artificial Sequence
  f10_43J3_Fw1
ttgaagccttggtgactgag

SEQ ID NO: 165 - DNA, 20 bp, Artificial Sequence
  f10_43J3_Rv1
ttagcagccgtttccaactg

SEQ ID NO: 166 - DNA, 21 bp, Artificial Sequence
  f12_42H4_Fw1
acacgtgatcgcatgatcgag

SEQ ID NO: 167 - DNA, 20 bp, Artificial Sequence
  f12_42H4_Rv1
ccaactagctaatcagacgc

SEQ ID NO: 168 - DNA, 19 bp, Artificial Sequence
  f13_42H8_Fw1
acagcttcgcatggagcag

SEQ ID NO: 169 - DNA, 20 bp, Artificial Sequence
  f13_42H8_Rv1
ctgatcgtcgccttggtaag

SEQ ID NO: 170 - DNA, 21 bp, Artificial Sequence
  f14_42L4_Fw1
acagtgctgcatggcacagtg

SEQ ID NO: 171 - DNA, 20 bp, Artificial Sequence
  f14_42L4_Rv1
tcgccttggtaggccgttac

SEQ ID NO: 172 - DNA, 20 bp, Artificial Sequence
  f16_43M1_Fw2
ctgaagatttggtgattgag

SEQ ID NO: 173 - DNA, 22 bp, Artificial Sequence
  f16_43M1_Rv2
accatgcggtgctgtggtctta

SEQ ID NO: 174 - DNA, 22 bp, Artificial Sequence
  f17_42I7_Fw3
atggaagcttcggtggaaatag

SEQ ID NO: 175 - DNA, 20 bp, Artificial Sequence
  f17_42I7_Rv3
cacactgaatcatgcagtcc

SEQ ID NO: 176 - DNA, 20 bp, Artificial Sequence
  f18_42I2_Fw5
gcgaagcaagtctgaagtga

SEQ ID NO: 177 - DNA, 20 bp, Artificial Sequence
  f18_42I2_Rv5
ctccgacactctagcaaaac

SEQ ID NO: 178 - DNA, 21 bp, Artificial Sequence
  f19_43G2_Fw2
cggttgaagtcgttataatcc

SEQ ID NO: 179 - DNA, 21 bp, Artificial Sequence
  f19_43G2_Rv2
ccatgcagtcccgtgcgctta

SEQ ID NO: 180 - DNA, 21 bp, Artificial Sequence
  f20_43G1_Fw2
cttgcttccaaagagacttag

SEQ ID NO: 181 - DNA, 20 bp, Artificial Sequence
  f20_43G1_Rv2
gcagttatcccggacacatg

SEQ ID NO: 182 - DNA, 20 bp, Artificial Sequence
  f21_42A8_Fw2
aagtggatctcttcggattg

SEQ ID NO: 183 - DNA, 20 bp, Artificial Sequence
  f21_42A8_Rv6
ttatgcggtattagcagcca

SEQ ID NO: 184 - DNA, 20 bp, Artificial Sequence
  f22_43C3_Fw2
gattctgagatgactgagtg

SEQ ID NO: 185 - DNA, 20 bp, Artificial Sequence
  f22_43C3_Rv2
gcagtcatttctaactgttg

SEQ ID NO: 186 - DNA, 20 bp, Artificial Sequence
  f24_42I4_Fw1
tcggtataacttagtggcgg

SEQ ID NO: 187 - DNA, 20 bp, Artificial Sequence
  f24_42I4_Rv1
acaaccatgcggttccgtgc

SEQ ID NO: 188 - DNA, 20 bp, Artificial Sequence
  f25_42J1_Fw2
taccggatttcttcgggatg

SEQ ID NO: 189 - DNA, 20 bp, Artificial Sequence
  f25_42J1_Rv2
gatcatgcaatcctgtggtc

SEQ ID NO: 190 - DNA, 20 bp, Artificial Sequence
  f26_42K2_Fw1
tttatcgctctgagatggcc

SEQ ID NO: 191 - DNA, 20 bp, Artificial Sequence
  f26_42K2_Rv1
tcaacctctcagtccggcta

SEQ ID NO: 192 - DNA, 20 bp, Artificial Sequence
  f27_42J5_Fw2
gggaatcacttcattgagac

SEQ ID NO: 193 - DNA, 20 bp, Artificial Sequence
  f27_42J5_Rv2
gactgttatccccctgtata

SEQ ID NO: 194 - DNA, 20 bp, Artificial Sequence
  f28_43A3_Fw1
gtacacacggataacatacc

SEQ ID NO: 195 - DNA, 20 bp, Artificial Sequence
  f28_43A3_Rv1
accaactagctaatcagacg

SEQ ID NO: 196 - DNA, 19 bp, Artificial Sequence
  f29_43J8_Fw2
cttcggattgaagcaattg

SEQ ID NO: 197 - DNA, 20 bp, Artificial Sequence
  f29_43J8_Rv2
ttagcagccgtttccaactg

SEQ ID NO: 198 - DNA, 20 bp, Artificial Sequence
  f30_43A5_Fw1
tatcccacgggatagcacag

SEQ ID NO: 199 - DNA, 20 bp, Artificial Sequence
  f30_43A5_Rv1
tctcaggccggctacgcatc

SEQ ID NO: 200 - DNA, 20 bp, Artificial Sequence
  f31_43J5_Fw1
ttccttaatgactgagtggc

SEQ ID NO: 201 - DNA, 20 bp, Artificial Sequence
  f31_43J5_Rv2
cacaccgaatcatgcgattc

SEQ ID NO: 202 - DNA, 20 bp, Artificial Sequence
  f32_42A7_Fw1
tgaagtctttgtgactgagc

SEQ ID NO: 203 - DNA, 18 bp, Artificial Sequence
  f32_42A7_Rv2
atgcggtattagcagtca

SEQ ID NO: 204 - DNA, 20 bp, Artificial Sequence
  f33_43N2_Fw1
gtgcctcaaagcactggtag

SEQ ID NO: 205 - DNA, 20 bp, Artificial Sequence
  f33_43N2_Rv1
tctcaggtcggctacgcatc

SEQ ID NO: 206 - DNA, 20 bp, Artificial Sequence
  f34_43K4_Fw1
taagctatcactgaaggagg

SEQ ID NO: 207 - DNA, 20 bp, Artificial Sequence
  f34_43K4_Rv1
cagaccggctactgatcatc

SEQ ID NO: 208 - DNA, 20 bp, Artificial Sequence
  f35_42L8_Fw2
acttgatccttcgggtgaag

SEQ ID NO: 209 - DNA, 20 bp, Artificial Sequence
  f35_42L8_Rv2
atgttgtcccagtctgtaag

SEQ ID NO: 210 - DNA, 20 bp, Artificial Sequence
  f37_42G1_Fw3
gctgctttgctgacgagtgg

SEQ ID NO: 211 - DNA, 20 bp, Artificial Sequence
  f37_42G1_Rv4
ttggtcttgcgacgttatgc

SEQ ID NO: 212 - DNA, 19 bp, Artificial Sequence
  KPC-F684
ggcagtcggagacaaaacc

SEQ ID NO: 213 - DNA, 18 bp, Artificial Sequence
  KPC-R860
ccctcgagcgcgagtcta

SEQ ID NO: 214 - DNA, 21 bp, Artificial Sequence
  VanABF_JCM1998?
gtaggctgcgatattcaaagc

SEQ ID NO: 215 - DNA, 21 bp, Artificial Sequence
  VanAR_JCM1998?
cgattcaattgcgtagtccaa

SEQ ID NO: 216 - DNA, 24 bp, Artificial Sequence
  ESBL-F_AAC2001
gaaagatccactatcgccagcagg

SEQ ID NO: 217 - DNA, 22 bp, Artificial Sequence
  ESBL-R_AAC2001
gttgccagtgctcgatcagcgc

SEQ ID NO: 218 - DNA, 21 bp, Artificial Sequence
  LF82-F
ccattcatgcagcagctcttt

SEQ ID NO: 219 - DNA, 21 bp, Artificial Sequence
  LF82-R
atcggacaacattagcggtgt

SEQ ID NO: 220 - DNA, 25 bp, Artificial Sequence
  C.jejuni_F
ctgaatttgataccttaagtgcagc

SEQ ID NO: 221 - DNA, 22 bp, Artificial Sequence
  C.jejuni_R
aggcacgcctaaacctatagct

SEQ ID NO: 222 - DNA, 20 bp, Artificial Sequence
  Universal_Fw_1387
cttgtacacaccgcccgtca

SEQ ID NO: 223 - DNA, 22 bp, Artificial Sequence
  Universal_Rv_1492
tacggctaccttgttacgactt

SEQ ID NO: 224 - DNA, 23 bp, Artificial Sequence
  tpi-F
aaagaagctactaagggtacaaa

SEQ ID NO: 225 - DNA, 23 bp, Artificial Sequence
  tpi-R
cataatattgggtctattcctac

SEQ ID NO: 226 - DNA, 20 bp, Artificial Sequence
  Cupsaliensis_2F
aaatcagccatgttgcggtg

SEQ ID NO: 227 - DNA, 20 bp, Artificial Sequence
  Cupsaliensis_2R
tcaactcccatggtgtgacg

SEQ ID NO: 228 - DNA, 20 bp, Artificial Sequence
  Cupsaliensis_3F
caaatcagccatgttgcggt

SEQ ID NO: 229 - DNA, 20 bp, Artificial Sequence
  Cupsaliensis_3R
ccagtcgctgattccactgt

SEQ ID NO: 230 - DNA, 16 bp, Artificial Sequence
  khe-Fw
tggggatccaccacga

SEQ ID NO: 231 - DNA, 22 bp, Artificial Sequence
  khe-RV
agagatagccgtttatccacac

SEQ ID NO: 232 - DNA, 20 bp, Artificial Sequence
  Eg_2F
tgcgtcactgatggatggac

SEQ ID NO: 233 - DNA, 20 bp, Artificial Sequence
  Eg_2R
tgccgaagattccctactgc

SEQ ID NO: 234 - DNA, 20 bp, Artificial Sequence
  P.mirabillis_NatMicro_F
gttattcgtgatggtatggg

SEQ ID NO: 235 - DNA, 20 bp, Artificial Sequence
  P.mirabillis_NatMicro_R
ataaaggtggttacgccaga